European Patent Specification EP 4 041 918 B1, published December 10, 2025. Title: COMPOSITIONS AND METHODS FOR ASSESSING MICROBIAL POPULATIONS. Applicant: Life Technologies Corporation. The sequence listing filed with the application follows.

SEQUENCE LISTING (1979 sequences)

SEQ ID NO: 1 - DNA, 17 bp, Artificial
  synthetic sequence
ggcggacgggugaguaa

SEQ ID NO: 2 - DNA, 18 bp, Artificial
  synthetic sequence
agtcuggaccgtgtcuca

SEQ ID NO: 3 - DNA, 17 bp, Artificial
  synthetic sequence
ggcgcacgggugaguaa

SEQ ID NO: 4 - DNA, 18 bp, Artificial
  synthetic sequence
agtcuggaccgtgtcuca

SEQ ID NO: 5 - DNA, 17 bp, Artificial
  synthetic sequence
ggcgaacgggugaguaa

SEQ ID NO: 6 - DNA, 18 bp, Artificial
  synthetic sequence
agtcuggaccgtgtcuca

SEQ ID NO: 7 - DNA, 20 bp, Artificial
  synthetic sequence
acuccuacgggaggcagcag

SEQ ID NO: 8 - DNA, 19 bp, Artificial
  synthetic sequence
acggagtuagccggtgcut

SEQ ID NO: 9 - DNA, 18 bp, Artificial
  synthetic sequence
cagcagccgcgguaauac

SEQ ID NO: 10 - DNA, 18 bp, Artificial
  synthetic sequence
cgcattucaccgcuacac

SEQ ID NO: 11 - DNA, 24 bp, Artificial
  synthetic sequence
gggagcaaacaggautagauaccc

SEQ ID NO: 12 - DNA, 23 bp, Artificial
  synthetic sequence
cccccgtcaautcatttgagtut

SEQ ID NO: 13 - DNA, 24 bp, Artificial
  synthetic sequence
atgtgguttaattcgaugcaacgc

SEQ ID NO: 14 - DNA, 21 bp, Artificial
  synthetic sequence
tucacaacacgagcugacgac

SEQ ID NO: 15 - DNA, 19 bp, Artificial
  synthetic sequence
tgggutaagucccgcaacg

SEQ ID NO: 16 - DNA, 21 bp, Artificial
  synthetic sequence
aagggccaugatgactugacg

SEQ ID NO: 17 - DNA, 18 bp, Artificial
  synthetic sequence
gggcuacacacgcgcuac

SEQ ID NO: 18 - DNA, 18 bp, Artificial
  synthetic sequence
cccgggaacguatucacc

SEQ ID NO: 19 - DNA, 18 bp, Artificial
  synthetic sequence
gggcuacacacgugcaac

SEQ ID NO: 20 - DNA, 18 bp, Artificial
  synthetic sequence
cccgggaacguatucacc

SEQ ID NO: 21 - DNA, 18 bp, Artificial
  synthetic sequence
gggcuacacacgtgcuac

SEQ ID NO: 22 - DNA, 18 bp, Artificial
  synthetic sequence
cccgggaacguatucacc

SEQ ID NO: 23 - DNA, 18 bp, Artificial
  synthetic sequence
ttcccgggccutguacac

SEQ ID NO: 24 - DNA, 22 bp, Artificial
  synthetic sequence
cutgttacgactucaccccagt

SEQ ID NO: 25 - DNA, 17 bp, Artificial
  synthetic sequence
ggcggacgggtgagtaa

SEQ ID NO: 26 - DNA, 18 bp, Artificial
  synthetic sequence
agtctggaccgtgtctca

SEQ ID NO: 27 - DNA, 17 bp, Artificial
  synthetic sequence
ggcgcacgggtgagtaa

SEQ ID NO: 28 - DNA, 18 bp, Artificial
  synthetic sequence
agtctggaccgtgtctca

SEQ ID NO: 29 - DNA, 17 bp, Artificial
  synthetic sequence
ggcgaacgggtgagtaa

SEQ ID NO: 30 - DNA, 18 bp, Artificial
  synthetic sequence
agtctggaccgtgtctca

SEQ ID NO: 31 - DNA, 20 bp, Artificial
  synthetic sequence
actcctacgggaggcagcag

SEQ ID NO: 32 - DNA, 19 bp, Artificial
  synthetic sequence
acggagttagccggtgctt

SEQ ID NO: 33 - DNA, 18 bp, Artificial
  synthetic sequence
cagcagccgcggtaatac

SEQ ID NO: 34 - DNA, 18 bp, Artificial
  synthetic sequence
cgcatttcaccgctacac

SEQ ID NO: 35 - DNA, 24 bp, Artificial
  synthetic sequence
gggagcaaacaggattagataccc

SEQ ID NO: 36 - DNA, 23 bp, Artificial
  synthetic sequence
cccccgtcaattcatttgagttt

SEQ ID NO: 37 - DNA, 24 bp, Artificial
  synthetic sequence
atgtggtttaattcgatgcaacgc

SEQ ID NO: 38 - DNA, 21 bp, Artificial
  synthetic sequence
ttcacaacacgagctgacgac

SEQ ID NO: 39 - DNA, 19 bp, Artificial
  synthetic sequence
tgggttaagtcccgcaacg

SEQ ID NO: 40 - DNA, 21 bp, Artificial
  synthetic sequence
aagggccatgatgacttgacg

SEQ ID NO: 41 - DNA, 18 bp, Artificial
  synthetic sequence
gggctacacacgcgctac

SEQ ID NO: 42 - DNA, 18 bp, Artificial
  synthetic sequence
cccgggaacgtattcacc

SEQ ID NO: 43 - DNA, 18 bp, Artificial
  synthetic sequence
gggctacacacgtgcaac

SEQ ID NO: 44 - DNA, 18 bp, Artificial
  synthetic sequence
cccgggaacgtattcacc

SEQ ID NO: 45 - DNA, 18 bp, Artificial
  synthetic sequence
gggctacacacgtgctac

SEQ ID NO: 46 - DNA, 18 bp, Artificial
  synthetic sequence
cccgggaacgtattcacc

SEQ ID NO: 47 - DNA, 18 bp, Artificial
  synthetic sequence
ttcccgggccttgtacac

SEQ ID NO: 48 - DNA, 22 bp, Artificial
  synthetic sequence
cttgttacgacttcaccccagt

SEQ ID NO: 49 - DNA, 18 bp, Artificial
  synthetic sequence
accaaggutcuagccggt

SEQ ID NO: 50 - DNA, 19 bp, Artificial
  synthetic sequence
ggcttgguggcagtaagug

SEQ ID NO: 51 - DNA, 18 bp, Artificial
  synthetic sequence
accauctggatugccgca

SEQ ID NO: 52 - DNA, 24 bp, Artificial
  synthetic sequence
agtgaaacaacaguattgaugccg

SEQ ID NO: 53 - DNA, 30 bp, Artificial
  synthetic sequence
acatttgctgaaucttttgctcttttuact

SEQ ID NO: 54 - DNA, 28 bp, Artificial
  synthetic sequence
tcaagataaaggacaucaagtgtuaggt

SEQ ID NO: 55 - DNA, 27 bp, Artificial
  synthetic sequence
catctactgaagcugcttcaaatuagt

SEQ ID NO: 56 - DNA, 30 bp, Artificial
  synthetic sequence
tttgctctttgauatttttgccauacagat

SEQ ID NO: 57 - DNA, 31 bp, Artificial
  synthetic sequence
atcttgaataguaacttttaaacttugccct

SEQ ID NO: 58 - DNA, 30 bp, Artificial
  synthetic sequence
gattctgctaaacuaatcgaagaggtuaga

SEQ ID NO: 59 - DNA, 26 bp, Artificial
  synthetic sequence
cagcgaataauaattcccctugacag

SEQ ID NO: 60 - DNA, 24 bp, Artificial
  synthetic sequence
ggatgactttcuatcggcactuca

SEQ ID NO: 61 - DNA, 21 bp, Artificial
  synthetic sequence
gcaacagcacutcguaacgat

SEQ ID NO: 62 - DNA, 25 bp, Artificial
  synthetic sequence
ggagaaccaaautcaacacgagtut

SEQ ID NO: 63 - DNA, 25 bp, Artificial
  synthetic sequence
aattcacagctugaggaaaaggugt

SEQ ID NO: 64 - DNA, 20 bp, Artificial
  synthetic sequence
tggcaacauctgtucaggac

SEQ ID NO: 65 - DNA, 17 bp, Artificial
  synthetic sequence
tgcgttgcucgctcuct

SEQ ID NO: 66 - DNA, 25 bp, Artificial
  synthetic sequence
tgcactcttucagaaagaaggtcut

SEQ ID NO: 67 - DNA, 21 bp, Artificial
  synthetic sequence
acgaagaagcuguggagaagt

SEQ ID NO: 68 - DNA, 20 bp, Artificial
  synthetic sequence
ccutgagacuaccagggagc

SEQ ID NO: 69 - DNA, 33 bp, Artificial
  synthetic sequence
aaaagtaaacaauaagaaagaggttcaataugc

SEQ ID NO: 70 - DNA, 18 bp, Artificial
  synthetic sequence
cgcgcaacauagacuccc

SEQ ID NO: 71 - DNA, 32 bp, Artificial
  synthetic sequence
aattgttcctcaucaactattttaattcctug

SEQ ID NO: 72 - DNA, 26 bp, Artificial
  synthetic sequence
gtagcgaggaggautatagugaaaga

SEQ ID NO: 73 - DNA, 26 bp, Artificial
  synthetic sequence
gtggctttcttaugtgcatggattug

SEQ ID NO: 74 - DNA, 32 bp, Artificial
  synthetic sequence
tattcgtaattagaguaggaggagaagcttut

SEQ ID NO: 75 - DNA, 21 bp, Artificial
  synthetic sequence
tgtggcacaugacagtcgtug

SEQ ID NO: 76 - DNA, 20 bp, Artificial
  synthetic sequence
cataagguctttgcgcuggt

SEQ ID NO: 77 - DNA, 23 bp, Artificial
  synthetic sequence
gtggcaatuacttgcgtattugg

SEQ ID NO: 78 - DNA, 20 bp, Artificial
  synthetic sequence
cctgcucaacccctatcugg

SEQ ID NO: 79 - DNA, 28 bp, Artificial
  synthetic sequence
agacaaagtaucaacattgctcauacct

SEQ ID NO: 80 - DNA, 20 bp, Artificial
  synthetic sequence
cgaaagcgggaaugcuccaa

SEQ ID NO: 81 - DNA, 24 bp, Artificial
  synthetic sequence
aaatgaatggguagaagctggugt

SEQ ID NO: 82 - DNA, 25 bp, Artificial
  synthetic sequence
ttaagataactaggucgccgacuac

SEQ ID NO: 83 - DNA, 24 bp, Artificial
  synthetic sequence
ttcagcttcautagaagaccucgg

SEQ ID NO: 84 - DNA, 26 bp, Artificial
  synthetic sequence
cgtcaattuggactttactgatugga

SEQ ID NO: 85 - DNA, 29 bp, Artificial
  synthetic sequence
tcaccatcaaguagaactgtattttgugt

SEQ ID NO: 86 - DNA, 21 bp, Artificial
  synthetic sequence
ccagaagaautgctuccccat

SEQ ID NO: 87 - DNA, 32 bp, Artificial
  synthetic sequence
acaatattggtctuttatttttagcaactugt

SEQ ID NO: 88 - DNA, 27 bp, Artificial
  synthetic sequence
agcttatatugaggattgtggcuacac

SEQ ID NO: 89 - DNA, 20 bp, Artificial
  synthetic sequence
tcggtgucattgggaucgac

SEQ ID NO: 90 - DNA, 17 bp, Artificial
  synthetic sequence
cugggcgacgacgctut

SEQ ID NO: 91 - DNA, 20 bp, Artificial
  synthetic sequence
gugccgtcatugaccagcat

SEQ ID NO: 92 - DNA, 17 bp, Artificial
  synthetic sequence
cggagggcuaucgcgga

SEQ ID NO: 93 - DNA, 23 bp, Artificial
  synthetic sequence
gtgccuaaaagcacaagcaatug

SEQ ID NO: 94 - DNA, 28 bp, Artificial
  synthetic sequence
agggagtttaaaaaugaaacgcttucaa

SEQ ID NO: 95 - DNA, 32 bp, Artificial
  synthetic sequence
aaaggtgagaggauttaggactttttacuaaa

SEQ ID NO: 96 - DNA, 32 bp, Artificial
  synthetic sequence
ctagagagatagcaccuactataacagattuc

SEQ ID NO: 97 - DNA, 23 bp, Artificial
  synthetic sequence
agagaaaccagutggcctttugg

SEQ ID NO: 98 - DNA, 28 bp, Artificial
  synthetic sequence
aacaaatccucgatttatttcauggcag

SEQ ID NO: 99 - DNA, 32 bp, Artificial
  synthetic sequence
aatggatttattttgautccgaatatgcttut

SEQ ID NO: 100 - DNA, 33 bp, Artificial
  synthetic sequence
attgccaatattcaaucttctaaattcaucaat

SEQ ID NO: 101 - DNA, 31 bp, Artificial
  synthetic sequence
ttggcaatgtgauctttattgcaatttaaut

SEQ ID NO: 102 - DNA, 31 bp, Artificial
  synthetic sequence
agaaatgagatagcutttaataatcacugca

SEQ ID NO: 103 - DNA, 24 bp, Artificial
  synthetic sequence
gctgcagggautattctttcucca

SEQ ID NO: 104 - DNA, 25 bp, Artificial
  synthetic sequence
agggctcuatctatcagaaucggaa

SEQ ID NO: 105 - DNA, 22 bp, Artificial
  synthetic sequence
agagcccutctcgaatauggga

SEQ ID NO: 106 - DNA, 22 bp, Artificial
  synthetic sequence
aaatcgggugcaccttctguaa

SEQ ID NO: 107 - DNA, 22 bp, Artificial
  synthetic sequence
agcaaaagcutgcatatuggca

SEQ ID NO: 108 - DNA, 28 bp, Artificial
  synthetic sequence
acctctataggugtccgttattttgaug

SEQ ID NO: 109 - DNA, 30 bp, Artificial
  synthetic sequence
gcgttctccaucttttatagcagaaauacg

SEQ ID NO: 110 - DNA, 31 bp, Artificial
  synthetic sequence
ttattttagtgggtuctgcaatgacaagaua

SEQ ID NO: 111 - DNA, 27 bp, Artificial
  synthetic sequence
aacaattctttuagcctaacagugcca

SEQ ID NO: 112 - DNA, 25 bp, Artificial
  synthetic sequence
gcgaaagttacutaggtggtctugc

SEQ ID NO: 113 - DNA, 32 bp, Artificial
  synthetic sequence
gttatgaagcttatuaatggtagtggtgauga

SEQ ID NO: 114 - DNA, 29 bp, Artificial
  synthetic sequence
cctcaaattgatcutctgctgaagtatua

SEQ ID NO: 115 - DNA, 17 bp, Artificial
  synthetic sequence
tuggcggauacagccct

SEQ ID NO: 116 - DNA, 23 bp, Artificial
  synthetic sequence
atccagacuctcctgattgucca

SEQ ID NO: 117 - DNA, 22 bp, Artificial
  synthetic sequence
gatctgccauagaatctcgucg

SEQ ID NO: 118 - DNA, 20 bp, Artificial
  synthetic sequence
cggcugaagaagagugggaa

SEQ ID NO: 119 - DNA, 17 bp, Artificial
  synthetic sequence
tccgggcagcgagucug

SEQ ID NO: 120 - DNA, 19 bp, Artificial
  synthetic sequence
ggcagaucgatugcagggt

SEQ ID NO: 121 - DNA, 30 bp, Artificial
  synthetic sequence
aaaaacggaggagacuaattaatauggcaa

SEQ ID NO: 122 - DNA, 31 bp, Artificial
  synthetic sequence
tgcttttgcttcutgtaattacgaatuaact

SEQ ID NO: 123 - DNA, 22 bp, Artificial
  synthetic sequence
ccggtugaccgtatacuacgct

SEQ ID NO: 124 - DNA, 29 bp, Artificial
  synthetic sequence
cacaatcgttttuagctagaatcactgut

SEQ ID NO: 125 - DNA, 19 bp, Artificial
  synthetic sequence
ggaacagccguctgaucac

SEQ ID NO: 126 - DNA, 30 bp, Artificial
  synthetic sequence
aaaaacactcatugttttcatcgttttuca

SEQ ID NO: 127 - DNA, 23 bp, Artificial
  synthetic sequence
ccaaagactucgagtagggctug

SEQ ID NO: 128 - DNA, 26 bp, Artificial
  synthetic sequence
gattgttcataugggctctcctaucc

SEQ ID NO: 129 - DNA, 25 bp, Artificial
  synthetic sequence
cgccgaatgaugttcgaaatauggt

SEQ ID NO: 130 - DNA, 25 bp, Artificial
  synthetic sequence
ccgacaatcucaagaaaacgcugat

SEQ ID NO: 131 - DNA, 20 bp, Artificial
  synthetic sequence
acgggtctuagcattggcut

SEQ ID NO: 132 - DNA, 19 bp, Artificial
  synthetic sequence
gcacgcgucaatuaagccc

SEQ ID NO: 133 - DNA, 22 bp, Artificial
  synthetic sequence
tcaatggtuaagttggccguag

SEQ ID NO: 134 - DNA, 21 bp, Artificial
  synthetic sequence
acgatcacucaaaatggugcg

SEQ ID NO: 135 - DNA, 24 bp, Artificial
  synthetic sequence
ccaaagcatuggcatatgcagaua

SEQ ID NO: 136 - DNA, 25 bp, Artificial
  synthetic sequence
aagcccaatcgucatctttgtagut

SEQ ID NO: 137 - DNA, 33 bp, Artificial
  synthetic sequence
actaataataagggautttctgaatttggugat

SEQ ID NO: 138 - DNA, 29 bp, Artificial
  synthetic sequence
aactttttagtauccttagcgaagtugac

SEQ ID NO: 139 - DNA, 30 bp, Artificial
  synthetic sequence
tgctcaaagugagaacttttcaaatcguaa

SEQ ID NO: 140 - DNA, 28 bp, Artificial
  synthetic sequence
tctgtttgtgaauaactaccgtuaggac

SEQ ID NO: 141 - DNA, 33 bp, Artificial
  synthetic sequence
agcattactacaaaaagaaucaagcaataauaa

SEQ ID NO: 142 - DNA, 33 bp, Artificial
  synthetic sequence
atttagggtguaacaaagatgaaaaacatuaat

SEQ ID NO: 143 - DNA, 27 bp, Artificial
  synthetic sequence
gcacctgctuttataacatcattucca

SEQ ID NO: 144 - DNA, 31 bp, Artificial
  synthetic sequence
acagaagaaaataugtctgctacaaauagat

SEQ ID NO: 145 - DNA, 32 bp, Artificial
  synthetic sequence
gtaatccuactttcatcataugaagaagaact

SEQ ID NO: 146 - DNA, 23 bp, Artificial
  synthetic sequence
ggtgcaacaugaaatcaagguga

SEQ ID NO: 147 - DNA, 26 bp, Artificial
  synthetic sequence
gaaattgcuacagagatagucccacc

SEQ ID NO: 148 - DNA, 32 bp, Artificial
  synthetic sequence
gtaatgctttuaaaaatcattctaaugaccca

SEQ ID NO: 149 - DNA, 29 bp, Artificial
  synthetic sequence
actggcaattcaucagaaaatacatcuac

SEQ ID NO: 150 - DNA, 22 bp, Artificial
  synthetic sequence
ccgtagttuttccttgcugacc

SEQ ID NO: 151 - DNA, 20 bp, Artificial
  synthetic sequence
ggacagcuacccttgtugca

SEQ ID NO: 152 - DNA, 33 bp, Artificial
  synthetic sequence
aaagcacgautaatagttaaatuaccaaaaaca

SEQ ID NO: 153 - DNA, 28 bp, Artificial
  synthetic sequence
cgcttcaactgaucatgtagaaaaagug

SEQ ID NO: 154 - DNA, 26 bp, Artificial
  synthetic sequence
cagcatgactgutatcagtgtttgut

SEQ ID NO: 155 - DNA, 26 bp, Artificial
  synthetic sequence
ggtgttaaggugaattggacucaaac

SEQ ID NO: 156 - DNA, 29 bp, Artificial
  synthetic sequence
cctgtgcccaautcattattagtatucat

SEQ ID NO: 157 - DNA, 18 bp, Artificial
  synthetic sequence
aaaccttugccgggcguc

SEQ ID NO: 158 - DNA, 17 bp, Artificial
  synthetic sequence
cgcaucaggcucccgca

SEQ ID NO: 159 - DNA, 17 bp, Artificial
  synthetic sequence
gcggauaucacggacgc

SEQ ID NO: 160 - DNA, 17 bp, Artificial
  synthetic sequence
ggctgcggutgtggucg

SEQ ID NO: 161 - DNA, 19 bp, Artificial
  synthetic sequence
agguaccggcctgcugcat

SEQ ID NO: 162 - DNA, 17 bp, Artificial
  synthetic sequence
tucgcugcccgaagccg

SEQ ID NO: 163 - DNA, 21 bp, Artificial
  synthetic sequence
agcagaaagacaggcaugaug

SEQ ID NO: 164 - DNA, 18 bp, Artificial
  synthetic sequence
agcaccuactgcaucgcc

SEQ ID NO: 165 - DNA, 19 bp, Artificial
  synthetic sequence
augcagccacaaccaaucg

SEQ ID NO: 166 - DNA, 21 bp, Artificial
  synthetic sequence
ttcggccacautccatccuaa

SEQ ID NO: 167 - DNA, 20 bp, Artificial
  synthetic sequence
tugcugaccaaaaccaccac

SEQ ID NO: 168 - DNA, 26 bp, Artificial
  synthetic sequence
tttttatggaaugtttttctgucggg

SEQ ID NO: 169 - DNA, 26 bp, Artificial
  synthetic sequence
gttcctattccuatctcttccggugg

SEQ ID NO: 170 - DNA, 20 bp, Artificial
  synthetic sequence
ccgccuttgatagauccgct

SEQ ID NO: 171 - DNA, 19 bp, Artificial
  synthetic sequence
agucccaacgccattgugc

SEQ ID NO: 172 - DNA, 26 bp, Artificial
  synthetic sequence
caaggaugtttaugaacggcaaaaca

SEQ ID NO: 173 - DNA, 26 bp, Artificial
  synthetic sequence
gaatatgagccaugagatacguacgc

SEQ ID NO: 174 - DNA, 26 bp, Artificial
  synthetic sequence
agaaagacatgcuaccggattctaug

SEQ ID NO: 175 - DNA, 21 bp, Artificial
  synthetic sequence
gaagctggauttgccgaccua

SEQ ID NO: 176 - DNA, 19 bp, Artificial
  synthetic sequence
gcgggcacaaaacuctuca

SEQ ID NO: 177 - DNA, 20 bp, Artificial
  synthetic sequence
actcaggcgacucagtctug

SEQ ID NO: 178 - DNA, 17 bp, Artificial
  synthetic sequence
ggcggutctggucaagc

SEQ ID NO: 179 - DNA, 19 bp, Artificial
  synthetic sequence
ttcugacgcctaugggaca

SEQ ID NO: 180 - DNA, 17 bp, Artificial
  synthetic sequence
ggtugcggacctgcauc

SEQ ID NO: 181 - DNA, 18 bp, Artificial
  synthetic sequence
cccacgaaugcgaucacg

SEQ ID NO: 182 - DNA, 21 bp, Artificial
  synthetic sequence
cagcaaggccgaugagauaag

SEQ ID NO: 183 - DNA, 26 bp, Artificial
  synthetic sequence
gtgacatcugaggtagatgatauggc

SEQ ID NO: 184 - DNA, 20 bp, Artificial
  synthetic sequence
acucggcacagauacaagca

SEQ ID NO: 185 - DNA, 18 bp, Artificial
  synthetic sequence
agccagauctccacgcuc

SEQ ID NO: 186 - DNA, 31 bp, Artificial
  synthetic sequence
tagggcatatcgauaaaagctgtaauaaaaa

SEQ ID NO: 187 - DNA, 21 bp, Artificial
  synthetic sequence
atgcccuaaaaaucgcaagct

SEQ ID NO: 188 - DNA, 19 bp, Artificial
  synthetic sequence
gauatggcugcaaacgcga

SEQ ID NO: 189 - DNA, 28 bp, Artificial
  synthetic sequence
gccggagtaucaagatttaaaccauaag

SEQ ID NO: 190 - DNA, 32 bp, Artificial
  synthetic sequence
agattgttttattuatttgcaaagagaugacg

SEQ ID NO: 191 - DNA, 27 bp, Artificial
  synthetic sequence
ctttgcaaaautttgcatatucaccga

SEQ ID NO: 192 - DNA, 28 bp, Artificial
  synthetic sequence
gattgatguggctattaaaagtaucggc

SEQ ID NO: 193 - DNA, 21 bp, Artificial
  synthetic sequence
gctgacgcuctcauaaacgga

SEQ ID NO: 194 - DNA, 25 bp, Artificial
  synthetic sequence
ttgcaaagaattutgcgccattaut

SEQ ID NO: 195 - DNA, 33 bp, Artificial
  synthetic sequence
aggtttaaagtatuttctacaaaaactucaaca

SEQ ID NO: 196 - DNA, 19 bp, Artificial
  synthetic sequence
acuccggcagaaagggaut

SEQ ID NO: 197 - DNA, 26 bp, Artificial
  synthetic sequence
catcgataagcucatcatcaugccaa

SEQ ID NO: 198 - DNA, 32 bp, Artificial
  synthetic sequence
taaatttatctcauagtctgagataucgacct

SEQ ID NO: 199 - DNA, 24 bp, Artificial
  synthetic sequence
ataauacgagcagcacaccuaccg

SEQ ID NO: 200 - DNA, 23 bp, Artificial
  synthetic sequence
aaatgaaccggaucaaagcuccc

SEQ ID NO: 201 - DNA, 31 bp, Artificial
  synthetic sequence
agaggagtcutttaaaaagacugaagaagat

SEQ ID NO: 202 - DNA, 24 bp, Artificial
  synthetic sequence
ttgcgucagtgatcucagaaacat

SEQ ID NO: 203 - DNA, 20 bp, Artificial
  synthetic sequence
ggcautctgagguaccggaa

SEQ ID NO: 204 - DNA, 27 bp, Artificial
  synthetic sequence
ttttcgcctcucacattggaaattaut

SEQ ID NO: 205 - DNA, 22 bp, Artificial
  synthetic sequence
tgggcaugaucggagaaagaag

SEQ ID NO: 206 - DNA, 21 bp, Artificial
  synthetic sequence
ttgccauggtattcctuggcg

SEQ ID NO: 207 - DNA, 26 bp, Artificial
  synthetic sequence
ccaattgaacuactgacctgtuggag

SEQ ID NO: 208 - DNA, 18 bp, Artificial
  synthetic sequence
caccgugggtgctggucg

SEQ ID NO: 209 - DNA, 23 bp, Artificial
  synthetic sequence
cgcagtacauggatcacctgtuc

SEQ ID NO: 210 - DNA, 18 bp, Artificial
  synthetic sequence
cgtatgcgaugcgtucgc

SEQ ID NO: 211 - DNA, 17 bp, Artificial
  synthetic sequence
cgcauacgugcagcggt

SEQ ID NO: 212 - DNA, 17 bp, Artificial
  synthetic sequence
ggacaggugcccggugg

SEQ ID NO: 213 - DNA, 20 bp, Artificial
  synthetic sequence
ctgttcugctggttcugcga

SEQ ID NO: 214 - DNA, 19 bp, Artificial
  synthetic sequence
gccgtaguaacagccucga

SEQ ID NO: 215 - DNA, 21 bp, Artificial
  synthetic sequence
actacggcaucatcgttguct

SEQ ID NO: 216 - DNA, 17 bp, Artificial
  synthetic sequence
gtuacgcgcaucgagcc

SEQ ID NO: 217 - DNA, 17 bp, Artificial
  synthetic sequence
gcagccagcccutctug

SEQ ID NO: 218 - DNA, 22 bp, Artificial
  synthetic sequence
ggcagaagauttgatgcuccat

SEQ ID NO: 219 - DNA, 28 bp, Artificial
  synthetic sequence
acagccgctugattatatttaaacugcc

SEQ ID NO: 220 - DNA, 26 bp, Artificial
  synthetic sequence
agaggtattccaaaugcagcttatug

SEQ ID NO: 221 - DNA, 33 bp, Artificial
  synthetic sequence
acgataccagtaauacttattaaactcaucaaa

SEQ ID NO: 222 - DNA, 18 bp, Artificial
  synthetic sequence
tggcugctuggaaacgag

SEQ ID NO: 223 - DNA, 26 bp, Artificial
  synthetic sequence
gctggtattgguatgattccagaugg

SEQ ID NO: 224 - DNA, 21 bp, Artificial
  synthetic sequence
aaaccaaaccgutgccccaua

SEQ ID NO: 225 - DNA, 31 bp, Artificial
  synthetic sequence
tcgactgatataucaagagaaagaaagtgua

SEQ ID NO: 226 - DNA, 23 bp, Artificial
  synthetic sequence
catcagccaugtguacaaaacct

SEQ ID NO: 227 - DNA, 28 bp, Artificial
  synthetic sequence
agaaacggcuataccaattcaugaagag

SEQ ID NO: 228 - DNA, 31 bp, Artificial
  synthetic sequence
cttcgttcgtaauagatggctctacaauaag

SEQ ID NO: 229 - DNA, 19 bp, Artificial
  synthetic sequence
gcggaauggcgttuacagt

SEQ ID NO: 230 - DNA, 33 bp, Artificial
  synthetic sequence
tttagcttatcaauagcacaatttuagaaaaca

SEQ ID NO: 231 - DNA, 17 bp, Artificial
  synthetic sequence
gccacccagccaugaug

SEQ ID NO: 232 - DNA, 18 bp, Artificial
  synthetic sequence
gcgcgguggaggtgtcua

SEQ ID NO: 233 - DNA, 33 bp, Artificial
  synthetic sequence
actatgaataaaauttatttctcucaagacccg

SEQ ID NO: 234 - DNA, 17 bp, Artificial
  synthetic sequence
tggguggcggagcauca

SEQ ID NO: 235 - DNA, 20 bp, Artificial
  synthetic sequence
ctggauacgcagaccgaugt

SEQ ID NO: 236 - DNA, 21 bp, Artificial
  synthetic sequence
cattccgcugtttcatcugca

SEQ ID NO: 237 - DNA, 24 bp, Artificial
  synthetic sequence
atgttgttcaaggugacggtacug

SEQ ID NO: 238 - DNA, 29 bp, Artificial
  synthetic sequence
caaggtttcaaggaacautgaagtgauaa

SEQ ID NO: 239 - DNA, 31 bp, Artificial
  synthetic sequence
caaaacaggagauaagatttttgucacagga

SEQ ID NO: 240 - DNA, 22 bp, Artificial
  synthetic sequence
aaacagtucagcacgttccuga

SEQ ID NO: 241 - DNA, 30 bp, Artificial
  synthetic sequence
cggtgacaccuaaagaactgatgatatuct

SEQ ID NO: 242 - DNA, 32 bp, Artificial
  synthetic sequence
tgacgatatcctutttattcaagtctcuaagg

SEQ ID NO: 243 - DNA, 33 bp, Artificial
  synthetic sequence
taatgaaatccaaauattctctttctttauggc

SEQ ID NO: 244 - DNA, 18 bp, Artificial
  synthetic sequence
aacgagcuagcgaucgca

SEQ ID NO: 245 - DNA, 17 bp, Artificial
  synthetic sequence
tccugcaaucaccggca

SEQ ID NO: 246 - DNA, 20 bp, Artificial
  synthetic sequence
tcacgccgaugaaugaagag

SEQ ID NO: 247 - DNA, 27 bp, Artificial
  synthetic sequence
attctacccatguctctgggatttuga

SEQ ID NO: 248 - DNA, 25 bp, Artificial
  synthetic sequence
agaaaaaccaaaagcaacugguacg

SEQ ID NO: 249 - DNA, 24 bp, Artificial
  synthetic sequence
ggautcatggauaggagaaaggct

SEQ ID NO: 250 - DNA, 21 bp, Artificial
  synthetic sequence
tgccgccuacctaccagtaug

SEQ ID NO: 251 - DNA, 32 bp, Artificial
  synthetic sequence
gtatcctagatatgucatttaggtcttcuaca

SEQ ID NO: 252 - DNA, 28 bp, Artificial
  synthetic sequence
agagattgatgaccugactatagaguct

SEQ ID NO: 253 - DNA, 24 bp, Artificial
  synthetic sequence
ttgaacttgaaucgaccctaugca

SEQ ID NO: 254 - DNA, 29 bp, Artificial
  synthetic sequence
atgaatccaaauagggattctgactaugt

SEQ ID NO: 255 - DNA, 27 bp, Artificial
  synthetic sequence
atctctataucaaagctccuggacaca

SEQ ID NO: 256 - DNA, 31 bp, Artificial
  synthetic sequence
aggtttaggaaggaauttacaactgaaaaua

SEQ ID NO: 257 - DNA, 28 bp, Artificial
  synthetic sequence
tccttgcgacutttgcaaataatatuga

SEQ ID NO: 258 - DNA, 32 bp, Artificial
  synthetic sequence
aaagatcttgattaugaaattcaagagcaaut

SEQ ID NO: 259 - DNA, 30 bp, Artificial
  synthetic sequence
tttttcagctugcaaacgctttattaaaut

SEQ ID NO: 260 - DNA, 31 bp, Artificial
  synthetic sequence
tgaattgcctattuatacacgcaataaatut

SEQ ID NO: 261 - DNA, 32 bp, Artificial
  synthetic sequence
tcggttaatttacugaatgcaaaaaguaaaaa

SEQ ID NO: 262 - DNA, 30 bp, Artificial
  synthetic sequence
aatacaaataatctaucgctttttgggugt

SEQ ID NO: 263 - DNA, 31 bp, Artificial
  synthetic sequence
ttttacattctgttuaccaggatcaatuaca

SEQ ID NO: 264 - DNA, 30 bp, Artificial
  synthetic sequence
gccttcttcaaautctttatagcttttugc

SEQ ID NO: 265 - DNA, 18 bp, Artificial
  synthetic sequence
ttucgcggtguagagccg

SEQ ID NO: 266 - DNA, 17 bp, Artificial
  synthetic sequence
cugcagagccggcccuc

SEQ ID NO: 267 - DNA, 17 bp, Artificial
  synthetic sequence
gcugagccggtcaaugc

SEQ ID NO: 268 - DNA, 19 bp, Artificial
  synthetic sequence
agtguggcaccaaugaacc

SEQ ID NO: 269 - DNA, 20 bp, Artificial
  synthetic sequence
gttccgguaaaagcaggugt

SEQ ID NO: 270 - DNA, 20 bp, Artificial
  synthetic sequence
acccgcuggtcaatttcuct

SEQ ID NO: 271 - DNA, 30 bp, Artificial
  synthetic sequence
caccttacatguaaaaattcttgcgattuc

SEQ ID NO: 272 - DNA, 18 bp, Artificial
  synthetic sequence
ccggaaccccaucccugt

SEQ ID NO: 273 - DNA, 20 bp, Artificial
  synthetic sequence
cttctgcaucccgaaccucc

SEQ ID NO: 274 - DNA, 25 bp, Artificial
  synthetic sequence
tatutcgttggcaauagaagagcca

SEQ ID NO: 275 - DNA, 26 bp, Artificial
  synthetic sequence
cacttttauactgtaccucgaccaca

SEQ ID NO: 276 - DNA, 17 bp, Artificial
  synthetic sequence
gggcguagtcggugagt

SEQ ID NO: 277 - DNA, 22 bp, Artificial
  synthetic sequence
cgacccugacactttttgcaut

SEQ ID NO: 278 - DNA, 28 bp, Artificial
  synthetic sequence
tcatgatgagaacutggagauaaagcct

SEQ ID NO: 279 - DNA, 22 bp, Artificial
  synthetic sequence
ctacgcccacuttaaactgugg

SEQ ID NO: 280 - DNA, 27 bp, Artificial
  synthetic sequence
cagggtcgataucgatatcgataaugt

SEQ ID NO: 281 - DNA, 19 bp, Artificial
  synthetic sequence
tcctugcaggcatucaggt

SEQ ID NO: 282 - DNA, 32 bp, Artificial
  synthetic sequence
actgactataaatugatattgtgtgaugacag

SEQ ID NO: 283 - DNA, 22 bp, Artificial
  synthetic sequence
aagccgaaauctgaaugaccga

SEQ ID NO: 284 - DNA, 23 bp, Artificial
  synthetic sequence
tcgaagaagcacugcatcatguc

SEQ ID NO: 285 - DNA, 22 bp, Artificial
  synthetic sequence
gtgcaggcgauctacaacatuc

SEQ ID NO: 286 - DNA, 25 bp, Artificial
  synthetic sequence
aataautatcagttgcucgcagcct

SEQ ID NO: 287 - DNA, 29 bp, Artificial
  synthetic sequence
ctaaagcttugtctatcttaucaacagct

SEQ ID NO: 288 - DNA, 23 bp, Artificial
  synthetic sequence
ggtaacucagacgagttctcgug

SEQ ID NO: 289 - DNA, 28 bp, Artificial
  synthetic sequence
agatggattgttuatccagttttctgug

SEQ ID NO: 290 - DNA, 33 bp, Artificial
  synthetic sequence
ggaactacactutcttttaatgctttuaaagat

SEQ ID NO: 291 - DNA, 28 bp, Artificial
  synthetic sequence
gcgaataaatatuctactgacgctucat

SEQ ID NO: 292 - DNA, 23 bp, Artificial
  synthetic sequence
tcttgtugccttcagtuccaact

SEQ ID NO: 293 - DNA, 28 bp, Artificial
  synthetic sequence
ccattgttgagucgtcagcttcattuat

SEQ ID NO: 294 - DNA, 27 bp, Artificial
  synthetic sequence
agcttuagcaagagctauaaaccaagt

SEQ ID NO: 295 - DNA, 26 bp, Artificial
  synthetic sequence
gctgagacaautctttttcgaacuca

SEQ ID NO: 296 - DNA, 21 bp, Artificial
  synthetic sequence
gccagaagcgacaguagctua

SEQ ID NO: 297 - DNA, 32 bp, Artificial
  synthetic sequence
tgatatcatcaacautaaacatctcatagucc

SEQ ID NO: 298 - DNA, 27 bp, Artificial
  synthetic sequence
accaagcttttauaagagagttgcuct

SEQ ID NO: 299 - DNA, 28 bp, Artificial
  synthetic sequence
agcttggtaatucagacaaatcaatucg

SEQ ID NO: 300 - DNA, 27 bp, Artificial
  synthetic sequence
gtctcagcaugattatttccatucacg

SEQ ID NO: 301 - DNA, 17 bp, Artificial
  synthetic sequence
cgucgccaagcctucga

SEQ ID NO: 302 - DNA, 18 bp, Artificial
  synthetic sequence
tggttcuggtcgaccugt

SEQ ID NO: 303 - DNA, 18 bp, Artificial
  synthetic sequence
gaccucgctuacccggaa

SEQ ID NO: 304 - DNA, 22 bp, Artificial
  synthetic sequence
acctccugaatcttauccgcga

SEQ ID NO: 305 - DNA, 19 bp, Artificial
  synthetic sequence
cacgguggccgctttaaug

SEQ ID NO: 306 - DNA, 17 bp, Artificial
  synthetic sequence
tggcgacgguactuggc

SEQ ID NO: 307 - DNA, 24 bp, Artificial
  synthetic sequence
catcagcgucaaatcagucaaccg

SEQ ID NO: 308 - DNA, 17 bp, Artificial
  synthetic sequence
gguacgctgtucgccgt

SEQ ID NO: 309 - DNA, 23 bp, Artificial
  synthetic sequence
aggagtagacauccatgaauccg

SEQ ID NO: 310 - DNA, 20 bp, Artificial
  synthetic sequence
ttcgcgucatggcataugct

SEQ ID NO: 311 - DNA, 22 bp, Artificial
  synthetic sequence
ggaactggaugtatcgcgauga

SEQ ID NO: 312 - DNA, 17 bp, Artificial
  synthetic sequence
gucgccaaaugggcgat

SEQ ID NO: 313 - DNA, 19 bp, Artificial
  synthetic sequence
tguaaaaccggcgaggugg

SEQ ID NO: 314 - DNA, 18 bp, Artificial
  synthetic sequence
cgctcaaaugtccucgct

SEQ ID NO: 315 - DNA, 20 bp, Artificial
  synthetic sequence
ttugagcgcacaaguagggt

SEQ ID NO: 316 - DNA, 19 bp, Artificial
  synthetic sequence
ccagtucccagtccaugca

SEQ ID NO: 317 - DNA, 17 bp, Artificial
  synthetic sequence
ccggttuccctggtucg

SEQ ID NO: 318 - DNA, 21 bp, Artificial
  synthetic sequence
ctgaattuacgcgtgagguga

SEQ ID NO: 319 - DNA, 24 bp, Artificial
  synthetic sequence
cgatcactccaaauccggagcaua

SEQ ID NO: 320 - DNA, 18 bp, Artificial
  synthetic sequence
aaccggguggcagccgua

SEQ ID NO: 321 - DNA, 17 bp, Artificial
  synthetic sequence
cggcaccuttcuggcac

SEQ ID NO: 322 - DNA, 17 bp, Artificial
  synthetic sequence
gactguggcttgcugca

SEQ ID NO: 323 - DNA, 19 bp, Artificial
  synthetic sequence
ctgcccgguatttcgcaut

SEQ ID NO: 324 - DNA, 20 bp, Artificial
  synthetic sequence
acgggcacagautatcgugt

SEQ ID NO: 325 - DNA, 28 bp, Artificial
  synthetic sequence
tttggagcaatgautatcggtccatuaa

SEQ ID NO: 326 - DNA, 28 bp, Artificial
  synthetic sequence
ctccaattaagccugcagaaaaatuacg

SEQ ID NO: 327 - DNA, 25 bp, Artificial
  synthetic sequence
attacgguacctggaaaugaaggct

SEQ ID NO: 328 - DNA, 32 bp, Artificial
  synthetic sequence
gatagcacgaccgaucaaataaaaatactaut

SEQ ID NO: 329 - DNA, 24 bp, Artificial
  synthetic sequence
atggttggtauggcagttatuggc

SEQ ID NO: 330 - DNA, 25 bp, Artificial
  synthetic sequence
ttgataatgccutgtaagaaugccc

SEQ ID NO: 331 - DNA, 23 bp, Artificial
  synthetic sequence
ccacaccauttttgcccttucac

SEQ ID NO: 332 - DNA, 17 bp, Artificial
  synthetic sequence
cggctucacccagtucg

SEQ ID NO: 333 - DNA, 18 bp, Artificial
  synthetic sequence
tgaagccggauggctuga

SEQ ID NO: 334 - DNA, 33 bp, Artificial
  synthetic sequence
tcttcaaattttaautcttagatgttgauccac

SEQ ID NO: 335 - DNA, 17 bp, Artificial
  synthetic sequence
cgucccagcugacgcaa

SEQ ID NO: 336 - DNA, 22 bp, Artificial
  synthetic sequence
tcggtaugggattatccgucct

SEQ ID NO: 337 - DNA, 32 bp, Artificial
  synthetic sequence
ctttaaaatcagauccagattttcatgtucca

SEQ ID NO: 338 - DNA, 21 bp, Artificial
  synthetic sequence
tgaagaaaatuccgccgcuga

SEQ ID NO: 339 - DNA, 22 bp, Artificial
  synthetic sequence
gccatagaccgcuctgactucc

SEQ ID NO: 340 - DNA, 22 bp, Artificial
  synthetic sequence
cgcagcucagaccattcatugg

SEQ ID NO: 341 - DNA, 28 bp, Artificial
  synthetic sequence
ttggaagacgucatcctcgatataauga

SEQ ID NO: 342 - DNA, 20 bp, Artificial
  synthetic sequence
tcaaugcaacccttucccag

SEQ ID NO: 343 - DNA, 25 bp, Artificial
  synthetic sequence
agagtgagacaautacgctacctug

SEQ ID NO: 344 - DNA, 33 bp, Artificial
  synthetic sequence
ttgatatttcatttucaaggtgtttaaagugag

SEQ ID NO: 345 - DNA, 31 bp, Artificial
  synthetic sequence
agattctaaagaagugctagatttaagugcg

SEQ ID NO: 346 - DNA, 31 bp, Artificial
  synthetic sequence
ttgatgacatttugagagaatgtcttgcaua

SEQ ID NO: 347 - DNA, 18 bp, Artificial
  synthetic sequence
ggaaugtgcgucgaacgg

SEQ ID NO: 348 - DNA, 18 bp, Artificial
  synthetic sequence
ccagcugcggttgcgaut

SEQ ID NO: 349 - DNA, 21 bp, Artificial
  synthetic sequence
ccgtaccggautccagcguat

SEQ ID NO: 350 - DNA, 31 bp, Artificial
  synthetic sequence
gtctggaatguagaactatgcgatgatauat

SEQ ID NO: 351 - DNA, 18 bp, Artificial
  synthetic sequence
ctctuggcgcgaauggac

SEQ ID NO: 352 - DNA, 18 bp, Artificial
  synthetic sequence
tgggcggcuatctggaug

SEQ ID NO: 353 - DNA, 28 bp, Artificial
  synthetic sequence
aaggacttaugcctcaattaatucaacc

SEQ ID NO: 354 - DNA, 25 bp, Artificial
  synthetic sequence
tctaccgcagauaaaactcccacua

SEQ ID NO: 355 - DNA, 28 bp, Artificial
  synthetic sequence
acctatagtcauatcaactggaatugcg

SEQ ID NO: 356 - DNA, 21 bp, Artificial
  synthetic sequence
aagtcctugcatccacttugg

SEQ ID NO: 357 - DNA, 28 bp, Artificial
  synthetic sequence
tactggagatgtautagtgggagaagut

SEQ ID NO: 358 - DNA, 32 bp, Artificial
  synthetic sequence
ttgcataataatttguaaggtttttcatccuc

SEQ ID NO: 359 - DNA, 17 bp, Artificial
  synthetic sequence
cgutccaucccacccct

SEQ ID NO: 360 - DNA, 24 bp, Artificial
  synthetic sequence
gcatccagaaugcttttctuaccg

SEQ ID NO: 361 - DNA, 21 bp, Artificial
  synthetic sequence
tccccaaucttccgtauagcg

SEQ ID NO: 362 - DNA, 21 bp, Artificial
  synthetic sequence
atcagcgaaaugccgtucaaa

SEQ ID NO: 363 - DNA, 22 bp, Artificial
  synthetic sequence
aaagaccgccgutgcggtttua

SEQ ID NO: 364 - DNA, 17 bp, Artificial
  synthetic sequence
auggaacggcccaugca

SEQ ID NO: 365 - DNA, 21 bp, Artificial
  synthetic sequence
atgcatcugtttccuggccat

SEQ ID NO: 366 - DNA, 25 bp, Artificial
  synthetic sequence
ttttgcaatcugaatgtgatcuggg

SEQ ID NO: 367 - DNA, 24 bp, Artificial
  synthetic sequence
aaacagatcacguccaaggtcauc

SEQ ID NO: 368 - DNA, 17 bp, Artificial
  synthetic sequence
gggccgaugcauggaga

SEQ ID NO: 369 - DNA, 18 bp, Artificial
  synthetic sequence
aucggcccagtauccgat

SEQ ID NO: 370 - DNA, 23 bp, Artificial
  synthetic sequence
atccgggutgatuaggaggaaga

SEQ ID NO: 371 - DNA, 31 bp, Artificial
  synthetic sequence
ttgcaaaataacatutgtaatcccaattucc

SEQ ID NO: 372 - DNA, 19 bp, Artificial
  synthetic sequence
aagagggcagaguaugccg

SEQ ID NO: 373 - DNA, 23 bp, Artificial
  synthetic sequence
atgccctggautatcccaaugaa

SEQ ID NO: 374 - DNA, 26 bp, Artificial
  synthetic sequence
ttcaatgcctcauaatgcatctgauc

SEQ ID NO: 375 - DNA, 23 bp, Artificial
  synthetic sequence
tcaacagctugagtagtctcguc

SEQ ID NO: 376 - DNA, 22 bp, Artificial
  synthetic sequence
ttctgcaguaactgcaggguac

SEQ ID NO: 377 - DNA, 23 bp, Artificial
  synthetic sequence
acggaatgtttuccgcaatcgut

SEQ ID NO: 378 - DNA, 21 bp, Artificial
  synthetic sequence
cagggcauaagaggcauaagc

SEQ ID NO: 379 - DNA, 18 bp, Artificial
  synthetic sequence
tgcagcaucacctgcuga

SEQ ID NO: 380 - DNA, 17 bp, Artificial
  synthetic sequence
gctgtugaagggcucgg

SEQ ID NO: 381 - DNA, 30 bp, Artificial
  synthetic sequence
gcttattacgcacaauagcgaatuaaaaca

SEQ ID NO: 382 - DNA, 30 bp, Artificial
  synthetic sequence
aatagttttguaataacaagaugcaaccag

SEQ ID NO: 383 - DNA, 26 bp, Artificial
  synthetic sequence
aaccgaagaaggagagutaaagacut

SEQ ID NO: 384 - DNA, 26 bp, Artificial
  synthetic sequence
cggtagtgguggtgttatcgtuaaat

SEQ ID NO: 385 - DNA, 27 bp, Artificial
  synthetic sequence
caggttgagggccauctaaataatuca

SEQ ID NO: 386 - DNA, 33 bp, Artificial
  synthetic sequence
attgacaaaatcauagttaaaaactccttugaa

SEQ ID NO: 387 - DNA, 24 bp, Artificial
  synthetic sequence
tttactaccaucgcgccgatatut

SEQ ID NO: 388 - DNA, 17 bp, Artificial
  synthetic sequence
atcgccgcguttugcgt

SEQ ID NO: 389 - DNA, 19 bp, Artificial
  synthetic sequence
aaacggcucatctgcguca

SEQ ID NO: 390 - DNA, 23 bp, Artificial
  synthetic sequence
gutgcaccguaaaagagaggact

SEQ ID NO: 391 - DNA, 27 bp, Artificial
  synthetic sequence
aacctagccatacuagtatagtcccut

SEQ ID NO: 392 - DNA, 26 bp, Artificial
  synthetic sequence
gagttgguatcaggagaugaagaagc

SEQ ID NO: 393 - DNA, 27 bp, Artificial
  synthetic sequence
ctgcaaacacaucaaaauaaaaggcag

SEQ ID NO: 394 - DNA, 31 bp, Artificial
  synthetic sequence
tgccaaaaataagauacaccttcctauaaga

SEQ ID NO: 395 - DNA, 26 bp, Artificial
  synthetic sequence
accaactctauatcggcaaaattugt

SEQ ID NO: 396 - DNA, 19 bp, Artificial
  synthetic sequence
acctgagggugacgactug

SEQ ID NO: 397 - DNA, 25 bp, Artificial
  synthetic sequence
tgtccctcaaccuaatttttggcut

SEQ ID NO: 398 - DNA, 23 bp, Artificial
  synthetic sequence
gtttgcagauaggtgtucaagca

SEQ ID NO: 399 - DNA, 23 bp, Artificial
  synthetic sequence
guttggcucaggaagagaaacct

SEQ ID NO: 400 - DNA, 27 bp, Artificial
  synthetic sequence
gatacuaccatcgcuagaaacacagaa

SEQ ID NO: 401 - DNA, 23 bp, Artificial
  synthetic sequence
gcaaaggcagagguggacatuac

SEQ ID NO: 402 - DNA, 20 bp, Artificial
  synthetic sequence
tcaaacgaacagccugtucc

SEQ ID NO: 403 - DNA, 22 bp, Artificial
  synthetic sequence
tcgttugacgaataacaugccg

SEQ ID NO: 404 - DNA, 28 bp, Artificial
  synthetic sequence
agagcctatcauagaagacatcaauagc

SEQ ID NO: 405 - DNA, 22 bp, Artificial
  synthetic sequence
agcacctaccutctggatgauc

SEQ ID NO: 406 - DNA, 18 bp, Artificial
  synthetic sequence
agcagcacaggucctgut

SEQ ID NO: 407 - DNA, 27 bp, Artificial
  synthetic sequence
ggatagcatggugcatgttacagauat

SEQ ID NO: 408 - DNA, 21 bp, Artificial
  synthetic sequence
gtuccacaagagagaugggca

SEQ ID NO: 409 - DNA, 21 bp, Artificial
  synthetic sequence
tttgggcaguaacctcuaggg

SEQ ID NO: 410 - DNA, 25 bp, Artificial
  synthetic sequence
tgcccuagaagccatttaugacaaa

SEQ ID NO: 411 - DNA, 24 bp, Artificial
  synthetic sequence
actgataugcacgccatagaucac

SEQ ID NO: 412 - DNA, 25 bp, Artificial
  synthetic sequence
ccaaagcatuttaaccgaaaauggt

SEQ ID NO: 413 - DNA, 17 bp, Artificial
  synthetic sequence
ggcgutgauaccccagc

SEQ ID NO: 414 - DNA, 32 bp, Artificial
  synthetic sequence
ttgtcagtctatautgtgagatgtttcucaaa

SEQ ID NO: 415 - DNA, 23 bp, Artificial
  synthetic sequence
tggtccaacagcugtttctacut

SEQ ID NO: 416 - DNA, 32 bp, Artificial
  synthetic sequence
atgaagcaaaagaaaaautatuagcacaacaa

SEQ ID NO: 417 - DNA, 26 bp, Artificial
  synthetic sequence
tttttgaggcuaactttgccattuct

SEQ ID NO: 418 - DNA, 21 bp, Artificial
  synthetic sequence
tcaacgccutctggtatuccc

SEQ ID NO: 419 - DNA, 27 bp, Artificial
  synthetic sequence
agattcggaccaaguttaactctucaa

SEQ ID NO: 420 - DNA, 25 bp, Artificial
  synthetic sequence
acctttagggaaguacggtatugaa

SEQ ID NO: 421 - DNA, 23 bp, Artificial
  synthetic sequence
accaagactgcugacagcataug

SEQ ID NO: 422 - DNA, 19 bp, Artificial
  synthetic sequence
tgcaggcacguatatuggc

SEQ ID NO: 423 - DNA, 19 bp, Artificial
  synthetic sequence
tgccugcattgtgauggag

SEQ ID NO: 424 - DNA, 22 bp, Artificial
  synthetic sequence
agacgacgugtccaactaucag

SEQ ID NO: 425 - DNA, 28 bp, Artificial
  synthetic sequence
cgaagcaattcaauaaaacacgaaagug

SEQ ID NO: 426 - DNA, 23 bp, Artificial
  synthetic sequence
agttgcguattatccagtugcga

SEQ ID NO: 427 - DNA, 28 bp, Artificial
  synthetic sequence
cgatgaatacuaagctcatactctucgg

SEQ ID NO: 428 - DNA, 30 bp, Artificial
  synthetic sequence
ttgcttcgaaguaagcgatatattgtttut

SEQ ID NO: 429 - DNA, 23 bp, Artificial
  synthetic sequence
aaaautgcgaccucccgaaaaat

SEQ ID NO: 430 - DNA, 32 bp, Artificial
  synthetic sequence
aattttctcacggauactcacattaattucgt

SEQ ID NO: 431 - DNA, 26 bp, Artificial
  synthetic sequence
accgataatuacaccaaacaacaugg

SEQ ID NO: 432 - DNA, 19 bp, Artificial
  synthetic sequence
cgtcgaucaacagtgcgut

SEQ ID NO: 433 - DNA, 24 bp, Artificial
  synthetic sequence
ccgatcacauaagccacaccuaac

SEQ ID NO: 434 - DNA, 28 bp, Artificial
  synthetic sequence
gtgagtcaaataucattgatgtgaucgt

SEQ ID NO: 435 - DNA, 18 bp, Artificial
  synthetic sequence
tcatcuggagcgacguga

SEQ ID NO: 436 - DNA, 25 bp, Artificial
  synthetic sequence
gaacugaccaacaaagatcaaugga

SEQ ID NO: 437 - DNA, 23 bp, Artificial
  synthetic sequence
atccgtgccutaagtagttugct

SEQ ID NO: 438 - DNA, 32 bp, Artificial
  synthetic sequence
caaggaaggtauaaatgatacacattauccca

SEQ ID NO: 439 - DNA, 22 bp, Artificial
  synthetic sequence
ccttgatgcutggcttgatgut

SEQ ID NO: 440 - DNA, 25 bp, Artificial
  synthetic sequence
ggcaaaataagcucctaaaacaucg

SEQ ID NO: 441 - DNA, 24 bp, Artificial
  synthetic sequence
tcctaccguaaagctctgtgtuac

SEQ ID NO: 442 - DNA, 30 bp, Artificial
  synthetic sequence
tttattaggtttgauttttcagaccugcct

SEQ ID NO: 443 - DNA, 33 bp, Artificial
  synthetic sequence
aggtattttctctaucctcttcccttuaaaacc

SEQ ID NO: 444 - DNA, 28 bp, Artificial
  synthetic sequence
gcaggcactuttaatattcaatgtuccg

SEQ ID NO: 445 - DNA, 20 bp, Artificial
  synthetic sequence
gaaagggucaacatugccgt

SEQ ID NO: 446 - DNA, 17 bp, Artificial
  synthetic sequence
gcgaucgccgtcgugac

SEQ ID NO: 447 - DNA, 21 bp, Artificial
  synthetic sequence
gaaggtgccgaucgagaagug

SEQ ID NO: 448 - DNA, 20 bp, Artificial
  synthetic sequence
accctutcaggatuggcaca

SEQ ID NO: 449 - DNA, 17 bp, Artificial
  synthetic sequence
ataaccggcgcggucut

SEQ ID NO: 450 - DNA, 18 bp, Artificial
  synthetic sequence
accuccgugacagaggga

SEQ ID NO: 451 - DNA, 23 bp, Artificial
  synthetic sequence
cgatcatcacguttgaggcttug

SEQ ID NO: 452 - DNA, 23 bp, Artificial
  synthetic sequence
tatgaatctuagcgcacgcaauc

SEQ ID NO: 453 - DNA, 25 bp, Artificial
  synthetic sequence
gactcagatttucaacccctgtcug

SEQ ID NO: 454 - DNA, 32 bp, Artificial
  synthetic sequence
tgctttatacgcauaaaaataagcttaatuca

SEQ ID NO: 455 - DNA, 20 bp, Artificial
  synthetic sequence
atacuccagggcactugccg

SEQ ID NO: 456 - DNA, 29 bp, Artificial
  synthetic sequence
tttacccttgggcautaccgtatatacua

SEQ ID NO: 457 - DNA, 28 bp, Artificial
  synthetic sequence
autaaggttgtugaagaaagcagaagaa

SEQ ID NO: 458 - DNA, 24 bp, Artificial
  synthetic sequence
aataccgccucacttactauagcc

SEQ ID NO: 459 - DNA, 24 bp, Artificial
  synthetic sequence
ttgtcgggacutcttgattaugca

SEQ ID NO: 460 - DNA, 25 bp, Artificial
  synthetic sequence
tcggtaucgcagctgaatttauagt

SEQ ID NO: 461 - DNA, 22 bp, Artificial
  synthetic sequence
cugacagggacagaaaguaacg

SEQ ID NO: 462 - DNA, 21 bp, Artificial
  synthetic sequence
tgcaacggcuttgtacucact

SEQ ID NO: 463 - DNA, 18 bp, Artificial
  synthetic sequence
ccgatcgutccgcttuca

SEQ ID NO: 464 - DNA, 21 bp, Artificial
  synthetic sequence
gtaactaucagcggcgguact

SEQ ID NO: 465 - DNA, 31 bp, Artificial
  synthetic sequence
acatcgatgttttugatggctttaatatugc

SEQ ID NO: 466 - DNA, 17 bp, Artificial
  synthetic sequence
acgaucggcggcgauat

SEQ ID NO: 467 - DNA, 32 bp, Artificial
  synthetic sequence
gaaaagccattttauattctcctgttctttut

SEQ ID NO: 468 - DNA, 29 bp, Artificial
  synthetic sequence
ctgaaaaagattggugacatcacagauat

SEQ ID NO: 469 - DNA, 19 bp, Artificial
  synthetic sequence
gcacugcgccagataggua

SEQ ID NO: 470 - DNA, 17 bp, Artificial
  synthetic sequence
ggcucggttuccgcgat

SEQ ID NO: 471 - DNA, 20 bp, Artificial
  synthetic sequence
tgtaagaccugcgcgttgug

SEQ ID NO: 472 - DNA, 19 bp, Artificial
  synthetic sequence
gcgatagccugacccagut

SEQ ID NO: 473 - DNA, 21 bp, Artificial
  synthetic sequence
gcaaaacccuctcttgctugt

SEQ ID NO: 474 - DNA, 23 bp, Artificial
  synthetic sequence
tggtggccutgataagagttuga

SEQ ID NO: 475 - DNA, 26 bp, Artificial
  synthetic sequence
gctgctcttccugtcaggtatttuag

SEQ ID NO: 476 - DNA, 20 bp, Artificial
  synthetic sequence
ggtttugcaacaagggctuc

SEQ ID NO: 477 - DNA, 17 bp, Artificial
  synthetic sequence
gcagggcuggcgaucaa

SEQ ID NO: 478 - DNA, 26 bp, Artificial
  synthetic sequence
atgggtttuaaacgcttgaaaaaugc

SEQ ID NO: 479 - DNA, 19 bp, Artificial
  synthetic sequence
gccaaggccuctcttcuca

SEQ ID NO: 480 - DNA, 18 bp, Artificial
  synthetic sequence
agcccugcccctaatugg

SEQ ID NO: 481 - DNA, 19 bp, Artificial
  synthetic sequence
agcaggccutttcucagga

SEQ ID NO: 482 - DNA, 22 bp, Artificial
  synthetic sequence
ggagcaacutgttagcagaugg

SEQ ID NO: 483 - DNA, 19 bp, Artificial
  synthetic sequence
agtugcaggtttugcgagt

SEQ ID NO: 484 - DNA, 26 bp, Artificial
  synthetic sequence
tgccaaaaagccutgagaatattcug

SEQ ID NO: 485 - DNA, 27 bp, Artificial
  synthetic sequence
ttgacgaatcuatttaaacctuaccgc

SEQ ID NO: 486 - DNA, 25 bp, Artificial
  synthetic sequence
ggcctgcuactaattcacttatugc

SEQ ID NO: 487 - DNA, 18 bp, Artificial
  synthetic sequence
acggtggucgctgtacug

SEQ ID NO: 488 - DNA, 17 bp, Artificial
  synthetic sequence
gcagggugcugaccgag

SEQ ID NO: 489 - DNA, 20 bp, Artificial
  synthetic sequence
tcagcgcgcagagaauacug

SEQ ID NO: 490 - DNA, 17 bp, Artificial
  synthetic sequence
accaccguaaccggcuc

SEQ ID NO: 491 - DNA, 17 bp, Artificial
  synthetic sequence
cacccugcgggctguct

SEQ ID NO: 492 - DNA, 20 bp, Artificial
  synthetic sequence
ggattacgcaucggaucggg

SEQ ID NO: 493 - DNA, 21 bp, Artificial
  synthetic sequence
tgcaatcutgtgaguggcaga

SEQ ID NO: 494 - DNA, 19 bp, Artificial
  synthetic sequence
cucgaccaccacgaaucgc

SEQ ID NO: 495 - DNA, 23 bp, Artificial
  synthetic sequence
caatcttcggcgutttgctguat

SEQ ID NO: 496 - DNA, 24 bp, Artificial
  synthetic sequence
gttgaagaugacatgagcgtugac

SEQ ID NO: 497 - DNA, 18 bp, Artificial
  synthetic sequence
cgccagcgaaggcuatut

SEQ ID NO: 498 - DNA, 21 bp, Artificial
  synthetic sequence
gtggtggaugttcctctggug

SEQ ID NO: 499 - DNA, 24 bp, Artificial
  synthetic sequence
cgtagccaaaacuaatccggatug

SEQ ID NO: 500 - DNA, 28 bp, Artificial
  synthetic sequence
catttggactuaagaggtattgcgatut

SEQ ID NO: 501 - DNA, 26 bp, Artificial
  synthetic sequence
gcattaagagcaaaucactgggaaut

SEQ ID NO: 502 - DNA, 30 bp, Artificial
  synthetic sequence
acgattautttaaaagcgtuagaagaagcc

SEQ ID NO: 503 - DNA, 24 bp, Artificial
  synthetic sequence
gttgttgtaaaugccatgggtucc

SEQ ID NO: 504 - DNA, 28 bp, Artificial
  synthetic sequence
tctgaagtacuagttgcagtgatucaac

SEQ ID NO: 505 - DNA, 30 bp, Artificial
  synthetic sequence
cttaaagaaagtcauaatcctcacctuccc

SEQ ID NO: 506 - DNA, 24 bp, Artificial
  synthetic sequence
gcgtttggguttatgagctugaaa

SEQ ID NO: 507 - DNA, 33 bp, Artificial
  synthetic sequence
ataaagaagcatatggugaaaaataaaactcug

SEQ ID NO: 508 - DNA, 19 bp, Artificial
  synthetic sequence
ggcattugcgcccatacug

SEQ ID NO: 509 - DNA, 21 bp, Artificial
  synthetic sequence
gtcgaguacgactugcgagaa

SEQ ID NO: 510 - DNA, 32 bp, Artificial
  synthetic sequence
gagtcacctatauaagcatcactctauaagat

SEQ ID NO: 511 - DNA, 19 bp, Artificial
  synthetic sequence
tcgtcggutctggccuact

SEQ ID NO: 512 - DNA, 25 bp, Artificial
  synthetic sequence
gagaagcgacgacaugattaacuct

SEQ ID NO: 513 - DNA, 18 bp, Artificial
  synthetic sequence
cgccacggcaauggttuc

SEQ ID NO: 514 - DNA, 21 bp, Artificial
  synthetic sequence
gcgcaaacguggttaatggua

SEQ ID NO: 515 - DNA, 19 bp, Artificial
  synthetic sequence
cgutatgucgggcgaacca

SEQ ID NO: 516 - DNA, 26 bp, Artificial
  synthetic sequence
gcaatcauggaaaacatcaacgucat

SEQ ID NO: 517 - DNA, 21 bp, Artificial
  synthetic sequence
cttcaccgccauttccguaac

SEQ ID NO: 518 - DNA, 21 bp, Artificial
  synthetic sequence
ccacaccgutagcagcaauca

SEQ ID NO: 519 - DNA, 19 bp, Artificial
  synthetic sequence
gacccauccggctgauacc

SEQ ID NO: 520 - DNA, 21 bp, Artificial
  synthetic sequence
ccgtgcucggcaatttuacat

SEQ ID NO: 521 - DNA, 17 bp, Artificial
  synthetic sequence
cgcatuggtgagcuggc

SEQ ID NO: 522 - DNA, 18 bp, Artificial
  synthetic sequence
gacagcaacucgcggauc

SEQ ID NO: 523 - DNA, 22 bp, Artificial
  synthetic sequence
tccguatcgatccugaacacca

SEQ ID NO: 524 - DNA, 17 bp, Artificial
  synthetic sequence
gccacucgccccttgut

SEQ ID NO: 525 - DNA, 18 bp, Artificial
  synthetic sequence
guacccaacgggccgtut

SEQ ID NO: 526 - DNA, 17 bp, Artificial
  synthetic sequence
cagauggugcccagacg

SEQ ID NO: 527 - DNA, 17 bp, Artificial
  synthetic sequence
gccucgcgcgagggaut

SEQ ID NO: 528 - DNA, 18 bp, Artificial
  synthetic sequence
accutggucgaggccgct

SEQ ID NO: 529 - DNA, 26 bp, Artificial
  synthetic sequence
acaagaaaggagcgauaactttggut

SEQ ID NO: 530 - DNA, 31 bp, Artificial
  synthetic sequence
ctcatcaatattuaaagctctttgtucagct

SEQ ID NO: 531 - DNA, 31 bp, Artificial
  synthetic sequence
tggatattaaaaguaaaactagctgatgugg

SEQ ID NO: 532 - DNA, 27 bp, Artificial
  synthetic sequence
atcatgttatcccucccaatttgtuct

SEQ ID NO: 533 - DNA, 32 bp, Artificial
  synthetic sequence
ttgatgagataucaacggaaataactagtaug

SEQ ID NO: 534 - DNA, 30 bp, Artificial
  synthetic sequence
aatttctcacccuagtaaatactgtttcuc

SEQ ID NO: 535 - DNA, 24 bp, Artificial
  synthetic sequence
gctccttgaguataaccattgguc

SEQ ID NO: 536 - DNA, 24 bp, Artificial
  synthetic sequence
tcagaugaaacaaaagcggcttuc

SEQ ID NO: 537 - DNA, 33 bp, Artificial
  synthetic sequence
gaaattcacttcaucaattataccauaaaccat

SEQ ID NO: 538 - DNA, 21 bp, Artificial
  synthetic sequence
gctgttgcaacugctttguca

SEQ ID NO: 539 - DNA, 27 bp, Artificial
  synthetic sequence
tctaaggcaautgcttttatcatuggg

SEQ ID NO: 540 - DNA, 33 bp, Artificial
  synthetic sequence
tttctgaaattcucttttatgtcatttuaggac

SEQ ID NO: 541 - DNA, 28 bp, Artificial
  synthetic sequence
gaattctacaaccaucttcaccactuca

SEQ ID NO: 542 - DNA, 26 bp, Artificial
  synthetic sequence
attcgctgatutttcaggtattugct

SEQ ID NO: 543 - DNA, 18 bp, Artificial
  synthetic sequence
cgccuatgtucaggcagc

SEQ ID NO: 544 - DNA, 18 bp, Artificial
  synthetic sequence
cgtcacucgatuccccgt

SEQ ID NO: 545 - DNA, 22 bp, Artificial
  synthetic sequence
gagugacggaatctttuacccc

SEQ ID NO: 546 - DNA, 19 bp, Artificial
  synthetic sequence
gagcctcugggttctgcug

SEQ ID NO: 547 - DNA, 32 bp, Artificial
  synthetic sequence
caaaaccaattaaagagutagagcaacataug

SEQ ID NO: 548 - DNA, 31 bp, Artificial
  synthetic sequence
aaatgtggattaauttgactgtaaagugcat

SEQ ID NO: 549 - DNA, 31 bp, Artificial
  synthetic sequence
tcctatcaagaatacucattggacattgaut

SEQ ID NO: 550 - DNA, 30 bp, Artificial
  synthetic sequence
tggttttgtaatucttctcaatacacugat

SEQ ID NO: 551 - DNA, 23 bp, Artificial
  synthetic sequence
caaccttuagcctcgccauagaa

SEQ ID NO: 552 - DNA, 29 bp, Artificial
  synthetic sequence
acctttgaaaauacaacagaggtgauaaa

SEQ ID NO: 553 - DNA, 18 bp, Artificial
  synthetic sequence
gagucgacaaccgtcugc

SEQ ID NO: 554 - DNA, 29 bp, Artificial
  synthetic sequence
cgagtatctgcugaaatgagtgatauaac

SEQ ID NO: 555 - DNA, 18 bp, Artificial
  synthetic sequence
agcuaaggcgcctugcaa

SEQ ID NO: 556 - DNA, 25 bp, Artificial
  synthetic sequence
gtcttcaccuttagaatccaucgct

SEQ ID NO: 557 - DNA, 31 bp, Artificial
  synthetic sequence
tgcaaagctaagcaauttagtcaagctttua

SEQ ID NO: 558 - DNA, 26 bp, Artificial
  synthetic sequence
gcaatgttgauactttgtctucacct

SEQ ID NO: 559 - DNA, 31 bp, Artificial
  synthetic sequence
ttcaaaaacatatcutctagatcttctuggt

SEQ ID NO: 560 - DNA, 28 bp, Artificial
  synthetic sequence
atggccaccauaattttgctttuaaagg

SEQ ID NO: 561 - DNA, 17 bp, Artificial
  synthetic sequence
gcccuccgcatcgcugt

SEQ ID NO: 562 - DNA, 21 bp, Artificial
  synthetic sequence
acgtauaccaggcucaaggct

SEQ ID NO: 563 - DNA, 17 bp, Artificial
  synthetic sequence
tcgcccaggugctcucc

SEQ ID NO: 564 - DNA, 17 bp, Artificial
  synthetic sequence
gggutgguggaacgcga

SEQ ID NO: 565 - DNA, 18 bp, Artificial
  synthetic sequence
gccgcagccgaacuggut

SEQ ID NO: 566 - DNA, 17 bp, Artificial
  synthetic sequence
accgcgaacucgggugg

SEQ ID NO: 567 - DNA, 17 bp, Artificial
  synthetic sequence
tucgcggucgacaccaa

SEQ ID NO: 568 - DNA, 21 bp, Artificial
  synthetic sequence
gagttgaggugctgaucaacg

SEQ ID NO: 569 - DNA, 23 bp, Artificial
  synthetic sequence
gtgagcgaaucaagaaagtucgt

SEQ ID NO: 570 - DNA, 26 bp, Artificial
  synthetic sequence
agaagctagtguatacactgcttguc

SEQ ID NO: 571 - DNA, 26 bp, Artificial
  synthetic sequence
tatagttggcguggagcaaaaatuga

SEQ ID NO: 572 - DNA, 32 bp, Artificial
  synthetic sequence
attttaatatttuccccagtatctttagugca

SEQ ID NO: 573 - DNA, 28 bp, Artificial
  synthetic sequence
aaggtctaaatttugtccatctagcaug

SEQ ID NO: 574 - DNA, 26 bp, Artificial
  synthetic sequence
tgctttcucaaaaaggatcucaaggt

SEQ ID NO: 575 - DNA, 28 bp, Artificial
  synthetic sequence
aaaacgaaaacgaaaaagaugaaggtut

SEQ ID NO: 576 - DNA, 28 bp, Artificial
  synthetic sequence
tctctcauaaaaacgcataccacuaagt

SEQ ID NO: 577 - DNA, 29 bp, Artificial
  synthetic sequence
agaaagcaucaaaaccaataaaggaucag

SEQ ID NO: 578 - DNA, 28 bp, Artificial
  synthetic sequence
tgctataaaagauggagaacgctauagt

SEQ ID NO: 579 - DNA, 32 bp, Artificial
  synthetic sequence
aataaggttttgautgcaaaattcttuaggaa

SEQ ID NO: 580 - DNA, 23 bp, Artificial
  synthetic sequence
ccactttagacauaggtgguggt

SEQ ID NO: 581 - DNA, 19 bp, Artificial
  synthetic sequence
agccgcaaaugaauacggc

SEQ ID NO: 582 - DNA, 19 bp, Artificial
  synthetic sequence
ccatggagcuggttggtug

SEQ ID NO: 583 - DNA, 25 bp, Artificial
  synthetic sequence
ggtataaatggaucgtacgttucga

SEQ ID NO: 584 - DNA, 22 bp, Artificial
  synthetic sequence
tccgccaacaaaaccuatguct

SEQ ID NO: 585 - DNA, 20 bp, Artificial
  synthetic sequence
ggcaaccacutccggaatut

SEQ ID NO: 586 - DNA, 17 bp, Artificial
  synthetic sequence
ttgcggcuggaugaggt

SEQ ID NO: 587 - DNA, 29 bp, Artificial
  synthetic sequence
gggatggacaautattttatggattcuga

SEQ ID NO: 588 - DNA, 17 bp, Artificial
  synthetic sequence
cuggccaguaacggcga

SEQ ID NO: 589 - DNA, 24 bp, Artificial
  synthetic sequence
agtattttggcucaccaagcauca

SEQ ID NO: 590 - DNA, 21 bp, Artificial
  synthetic sequence
tgccattgauccacctcacut

SEQ ID NO: 591 - DNA, 32 bp, Artificial
  synthetic sequence
attatgattattgguggaggatggtatacugt

SEQ ID NO: 592 - DNA, 21 bp, Artificial
  synthetic sequence
aatuacgccaacguacccacc

SEQ ID NO: 593 - DNA, 20 bp, Artificial
  synthetic sequence
ctggccaguatttuggcggt

SEQ ID NO: 594 - DNA, 26 bp, Artificial
  synthetic sequence
acagttgaggcugagagaaaacttug

SEQ ID NO: 595 - DNA, 18 bp, Artificial
  synthetic sequence
gccaauccccgtcauagc

SEQ ID NO: 596 - DNA, 19 bp, Artificial
  synthetic sequence
gatccggcggcugatatuc

SEQ ID NO: 597 - DNA, 18 bp, Artificial
  synthetic sequence
ccggttttugcgcgctuc

SEQ ID NO: 598 - DNA, 17 bp, Artificial
  synthetic sequence
gcgauggcagaagcgut

SEQ ID NO: 599 - DNA, 25 bp, Artificial
  synthetic sequence
aaaccttgaugattgctttuggcaa

SEQ ID NO: 600 - DNA, 18 bp, Artificial
  synthetic sequence
agacccguaaugccgcct

SEQ ID NO: 601 - DNA, 17 bp, Artificial
  synthetic sequence
gccaucgctctuggcgt

SEQ ID NO: 602 - DNA, 28 bp, Artificial
  synthetic sequence
actttggtttgaaucaagacttgaucac

SEQ ID NO: 603 - DNA, 20 bp, Artificial
  synthetic sequence
gtgatcgucatgtgcgaucc

SEQ ID NO: 604 - DNA, 30 bp, Artificial
  synthetic sequence
aaggatggaucaaccgttatccttaauaaa

SEQ ID NO: 605 - DNA, 23 bp, Artificial
  synthetic sequence
gctggtucaggtattacaacugc

SEQ ID NO: 606 - DNA, 29 bp, Artificial
  synthetic sequence
gcgattacgattugaaaagttctcactut

SEQ ID NO: 607 - DNA, 23 bp, Artificial
  synthetic sequence
ttattgcaggguatgguagccag

SEQ ID NO: 608 - DNA, 20 bp, Artificial
  synthetic sequence
ctccaccuagtccctguccg

SEQ ID NO: 609 - DNA, 20 bp, Artificial
  synthetic sequence
aaatcacccugguggagcga

SEQ ID NO: 610 - DNA, 23 bp, Artificial
  synthetic sequence
cuactgccttctuccgggaaaat

SEQ ID NO: 611 - DNA, 24 bp, Artificial
  synthetic sequence
taatgacgagaugcgttuggacag

SEQ ID NO: 612 - DNA, 33 bp, Artificial
  synthetic sequence
ctgaattaaattuagtgcattttcuagcaaagc

SEQ ID NO: 613 - DNA, 24 bp, Artificial
  synthetic sequence
cggtttaaacgaugctactcucga

SEQ ID NO: 614 - DNA, 29 bp, Artificial
  synthetic sequence
tttcagcauaccaaagtggatattuccat

SEQ ID NO: 615 - DNA, 17 bp, Artificial
  synthetic sequence
gcagcgaaaguccgucg

SEQ ID NO: 616 - DNA, 17 bp, Artificial
  synthetic sequence
atatccgcgcugcgcug

SEQ ID NO: 617 - DNA, 17 bp, Artificial
  synthetic sequence
ctgatgcgugccgugcc

SEQ ID NO: 618 - DNA, 18 bp, Artificial
  synthetic sequence
agaacagcgcaugcgcuc

SEQ ID NO: 619 - DNA, 24 bp, Artificial
  synthetic sequence
caaaccacttgutcaacttcccug

SEQ ID NO: 620 - DNA, 21 bp, Artificial
  synthetic sequence
gtcagcaaugtaaccgucagg

SEQ ID NO: 621 - DNA, 19 bp, Artificial
  synthetic sequence
aggcaugagcaugaaacgc

SEQ ID NO: 622 - DNA, 19 bp, Artificial
  synthetic sequence
ggtggaacugaccguaggc

SEQ ID NO: 623 - DNA, 18 bp, Artificial
  synthetic sequence
ttuggccacagcauggga

SEQ ID NO: 624 - DNA, 26 bp, Artificial
  synthetic sequence
aaaatgcttctugttccagttcaucc

SEQ ID NO: 625 - DNA, 18 bp, Artificial
  synthetic sequence
cccggucgtgtttauggg

SEQ ID NO: 626 - DNA, 18 bp, Artificial
  synthetic sequence
tctgcgcautcatguccg

SEQ ID NO: 627 - DNA, 17 bp, Artificial
  synthetic sequence
ccggagggaguggagut

SEQ ID NO: 628 - DNA, 22 bp, Artificial
  synthetic sequence
ccctuacccgtatcttucacgg

SEQ ID NO: 629 - DNA, 27 bp, Artificial
  synthetic sequence
gaggaaaaggcggaguttatagatcug

SEQ ID NO: 630 - DNA, 20 bp, Artificial
  synthetic sequence
ccctccggcaucatcaatug

SEQ ID NO: 631 - DNA, 24 bp, Artificial
  synthetic sequence
tgcgcagatucaggatatttgugc

SEQ ID NO: 632 - DNA, 31 bp, Artificial
  synthetic sequence
ccagatacgcuttattataataattcucgcc

SEQ ID NO: 633 - DNA, 21 bp, Artificial
  synthetic sequence
ccgcaaccuggtctuaaagag

SEQ ID NO: 634 - DNA, 19 bp, Artificial
  synthetic sequence
ttggcgcutcagccaguat

SEQ ID NO: 635 - DNA, 17 bp, Artificial
  synthetic sequence
gugcccgcugaaacgga

SEQ ID NO: 636 - DNA, 18 bp, Artificial
  synthetic sequence
ccggucaagtuccgggca

SEQ ID NO: 637 - DNA, 21 bp, Artificial
  synthetic sequence
ccttuaagagcagccgggaut

SEQ ID NO: 638 - DNA, 19 bp, Artificial
  synthetic sequence
gccugagtcaaucccgacc

SEQ ID NO: 639 - DNA, 17 bp, Artificial
  synthetic sequence
gcgacggaugacgucct

SEQ ID NO: 640 - DNA, 19 bp, Artificial
  synthetic sequence
ggatgtugctagcuagcgg

SEQ ID NO: 641 - DNA, 17 bp, Artificial
  synthetic sequence
cgcgcgaaaugcugaga

SEQ ID NO: 642 - DNA, 17 bp, Artificial
  synthetic sequence
ggugaagcgauggcgaa

SEQ ID NO: 643 - DNA, 18 bp, Artificial
  synthetic sequence
gcttcaccgaauccgucg

SEQ ID NO: 644 - DNA, 33 bp, Artificial
  synthetic sequence
tttagcatctatugaaaatagtaggattucacc

SEQ ID NO: 645 - DNA, 26 bp, Artificial
  synthetic sequence
ggtttgauggcaaaaatttgtguggt

SEQ ID NO: 646 - DNA, 30 bp, Artificial
  synthetic sequence
agttaattgtggcuttagctaggataaaut

SEQ ID NO: 647 - DNA, 23 bp, Artificial
  synthetic sequence
tgtaagcggcgutgtatttgucc

SEQ ID NO: 648 - DNA, 21 bp, Artificial
  synthetic sequence
ccaataccaguccagugcagc

SEQ ID NO: 649 - DNA, 26 bp, Artificial
  synthetic sequence
cattatcaacggutttcagcgtguag

SEQ ID NO: 650 - DNA, 26 bp, Artificial
  synthetic sequence
aagaaaguaaaccttactaucacggc

SEQ ID NO: 651 - DNA, 26 bp, Artificial
  synthetic sequence
taggtcctatautccccagacucaaa

SEQ ID NO: 652 - DNA, 28 bp, Artificial
  synthetic sequence
agtagttttgtcuactcttggagtagug

SEQ ID NO: 653 - DNA, 32 bp, Artificial
  synthetic sequence
tautgattcaagttttgugaagagagaaaaac

SEQ ID NO: 654 - DNA, 27 bp, Artificial
  synthetic sequence
aggacctauacttgcaattuaaacgac

SEQ ID NO: 655 - DNA, 23 bp, Artificial
  synthetic sequence
ggaacucacgaacugaccaaaga

SEQ ID NO: 656 - DNA, 32 bp, Artificial
  synthetic sequence
cagatttaataaaagcauccccattttuagcc

SEQ ID NO: 657 - DNA, 29 bp, Artificial
  synthetic sequence
gcgcccatuccaactaatacattatctuc

SEQ ID NO: 658 - DNA, 30 bp, Artificial
  synthetic sequence
ccaatgtacaggauaactctgtatuacacg

SEQ ID NO: 659 - DNA, 29 bp, Artificial
  synthetic sequence
aaaagaagcggauagttgagttaaucagc

SEQ ID NO: 660 - DNA, 25 bp, Artificial
  synthetic sequence
cacttgtggacugtagaatauggca

SEQ ID NO: 661 - DNA, 19 bp, Artificial
  synthetic sequence
gctggauggcggtaucact

SEQ ID NO: 662 - DNA, 21 bp, Artificial
  synthetic sequence
gagcaucaatccatgucggat

SEQ ID NO: 663 - DNA, 17 bp, Artificial
  synthetic sequence
tgaugcuccgccaccca

SEQ ID NO: 664 - DNA, 19 bp, Artificial
  synthetic sequence
aggtgtcuacggcacucac

SEQ ID NO: 665 - DNA, 33 bp, Artificial
  synthetic sequence
aacttgaaaaagcaaaagauacaagagttaaug

SEQ ID NO: 666 - DNA, 33 bp, Artificial
  synthetic sequence
agcttatacuaacgataataaaaatuaacccga

SEQ ID NO: 667 - DNA, 28 bp, Artificial
  synthetic sequence
agaaagcccaacgguataaacatuacaa

SEQ ID NO: 668 - DNA, 33 bp, Artificial
  synthetic sequence
caatcgctgtctcutacttcatttattttauga

SEQ ID NO: 669 - DNA, 17 bp, Artificial
  synthetic sequence
cggcgugaucagcgcca

SEQ ID NO: 670 - DNA, 22 bp, Artificial
  synthetic sequence
ggttgctgugcctcttatgugg

SEQ ID NO: 671 - DNA, 29 bp, Artificial
  synthetic sequence
agctttatacaaaagcauatctgctccut

SEQ ID NO: 672 - DNA, 25 bp, Artificial
  synthetic sequence
ctttaacgaacgugttcgcuaaaaa

SEQ ID NO: 673 - DNA, 21 bp, Artificial
  synthetic sequence
agctcgutctcatucagcaga

SEQ ID NO: 674 - DNA, 20 bp, Artificial
  synthetic sequence
acucaggaagcttuggcaga

SEQ ID NO: 675 - DNA, 32 bp, Artificial
  synthetic sequence
cctccatataccaacutaaatactaaacaugt

SEQ ID NO: 676 - DNA, 24 bp, Artificial
  synthetic sequence
cccaagaatautttgccaagguca

SEQ ID NO: 677 - DNA, 23 bp, Artificial
  synthetic sequence
tcttgggcuatacccauagacct

SEQ ID NO: 678 - DNA, 30 bp, Artificial
  synthetic sequence
gagtcgataauaaagaggcttttaagugat

SEQ ID NO: 679 - DNA, 26 bp, Artificial
  synthetic sequence
agccacttttugttcgtcttaguact

SEQ ID NO: 680 - DNA, 28 bp, Artificial
  synthetic sequence
attcagcatattuaccacttgcaatgut

SEQ ID NO: 681 - DNA, 28 bp, Artificial
  synthetic sequence
tggatggattutatgatgcttauccaca

SEQ ID NO: 682 - DNA, 24 bp, Artificial
  synthetic sequence
aagtggctttutagttccttcugc

SEQ ID NO: 683 - DNA, 18 bp, Artificial
  synthetic sequence
cacaagggucgccgcguc

SEQ ID NO: 684 - DNA, 20 bp, Artificial
  synthetic sequence
ccgcgaaauacggcgaacug

SEQ ID NO: 685 - DNA, 33 bp, Artificial
  synthetic sequence
aaacataaacgauggaaaacagattauggaaaa

SEQ ID NO: 686 - DNA, 29 bp, Artificial
  synthetic sequence
taagaaatuaacggaaggagaugaaacac

SEQ ID NO: 687 - DNA, 19 bp, Artificial
  synthetic sequence
tcaatguaccggugggcaa

SEQ ID NO: 688 - DNA, 25 bp, Artificial
  synthetic sequence
acagacagccuaattaacgtagucc

SEQ ID NO: 689 - DNA, 17 bp, Artificial
  synthetic sequence
tucggaaccauccggca

SEQ ID NO: 690 - DNA, 22 bp, Artificial
  synthetic sequence
ccaugcagaaaaaccgatuccg

SEQ ID NO: 691 - DNA, 23 bp, Artificial
  synthetic sequence
gccattgcgcaucgtcaaaaaua

SEQ ID NO: 692 - DNA, 23 bp, Artificial
  synthetic sequence
catugcaggcaaggaaugaagag

SEQ ID NO: 693 - DNA, 23 bp, Artificial
  synthetic sequence
taagccgaaauctgaaugaccga

SEQ ID NO: 694 - DNA, 24 bp, Artificial
  synthetic sequence
cagctgauggatgagatgaucgaa

SEQ ID NO: 695 - DNA, 20 bp, Artificial
  synthetic sequence
cctuaacggcaaccacgaug

SEQ ID NO: 696 - DNA, 17 bp, Artificial
  synthetic sequence
gcgctuccagcaugcca

SEQ ID NO: 697 - DNA, 23 bp, Artificial
  synthetic sequence
ccgguatgggaauaggaaaaagc

SEQ ID NO: 698 - DNA, 18 bp, Artificial
  synthetic sequence
augcccccgcgcaaaauc

SEQ ID NO: 699 - DNA, 25 bp, Artificial
  synthetic sequence
ccagcacuccgactatagattuagt

SEQ ID NO: 700 - DNA, 28 bp, Artificial
  synthetic sequence
aatacaaaaguattctgaugacggagag

SEQ ID NO: 701 - DNA, 28 bp, Artificial
  synthetic sequence
agctactgauccccaaagtaaaattcuc

SEQ ID NO: 702 - DNA, 22 bp, Artificial
  synthetic sequence
cggacaacgaaguccgttgtut

SEQ ID NO: 703 - DNA, 17 bp, Artificial
  synthetic sequence
agcguaccggaagcucg

SEQ ID NO: 704 - DNA, 17 bp, Artificial
  synthetic sequence
gucggcaaugccggcac

SEQ ID NO: 705 - DNA, 22 bp, Artificial
  synthetic sequence
ggccgaataugtttcgcggaua

SEQ ID NO: 706 - DNA, 20 bp, Artificial
  synthetic sequence
gcgaggucaagatauacggc

SEQ ID NO: 707 - DNA, 18 bp, Artificial
  synthetic sequence
cgccaccccaccucaaut

SEQ ID NO: 708 - DNA, 18 bp, Artificial
  synthetic sequence
acccccgutgcgcacaut

SEQ ID NO: 709 - DNA, 26 bp, Artificial
  synthetic sequence
gtcagattcuctgcataattttuccg

SEQ ID NO: 710 - DNA, 20 bp, Artificial
  synthetic sequence
agcgtcaaucaggaugaggt

SEQ ID NO: 711 - DNA, 19 bp, Artificial
  synthetic sequence
ttgacgcugtcatccugct

SEQ ID NO: 712 - DNA, 21 bp, Artificial
  synthetic sequence
aaaaatcgaggauctgcugcg

SEQ ID NO: 713 - DNA, 33 bp, Artificial
  synthetic sequence
gagaagataaguacctaaatcugaaagaaacgc

SEQ ID NO: 714 - DNA, 27 bp, Artificial
  synthetic sequence
caatgaaaacuggatcacccttcugat

SEQ ID NO: 715 - DNA, 26 bp, Artificial
  synthetic sequence
aaggatgtguccaacatgaaucagga

SEQ ID NO: 716 - DNA, 28 bp, Artificial
  synthetic sequence
tcaagaaatacugtctttcttcugaccg

SEQ ID NO: 717 - DNA, 24 bp, Artificial
  synthetic sequence
gaagccaatccuggtcctggttua

SEQ ID NO: 718 - DNA, 33 bp, Artificial
  synthetic sequence
aaatgggaaataaacutcatgaatacctccuat

SEQ ID NO: 719 - DNA, 28 bp, Artificial
  synthetic sequence
agtcattaugaaggagaccaattucgac

SEQ ID NO: 720 - DNA, 20 bp, Artificial
  synthetic sequence
gggcggauagattuccggca

SEQ ID NO: 721 - DNA, 17 bp, Artificial
  synthetic sequence
auccgcccagctuagcc

SEQ ID NO: 722 - DNA, 27 bp, Artificial
  synthetic sequence
ctgattttguagagaatccctcgtuga

SEQ ID NO: 723 - DNA, 20 bp, Artificial
  synthetic sequence
aaccutgcacaucgaagagg

SEQ ID NO: 724 - DNA, 33 bp, Artificial
  synthetic sequence
attgctttatcgtuactgaaattcataatctuc

SEQ ID NO: 725 - DNA, 26 bp, Artificial
  synthetic sequence
agacaattctuggcaaacaattcugg

SEQ ID NO: 726 - DNA, 23 bp, Artificial
  synthetic sequence
gcaaggtucctacgaaaucaagc

SEQ ID NO: 727 - DNA, 18 bp, Artificial
  synthetic sequence
acccucctuaccccacca

SEQ ID NO: 728 - DNA, 26 bp, Artificial
  synthetic sequence
aacaggcgaaggaaaaaugtactuac

SEQ ID NO: 729 - DNA, 19 bp, Artificial
  synthetic sequence
agcgucgacgctctaucca

SEQ ID NO: 730 - DNA, 20 bp, Artificial
  synthetic sequence
aggagggugaacgtttuggt

SEQ ID NO: 731 - DNA, 31 bp, Artificial
  synthetic sequence
aaacagaagaacaaautcaaatgcguaacaa

SEQ ID NO: 732 - DNA, 23 bp, Artificial
  synthetic sequence
tttgcatgguattctagcucagc

SEQ ID NO: 733 - DNA, 33 bp, Artificial
  synthetic sequence
ggatatgtataatcucaatccacaagataucac

SEQ ID NO: 734 - DNA, 24 bp, Artificial
  synthetic sequence
cgacaugatatgcacucccagaga

SEQ ID NO: 735 - DNA, 31 bp, Artificial
  synthetic sequence
ttatgcaacgaauatcctaaatacaauggat

SEQ ID NO: 736 - DNA, 30 bp, Artificial
  synthetic sequence
aaactccatuaagcataggtaatgaugaga

SEQ ID NO: 737 - DNA, 28 bp, Artificial
  synthetic sequence
aguctaaattctaaatcuagggcaacgg

SEQ ID NO: 738 - DNA, 24 bp, Artificial
  synthetic sequence
attgccgautttcaggauaagcca

SEQ ID NO: 739 - DNA, 27 bp, Artificial
  synthetic sequence
tcggcaatatcautttgatttcctuca

SEQ ID NO: 740 - DNA, 32 bp, Artificial
  synthetic sequence
aatagttgcggautatataatcaacaauccaa

SEQ ID NO: 741 - DNA, 18 bp, Artificial
  synthetic sequence
gagcagucgggtgtcucc

SEQ ID NO: 742 - DNA, 21 bp, Artificial
  synthetic sequence
gggaaaucagcccttgagauc

SEQ ID NO: 743 - DNA, 24 bp, Artificial
  synthetic sequence
aaccgggaaugactaatcaagugt

SEQ ID NO: 744 - DNA, 22 bp, Artificial
  synthetic sequence
ccgattcaucaaagcauacccc

SEQ ID NO: 745 - DNA, 28 bp, Artificial
  synthetic sequence
acaaaagaaatuattggaaccatuggca

SEQ ID NO: 746 - DNA, 19 bp, Artificial
  synthetic sequence
tcccggutcuaccgaaacc

SEQ ID NO: 747 - DNA, 23 bp, Artificial
  synthetic sequence
ccggaguttgataccaugggaca

SEQ ID NO: 748 - DNA, 19 bp, Artificial
  synthetic sequence
atacctgcugcccggtuga

SEQ ID NO: 749 - DNA, 20 bp, Artificial
  synthetic sequence
gccgcttutactggcatugt

SEQ ID NO: 750 - DNA, 20 bp, Artificial
  synthetic sequence
tctcuttttcctgucccgca

SEQ ID NO: 751 - DNA, 25 bp, Artificial
  synthetic sequence
ttgtttgcgtcutatactcgtguct

SEQ ID NO: 752 - DNA, 33 bp, Artificial
  synthetic sequence
cgataatttctuaaaatttagatgtcugacaca

SEQ ID NO: 753 - DNA, 28 bp, Artificial
  synthetic sequence
agtcattttgcutgactgtattttuggt

SEQ ID NO: 754 - DNA, 25 bp, Artificial
  synthetic sequence
gcaaacaaacggauttacgaagcua

SEQ ID NO: 755 - DNA, 30 bp, Artificial
  synthetic sequence
aaaaacaaacaaauttgagagcauagagga

SEQ ID NO: 756 - DNA, 31 bp, Artificial
  synthetic sequence
ttttgttttactttaucgtccatatcgacut

SEQ ID NO: 757 - DNA, 17 bp, Artificial
  synthetic sequence
guacaggcucccggcgt

SEQ ID NO: 758 - DNA, 17 bp, Artificial
  synthetic sequence
gcttgcugcagcccucg

SEQ ID NO: 759 - DNA, 17 bp, Artificial
  synthetic sequence
ctccaccgucgggtugt

SEQ ID NO: 760 - DNA, 19 bp, Artificial
  synthetic sequence
ttccaacaugttggcucgc

SEQ ID NO: 761 - DNA, 21 bp, Artificial
  synthetic sequence
tgttggaaugcccgcttauca

SEQ ID NO: 762 - DNA, 17 bp, Artificial
  synthetic sequence
cutacgccguggccggt

SEQ ID NO: 763 - DNA, 17 bp, Artificial
  synthetic sequence
cgcgccucgtcgatcut

SEQ ID NO: 764 - DNA, 18 bp, Artificial
  synthetic sequence
cgccgugcttttugacga

SEQ ID NO: 765 - DNA, 17 bp, Artificial
  synthetic sequence
gcacggcgucaatgcut

SEQ ID NO: 766 - DNA, 28 bp, Artificial
  synthetic sequence
tgccaacggcuttatatatttctacauc

SEQ ID NO: 767 - DNA, 24 bp, Artificial
  synthetic sequence
tcctagattugcgatcagcguaag

SEQ ID NO: 768 - DNA, 17 bp, Artificial
  synthetic sequence
agccgttutacgcgcug

SEQ ID NO: 769 - DNA, 19 bp, Artificial
  synthetic sequence
gcggcgautgagcgaaaut

SEQ ID NO: 770 - DNA, 20 bp, Artificial
  synthetic sequence
tgggcgagaguttatcgugc

SEQ ID NO: 771 - DNA, 25 bp, Artificial
  synthetic sequence
ccataacggucttactgctctugaa

SEQ ID NO: 772 - DNA, 28 bp, Artificial
  synthetic sequence
agttacaggtagucccatctctauacag

SEQ ID NO: 773 - DNA, 23 bp, Artificial
  synthetic sequence
agacttgcaugttctcctgauga

SEQ ID NO: 774 - DNA, 24 bp, Artificial
  synthetic sequence
gatcgtaaacguaaccacatgguc

SEQ ID NO: 775 - DNA, 28 bp, Artificial
  synthetic sequence
ttgataatgtguttaccaacaucaccac

SEQ ID NO: 776 - DNA, 25 bp, Artificial
  synthetic sequence
cagacggtcucagtattgttcugat

SEQ ID NO: 777 - DNA, 19 bp, Artificial
  synthetic sequence
accgcaacccutgugaggt

SEQ ID NO: 778 - DNA, 17 bp, Artificial
  synthetic sequence
aggugcuaacggcgaga

SEQ ID NO: 779 - DNA, 25 bp, Artificial
  synthetic sequence
gatccaaagugatgggtccauagag

SEQ ID NO: 780 - DNA, 24 bp, Artificial
  synthetic sequence
tgcccaaaauctccaaaagatugt

SEQ ID NO: 781 - DNA, 19 bp, Artificial
  synthetic sequence
tgcttuggcttcucccact

SEQ ID NO: 782 - DNA, 32 bp, Artificial
  synthetic sequence
cgattttatggatugcttaaaaagggtuaaga

SEQ ID NO: 783 - DNA, 27 bp, Artificial
  synthetic sequence
tgtggaacaaaugagtattcuagccaa

SEQ ID NO: 784 - DNA, 24 bp, Artificial
  synthetic sequence
ataaacatcggucgcacgatuagt

SEQ ID NO: 785 - DNA, 28 bp, Artificial
  synthetic sequence
aaaacttatgatugacaatcgaggcaut

SEQ ID NO: 786 - DNA, 22 bp, Artificial
  synthetic sequence
tggctgatguttggtctguaca

SEQ ID NO: 787 - DNA, 25 bp, Artificial
  synthetic sequence
aaacggaagaaggaguctatcauga

SEQ ID NO: 788 - DNA, 30 bp, Artificial
  synthetic sequence
atcctacacgacuaatcattagagaaagut

SEQ ID NO: 789 - DNA, 17 bp, Artificial
  synthetic sequence
cguagagcctucccggt

SEQ ID NO: 790 - DNA, 20 bp, Artificial
  synthetic sequence
gggcaccgaugagaaaagut

SEQ ID NO: 791 - DNA, 22 bp, Artificial
  synthetic sequence
tgatcacuccggcuacaaaggt

SEQ ID NO: 792 - DNA, 25 bp, Artificial
  synthetic sequence
tccggatauagatactatugcaccg

SEQ ID NO: 793 - DNA, 25 bp, Artificial
  synthetic sequence
aaacgccutaaattgatucaagcga

SEQ ID NO: 794 - DNA, 21 bp, Artificial
  synthetic sequence
gtggugaaagtttctgugccc

SEQ ID NO: 795 - DNA, 27 bp, Artificial
  synthetic sequence
tcaagtttcctuctaaaagtagcucgt

SEQ ID NO: 796 - DNA, 24 bp, Artificial
  synthetic sequence
ggcgttttcuggtgtttatgtuct

SEQ ID NO: 797 - DNA, 33 bp, Artificial
  synthetic sequence
aatctttgatuggaaggttagaagtauaaaagg

SEQ ID NO: 798 - DNA, 29 bp, Artificial
  synthetic sequence
acgcaagautttcattctugaaagaggag

SEQ ID NO: 799 - DNA, 21 bp, Artificial
  synthetic sequence
ctttgcgaccacacutagcuc

SEQ ID NO: 800 - DNA, 28 bp, Artificial
  synthetic sequence
attcataagcggucgtgacttttaacut

SEQ ID NO: 801 - DNA, 24 bp, Artificial
  synthetic sequence
tgactcaccutcatatucaaagcc

SEQ ID NO: 802 - DNA, 21 bp, Artificial
  synthetic sequence
acgtttugagcgatacggucc

SEQ ID NO: 803 - DNA, 33 bp, Artificial
  synthetic sequence
aattactcctctctucttttaacctttgatcug

SEQ ID NO: 804 - DNA, 31 bp, Artificial
  synthetic sequence
taccttattatgauatcgtcatcaaaucgcc

SEQ ID NO: 805 - DNA, 28 bp, Artificial
  synthetic sequence
tctcttgatguacttgttaataaugccg

SEQ ID NO: 806 - DNA, 21 bp, Artificial
  synthetic sequence
agagcactautcgacgcuacc

SEQ ID NO: 807 - DNA, 18 bp, Artificial
  synthetic sequence
agugctctuagcggacgc

SEQ ID NO: 808 - DNA, 28 bp, Artificial
  synthetic sequence
ttctaatagacgutcacgtgatatuggt

SEQ ID NO: 809 - DNA, 24 bp, Artificial
  synthetic sequence
cttccatccucaggtatacuccag

SEQ ID NO: 810 - DNA, 31 bp, Artificial
  synthetic sequence
tgctctgtaaauggaaaatagtccaucaaat

SEQ ID NO: 811 - DNA, 23 bp, Artificial
  synthetic sequence
gcgguatttaugaagaacagcgt

SEQ ID NO: 812 - DNA, 27 bp, Artificial
  synthetic sequence
cccgacaaaatutcttcaagagtaucc

SEQ ID NO: 813 - DNA, 20 bp, Artificial
  synthetic sequence
ccgtugcaaaggcttuacac

SEQ ID NO: 814 - DNA, 20 bp, Artificial
  synthetic sequence
cggcccaguaaccagaagua

SEQ ID NO: 815 - DNA, 23 bp, Artificial
  synthetic sequence
ggutctggttttucgaaagcgag

SEQ ID NO: 816 - DNA, 23 bp, Artificial
  synthetic sequence
cctgucagcaatagtucagcact

SEQ ID NO: 817 - DNA, 20 bp, Artificial
  synthetic sequence
ccuccacaaattugagggct

SEQ ID NO: 818 - DNA, 29 bp, Artificial
  synthetic sequence
acaaggacuatatgaagtataugcaagcg

SEQ ID NO: 819 - DNA, 28 bp, Artificial
  synthetic sequence
tcactaatctttuacttgccatctcucc

SEQ ID NO: 820 - DNA, 17 bp, Artificial
  synthetic sequence
tguggaggcgtuggcat

SEQ ID NO: 821 - DNA, 21 bp, Artificial
  synthetic sequence
ttgccgctauaggagcaguaa

SEQ ID NO: 822 - DNA, 25 bp, Artificial
  synthetic sequence
attctgctttaautgaacgcaaucg

SEQ ID NO: 823 - DNA, 18 bp, Artificial
  synthetic sequence
agcagcagucgtgttugg

SEQ ID NO: 824 - DNA, 20 bp, Artificial
  synthetic sequence
agcggcaacaacugagauga

SEQ ID NO: 825 - DNA, 20 bp, Artificial
  synthetic sequence
ttttggcaacutgggcuagg

SEQ ID NO: 826 - DNA, 19 bp, Artificial
  synthetic sequence
acccaagugacatugcgct

SEQ ID NO: 827 - DNA, 18 bp, Artificial
  synthetic sequence
accaaggttctagccggt

SEQ ID NO: 828 - DNA, 19 bp, Artificial
  synthetic sequence
ggcttggtggcagtaagtg

SEQ ID NO: 829 - DNA, 18 bp, Artificial
  synthetic sequence
accatctggattgccgca

SEQ ID NO: 830 - DNA, 24 bp, Artificial
  synthetic sequence
agtgaaacaacagtattgatgccg

SEQ ID NO: 831 - DNA, 30 bp, Artificial
  synthetic sequence
acatttgctgaatcttttgctctttttact

SEQ ID NO: 832 - DNA, 28 bp, Artificial
  synthetic sequence
tcaagataaaggacatcaagtgttaggt

SEQ ID NO: 833 - DNA, 27 bp, Artificial
  synthetic sequence
catctactgaagctgcttcaaattagt

SEQ ID NO: 834 - DNA, 30 bp, Artificial
  synthetic sequence
tttgctctttgatatttttgccatacagat

SEQ ID NO: 835 - DNA, 31 bp, Artificial
  synthetic sequence
atcttgaatagtaacttttaaactttgccct

SEQ ID NO: 836 - DNA, 30 bp, Artificial
  synthetic sequence
gattctgctaaactaatcgaagaggttaga

SEQ ID NO: 837 - DNA, 26 bp, Artificial
  synthetic sequence
cagcgaataataattccccttgacag

SEQ ID NO: 838 - DNA, 24 bp, Artificial
  synthetic sequence
ggatgactttctatcggcacttca

SEQ ID NO: 839 - DNA, 21 bp, Artificial
  synthetic sequence
gcaacagcacttcgtaacgat

SEQ ID NO: 840 - DNA, 25 bp, Artificial
  synthetic sequence
ggagaaccaaattcaacacgagttt

SEQ ID NO: 841 - DNA, 25 bp, Artificial
  synthetic sequence
aattcacagcttgaggaaaaggtgt

SEQ ID NO: 842 - DNA, 20 bp, Artificial
  synthetic sequence
tggcaacatctgttcaggac

SEQ ID NO: 843 - DNA, 17 bp, Artificial
  synthetic sequence
tgcgttgctcgctctct

SEQ ID NO: 844 - DNA, 25 bp, Artificial
  synthetic sequence
tgcactctttcagaaagaaggtctt

SEQ ID NO: 845 - DNA, 21 bp, Artificial
  synthetic sequence
acgaagaagctgtggagaagt

SEQ ID NO: 846 - DNA, 20 bp, Artificial
  synthetic sequence
ccttgagactaccagggagc

SEQ ID NO: 847 - DNA, 33 bp, Artificial
  synthetic sequence
aaaagtaaacaataagaaagaggttcaatatgc

SEQ ID NO: 848 - DNA, 18 bp, Artificial
  synthetic sequence
cgcgcaacatagactccc

SEQ ID NO: 849 - DNA, 32 bp, Artificial
  synthetic sequence
aattgttcctcatcaactattttaattccttg

SEQ ID NO: 850 - DNA, 26 bp, Artificial
  synthetic sequence
gtagcgaggaggattatagtgaaaga

SEQ ID NO: 851 - DNA, 26 bp, Artificial
  synthetic sequence
gtggctttcttatgtgcatggatttg

SEQ ID NO: 852 - DNA, 32 bp, Artificial
  synthetic sequence
tattcgtaattagagtaggaggagaagctttt

SEQ ID NO: 853 - DNA, 21 bp, Artificial
  synthetic sequence
tgtggcacatgacagtcgttg

SEQ ID NO: 854 - DNA, 20 bp, Artificial
  synthetic sequence
cataaggtctttgcgctggt

SEQ ID NO: 855 - DNA, 23 bp, Artificial
  synthetic sequence
gtggcaattacttgcgtatttgg

SEQ ID NO: 856 - DNA, 20 bp, Artificial
  synthetic sequence
cctgctcaacccctatctgg

SEQ ID NO: 857 - DNA, 28 bp, Artificial
  synthetic sequence
agacaaagtatcaacattgctcatacct

SEQ ID NO: 858 - DNA, 20 bp, Artificial
  synthetic sequence
cgaaagcgggaatgctccaa

SEQ ID NO: 859 - DNA, 24 bp, Artificial
  synthetic sequence
aaatgaatgggtagaagctggtgt

SEQ ID NO: 860 - DNA, 25 bp, Artificial
  synthetic sequence
ttaagataactaggtcgccgactac

SEQ ID NO: 861 - DNA, 24 bp, Artificial
  synthetic sequence
ttcagcttcattagaagacctcgg

SEQ ID NO: 862 - DNA, 26 bp, Artificial
  synthetic sequence
cgtcaatttggactttactgattgga

SEQ ID NO: 863 - DNA, 29 bp, Artificial
  synthetic sequence
tcaccatcaagtagaactgtattttgtgt

SEQ ID NO: 864 - DNA, 21 bp, Artificial
  synthetic sequence
ccagaagaattgcttccccat

SEQ ID NO: 865 - DNA, 32 bp, Artificial
  synthetic sequence
acaatattggtcttttatttttagcaacttgt

SEQ ID NO: 866 - DNA, 27 bp, Artificial
  synthetic sequence
agcttatattgaggattgtggctacac

SEQ ID NO: 867 - DNA, 20 bp, Artificial
  synthetic sequence
tcggtgtcattgggatcgac

SEQ ID NO: 868 - DNA, 17 bp, Artificial
  synthetic sequence
ctgggcgacgacgcttt

SEQ ID NO: 869 - DNA, 20 bp, Artificial
  synthetic sequence
gtgccgtcattgaccagcat

SEQ ID NO: 870 - DNA, 17 bp, Artificial
  synthetic sequence
cggagggctatcgcgga

SEQ ID NO: 871 - DNA, 23 bp, Artificial
  synthetic sequence
gtgcctaaaagcacaagcaattg

SEQ ID NO: 872 - DNA, 28 bp, Artificial
  synthetic sequence
agggagtttaaaaatgaaacgctttcaa

SEQ ID NO: 873 - DNA, 32 bp, Artificial
  synthetic sequence
aaaggtgagaggatttaggactttttactaaa

SEQ ID NO: 874 - DNA, 32 bp, Artificial
  synthetic sequence
ctagagagatagcacctactataacagatttc

SEQ ID NO: 875 - DNA, 23 bp, Artificial
  synthetic sequence
agagaaaccagttggccttttgg

SEQ ID NO: 876 - DNA, 28 bp, Artificial
  synthetic sequence
aacaaatcctcgatttatttcatggcag

SEQ ID NO: 877 - DNA, 32 bp, Artificial
  synthetic sequence
aatggatttattttgattccgaatatgctttt

SEQ ID NO: 878 - DNA, 33 bp, Artificial
  synthetic sequence
attgccaatattcaatcttctaaattcatcaat

SEQ ID NO: 879 - DNA, 31 bp, Artificial
  synthetic sequence
ttggcaatgtgatctttattgcaatttaatt

SEQ ID NO: 880 - DNA, 31 bp, Artificial
  synthetic sequence
agaaatgagatagcttttaataatcactgca

SEQ ID NO: 881 - DNA, 24 bp, Artificial
  synthetic sequence
gctgcagggattattctttctcca

SEQ ID NO: 882 - DNA, 25 bp, Artificial
  synthetic sequence
agggctctatctatcagaatcggaa

SEQ ID NO: 883 - DNA, 22 bp, Artificial
  synthetic sequence
agagcccttctcgaatatggga

SEQ ID NO: 884 - DNA, 22 bp, Artificial
  synthetic sequence
aaatcgggtgcaccttctgtaa

SEQ ID NO: 885 - DNA, 22 bp, Artificial
  synthetic sequence
agcaaaagcttgcatattggca

SEQ ID NO: 886 - DNA, 28 bp, Artificial
  synthetic sequence
acctctataggtgtccgttattttgatg

SEQ ID NO: 887 - DNA, 30 bp, Artificial
  synthetic sequence
gcgttctccatcttttatagcagaaatacg

SEQ ID NO: 888 - DNA, 31 bp, Artificial
  synthetic sequence
ttattttagtgggttctgcaatgacaagata

SEQ ID NO: 889 - DNA, 27 bp, Artificial
  synthetic sequence
aacaattcttttagcctaacagtgcca

SEQ ID NO: 890 - DNA, 25 bp, Artificial
  synthetic sequence
gcgaaagttacttaggtggtcttgc

SEQ ID NO: 891 - DNA, 32 bp, Artificial
  synthetic sequence
gttatgaagcttattaatggtagtggtgatga

SEQ ID NO: 892 - DNA, 29 bp, Artificial
  synthetic sequence
cctcaaattgatcttctgctgaagtatta

SEQ ID NO: 893 - DNA, 17 bp, Artificial
  synthetic sequence
ttggcggatacagccct

SEQ ID NO: 894 - DNA, 23 bp, Artificial
  synthetic sequence
atccagactctcctgattgtcca

SEQ ID NO: 895 - DNA, 22 bp, Artificial
  synthetic sequence
gatctgccatagaatctcgtcg

SEQ ID NO: 896 - DNA, 20 bp, Artificial
  synthetic sequence
cggctgaagaagagtgggaa

SEQ ID NO: 897 - DNA, 17 bp, Artificial
  synthetic sequence
tccgggcagcgagtctg

SEQ ID NO: 898 - DNA, 19 bp, Artificial
  synthetic sequence
ggcagatcgattgcagggt

SEQ ID NO: 899 - DNA, 30 bp, Artificial
  synthetic sequence
aaaaacggaggagactaattaatatggcaa

SEQ ID NO: 900 - DNA, 31 bp, Artificial
  synthetic sequence
tgcttttgcttcttgtaattacgaattaact

SEQ ID NO: 901 - DNA, 22 bp, Artificial
  synthetic sequence
ccggttgaccgtatactacgct

SEQ ID NO: 902 - DNA, 29 bp, Artificial
  synthetic sequence
cacaatcgtttttagctagaatcactgtt

SEQ ID NO: 903 - DNA, 19 bp, Artificial
  synthetic sequence
ggaacagccgtctgatcac

SEQ ID NO: 904 - DNA, 30 bp, Artificial
  synthetic sequence
aaaaacactcattgttttcatcgtttttca

SEQ ID NO: 905 - DNA, 23 bp, Artificial
  synthetic sequence
ccaaagacttcgagtagggcttg

SEQ ID NO: 906 - DNA, 26 bp, Artificial
  synthetic sequence
gattgttcatatgggctctcctatcc

SEQ ID NO: 907 - DNA, 25 bp, Artificial
  synthetic sequence
cgccgaatgatgttcgaaatatggt

SEQ ID NO: 908 - DNA, 25 bp, Artificial
  synthetic sequence
ccgacaatctcaagaaaacgctgat

SEQ ID NO: 909 - DNA, 20 bp, Artificial
  synthetic sequence
acgggtcttagcattggctt

SEQ ID NO: 910 - DNA, 19 bp, Artificial
  synthetic sequence
gcacgcgtcaattaagccc

SEQ ID NO: 911 - DNA, 22 bp, Artificial
  synthetic sequence
tcaatggttaagttggccgtag

SEQ ID NO: 912 - DNA, 21 bp, Artificial
  synthetic sequence
acgatcactcaaaatggtgcg

SEQ ID NO: 913 - DNA, 24 bp, Artificial
  synthetic sequence
ccaaagcattggcatatgcagata

SEQ ID NO: 914 - DNA, 25 bp, Artificial
  synthetic sequence
aagcccaatcgtcatctttgtagtt

SEQ ID NO: 915 - DNA, 33 bp, Artificial
  synthetic sequence
actaataataagggattttctgaatttggtgat

SEQ ID NO: 916 - DNA, 29 bp, Artificial
  synthetic sequence
aactttttagtatccttagcgaagttgac

SEQ ID NO: 917 - DNA, 30 bp, Artificial
  synthetic sequence
tgctcaaagtgagaacttttcaaatcgtaa

SEQ ID NO: 918 - DNA, 28 bp, Artificial
  synthetic sequence
tctgtttgtgaataactaccgttaggac

SEQ ID NO: 919 - DNA, 33 bp, Artificial
  synthetic sequence
agcattactacaaaaagaatcaagcaataataa

SEQ ID NO: 920 - DNA, 33 bp, Artificial
  synthetic sequence
atttagggtgtaacaaagatgaaaaacattaat

SEQ ID NO: 921 - DNA, 27 bp, Artificial
  synthetic sequence
gcacctgcttttataacatcatttcca

SEQ ID NO: 922 - DNA, 31 bp, Artificial
  synthetic sequence
acagaagaaaatatgtctgctacaaatagat

SEQ ID NO: 923 - DNA, 32 bp, Artificial
  synthetic sequence
gtaatcctactttcatcatatgaagaagaact

SEQ ID NO: 924 - DNA, 23 bp, Artificial
  synthetic sequence
ggtgcaacatgaaatcaaggtga

SEQ ID NO: 925 - DNA, 26 bp, Artificial
  synthetic sequence
gaaattgctacagagatagtcccacc

SEQ ID NO: 926 - DNA, 32 bp, Artificial
  synthetic sequence
gtaatgcttttaaaaatcattctaatgaccca

SEQ ID NO: 927 - DNA, 29 bp, Artificial
  synthetic sequence
actggcaattcatcagaaaatacatctac

SEQ ID NO: 928 - DNA, 22 bp, Artificial
  synthetic sequence
ccgtagtttttccttgctgacc

SEQ ID NO: 929 - DNA, 20 bp, Artificial
  synthetic sequence
ggacagctacccttgttgca

SEQ ID NO: 930 - DNA, 33 bp, Artificial
  synthetic sequence
aaagcacgattaatagttaaattaccaaaaaca

SEQ ID NO: 931 - DNA, 28 bp, Artificial
  synthetic sequence
cgcttcaactgatcatgtagaaaaagtg

SEQ ID NO: 932 - DNA, 26 bp, Artificial
  synthetic sequence
cagcatgactgttatcagtgtttgtt

SEQ ID NO: 933 - DNA, 26 bp, Artificial
  synthetic sequence
ggtgttaaggtgaattggactcaaac

SEQ ID NO: 934 - DNA, 29 bp, Artificial
  synthetic sequence
cctgtgcccaattcattattagtattcat

SEQ ID NO: 935 - DNA, 18 bp, Artificial
  synthetic sequence
aaacctttgccgggcgtc

SEQ ID NO: 936 - DNA, 17 bp, Artificial
  synthetic sequence
cgcatcaggctcccgca

SEQ ID NO: 937 - DNA, 17 bp, Artificial
  synthetic sequence
gcggatatcacggacgc

SEQ ID NO: 938 - DNA, 17 bp, Artificial
  synthetic sequence
ggctgcggttgtggtcg

SEQ ID NO: 939 - DNA, 19 bp, Artificial
  synthetic sequence
aggtaccggcctgctgcat

SEQ ID NO: 940 - DNA, 17 bp, Artificial
  synthetic sequence
ttcgctgcccgaagccg

SEQ ID NO: 941 - DNA, 21 bp, Artificial
  synthetic sequence
agcagaaagacaggcatgatg

SEQ ID NO: 942 - DNA, 18 bp, Artificial
  synthetic sequence
agcacctactgcatcgcc

SEQ ID NO: 943 - DNA, 19 bp, Artificial
  synthetic sequence
atgcagccacaaccaatcg

SEQ ID NO: 944 - DNA, 21 bp, Artificial
  synthetic sequence
ttcggccacattccatcctaa

SEQ ID NO: 945 - DNA, 20 bp, Artificial
  synthetic sequence
ttgctgaccaaaaccaccac

SEQ ID NO: 946 - DNA, 26 bp, Artificial
  synthetic sequence
tttttatggaatgtttttctgtcggg

SEQ ID NO: 947 - DNA, 26 bp, Artificial
  synthetic sequence
gttcctattcctatctcttccggtgg

SEQ ID NO: 948 - DNA, 20 bp, Artificial
  synthetic sequence
ccgcctttgatagatccgct

SEQ ID NO: 949 - DNA, 19 bp, Artificial
  synthetic sequence
agtcccaacgccattgtgc

SEQ ID NO: 950 - DNA, 26 bp, Artificial
  synthetic sequence
caaggatgtttatgaacggcaaaaca

SEQ ID NO: 951 - DNA, 26 bp, Artificial
  synthetic sequence
gaatatgagccatgagatacgtacgc

SEQ ID NO: 952 - DNA, 26 bp, Artificial
  synthetic sequence
agaaagacatgctaccggattctatg

SEQ ID NO: 953 - DNA, 21 bp, Artificial
  synthetic sequence
gaagctggatttgccgaccta

SEQ ID NO: 954 - DNA, 19 bp, Artificial
  synthetic sequence
gcgggcacaaaactcttca

SEQ ID NO: 955 - DNA, 20 bp, Artificial
  synthetic sequence
actcaggcgactcagtcttg

SEQ ID NO: 956 - DNA, 17 bp, Artificial
  synthetic sequence
ggcggttctggtcaagc

SEQ ID NO: 957 - DNA, 19 bp, Artificial
  synthetic sequence
ttctgacgcctatgggaca

SEQ ID NO: 958 - DNA, 17 bp, Artificial
  synthetic sequence
ggttgcggacctgcatc

SEQ ID NO: 959 - DNA, 18 bp, Artificial
  synthetic sequence
cccacgaatgcgatcacg

SEQ ID NO: 960 - DNA, 21 bp, Artificial
  synthetic sequence
cagcaaggccgatgagataag

SEQ ID NO: 961 - DNA, 26 bp, Artificial
  synthetic sequence
gtgacatctgaggtagatgatatggc

SEQ ID NO: 962 - DNA, 20 bp, Artificial
  synthetic sequence
actcggcacagatacaagca

SEQ ID NO: 963 - DNA, 18 bp, Artificial
  synthetic sequence
agccagatctccacgctc

SEQ ID NO: 964 - DNA, 31 bp, Artificial
  synthetic sequence
tagggcatatcgataaaagctgtaataaaaa

SEQ ID NO: 965 - DNA, 21 bp, Artificial
  synthetic sequence
atgccctaaaaatcgcaagct

SEQ ID NO: 966 - DNA, 19 bp, Artificial
  synthetic sequence
gatatggctgcaaacgcga

SEQ ID NO: 967 - DNA, 28 bp, Artificial
  synthetic sequence
gccggagtatcaagatttaaaccataag

SEQ ID NO: 968 - DNA, 32 bp, Artificial
  synthetic sequence
agattgttttatttatttgcaaagagatgacg

SEQ ID NO: 969 - DNA, 27 bp, Artificial
  synthetic sequence
ctttgcaaaattttgcatattcaccga

SEQ ID NO: 970 - DNA, 28 bp, Artificial
  synthetic sequence
gattgatgtggctattaaaagtatcggc

SEQ ID NO: 971 - DNA, 21 bp, Artificial
  synthetic sequence
gctgacgctctcataaacgga

SEQ ID NO: 972 - DNA, 25 bp, Artificial
  synthetic sequence
ttgcaaagaattttgcgccattatt

SEQ ID NO: 973 - DNA, 33 bp, Artificial
  synthetic sequence
aggtttaaagtattttctacaaaaacttcaaca

SEQ ID NO: 974 - DNA, 19 bp, Artificial
  synthetic sequence
actccggcagaaagggatt

SEQ ID NO: 975 - DNA, 26 bp, Artificial
  synthetic sequence
catcgataagctcatcatcatgccaa

SEQ ID NO: 976 - DNA, 32 bp, Artificial
  synthetic sequence
taaatttatctcatagtctgagatatcgacct

SEQ ID NO: 977 - DNA, 24 bp, Artificial
  synthetic sequence
ataatacgagcagcacacctaccg

SEQ ID NO: 978 - DNA, 23 bp, Artificial
  synthetic sequence
aaatgaaccggatcaaagctccc

SEQ ID NO: 979 - DNA, 31 bp, Artificial
  synthetic sequence
agaggagtcttttaaaaagactgaagaagat

SEQ ID NO: 980 - DNA, 24 bp, Artificial
  synthetic sequence
ttgcgtcagtgatctcagaaacat

SEQ ID NO: 981 - DNA, 20 bp, Artificial
  synthetic sequence
ggcattctgaggtaccggaa

SEQ ID NO: 982 - DNA, 27 bp, Artificial
  synthetic sequence
ttttcgcctctcacattggaaattatt

SEQ ID NO: 983 - DNA, 22 bp, Artificial
  synthetic sequence
tgggcatgatcggagaaagaag

SEQ ID NO: 984 - DNA, 21 bp, Artificial
  synthetic sequence
ttgccatggtattccttggcg

SEQ ID NO: 985 - DNA, 26 bp, Artificial
  synthetic sequence
ccaattgaactactgacctgttggag

SEQ ID NO: 986 - DNA, 18 bp, Artificial
  synthetic sequence
caccgtgggtgctggtcg

SEQ ID NO: 987 - DNA, 23 bp, Artificial
  synthetic sequence
cgcagtacatggatcacctgttc

SEQ ID NO: 988 - DNA, 18 bp, Artificial
  synthetic sequence
cgtatgcgatgcgttcgc

SEQ ID NO: 989 - DNA, 17 bp, Artificial
  synthetic sequence
cgcatacgtgcagcggt

SEQ ID NO: 990 - DNA, 17 bp, Artificial
  synthetic sequence
ggacaggtgcccggtgg

SEQ ID NO: 991 - DNA, 20 bp, Artificial
  synthetic sequence
ctgttctgctggttctgcga

SEQ ID NO: 992 - DNA, 19 bp, Artificial
  synthetic sequence
gccgtagtaacagcctcga

SEQ ID NO: 993 - DNA, 21 bp, Artificial
  synthetic sequence
actacggcatcatcgttgtct

SEQ ID NO: 994 - DNA, 17 bp, Artificial
  synthetic sequence
gttacgcgcatcgagcc

SEQ ID NO: 995 - DNA, 17 bp, Artificial
  synthetic sequence
gcagccagcccttcttg

SEQ ID NO: 996 - DNA, 22 bp, Artificial
  synthetic sequence
ggcagaagatttgatgctccat

SEQ ID NO: 997 - DNA, 28 bp, Artificial
  synthetic sequence
acagccgcttgattatatttaaactgcc

SEQ ID NO: 998 - DNA, 26 bp, Artificial
  synthetic sequence
agaggtattccaaatgcagcttattg

SEQ ID NO: 999 - DNA, 33 bp, Artificial
  synthetic sequence
acgataccagtaatacttattaaactcatcaaa

SEQ ID NO: 1000 - DNA, 18 bp, Artificial
  synthetic sequence
tggctgcttggaaacgag

SEQ ID NO: 1001 - DNA, 26 bp, Artificial
  synthetic sequence
gctggtattggtatgattccagatgg

SEQ ID NO: 1002 - DNA, 21 bp, Artificial
  synthetic sequence
aaaccaaaccgttgccccata

SEQ ID NO: 1003 - DNA, 31 bp, Artificial
  synthetic sequence
tcgactgatatatcaagagaaagaaagtgta

SEQ ID NO: 1004 - DNA, 23 bp, Artificial
  synthetic sequence
catcagccatgtgtacaaaacct

SEQ ID NO: 1005 - DNA, 28 bp, Artificial
  synthetic sequence
agaaacggctataccaattcatgaagag

SEQ ID NO: 1006 - DNA, 31 bp, Artificial
  synthetic sequence
cttcgttcgtaatagatggctctacaataag

SEQ ID NO: 1007 - DNA, 19 bp, Artificial
  synthetic sequence
gcggaatggcgtttacagt

SEQ ID NO: 1008 - DNA, 33 bp, Artificial
  synthetic sequence
tttagcttatcaatagcacaattttagaaaaca

SEQ ID NO: 1009 - DNA, 17 bp, Artificial
  synthetic sequence
gccacccagccatgatg

SEQ ID NO: 1010 - DNA, 18 bp, Artificial
  synthetic sequence
gcgcggtggaggtgtcta

SEQ ID NO: 1011 - DNA, 33 bp, Artificial
  synthetic sequence
actatgaataaaatttatttctctcaagacccg

SEQ ID NO: 1012 - DNA, 17 bp, Artificial
  synthetic sequence
tgggtggcggagcatca

SEQ ID NO: 1013 - DNA, 20 bp, Artificial
  synthetic sequence
ctggatacgcagaccgatgt

SEQ ID NO: 1014 - DNA, 21 bp, Artificial
  synthetic sequence
cattccgctgtttcatctgca

SEQ ID NO: 1015 - DNA, 24 bp, Artificial
  synthetic sequence
atgttgttcaaggtgacggtactg

SEQ ID NO: 1016 - DNA, 29 bp, Artificial
  synthetic sequence
caaggtttcaaggaacattgaagtgataa

SEQ ID NO: 1017 - DNA, 31 bp, Artificial
  synthetic sequence
caaaacaggagataagatttttgtcacagga

SEQ ID NO: 1018 - DNA, 22 bp, Artificial
  synthetic sequence
aaacagttcagcacgttcctga

SEQ ID NO: 1019 - DNA, 30 bp, Artificial
  synthetic sequence
cggtgacacctaaagaactgatgatattct

SEQ ID NO: 1020 - DNA, 32 bp, Artificial
  synthetic sequence
tgacgatatcctttttattcaagtctctaagg

SEQ ID NO: 1021 - DNA, 33 bp, Artificial
  synthetic sequence
taatgaaatccaaatattctctttctttatggc

SEQ ID NO: 1022 - DNA, 18 bp, Artificial
  synthetic sequence
aacgagctagcgatcgca

SEQ ID NO: 1023 - DNA, 17 bp, Artificial
  synthetic sequence
tcctgcaatcaccggca

SEQ ID NO: 1024 - DNA, 20 bp, Artificial
  synthetic sequence
tcacgccgatgaatgaagag

SEQ ID NO: 1025 - DNA, 27 bp, Artificial
  synthetic sequence
attctacccatgtctctgggattttga

SEQ ID NO: 1026 - DNA, 25 bp, Artificial
  synthetic sequence
agaaaaaccaaaagcaactggtacg

SEQ ID NO: 1027 - DNA, 24 bp, Artificial
  synthetic sequence
ggattcatggataggagaaaggct

SEQ ID NO: 1028 - DNA, 21 bp, Artificial
  synthetic sequence
tgccgcctacctaccagtatg

SEQ ID NO: 1029 - DNA, 32 bp, Artificial
  synthetic sequence
gtatcctagatatgtcatttaggtcttctaca

SEQ ID NO: 1030 - DNA, 28 bp, Artificial
  synthetic sequence
agagattgatgacctgactatagagtct

SEQ ID NO: 1031 - DNA, 24 bp, Artificial
  synthetic sequence
ttgaacttgaatcgaccctatgca

SEQ ID NO: 1032 - DNA, 29 bp, Artificial
  synthetic sequence
atgaatccaaatagggattctgactatgt

SEQ ID NO: 1033 - DNA, 27 bp, Artificial
  synthetic sequence
atctctatatcaaagctcctggacaca

SEQ ID NO: 1034 - DNA, 31 bp, Artificial
  synthetic sequence
aggtttaggaaggaatttacaactgaaaata

SEQ ID NO: 1035 - DNA, 28 bp, Artificial
  synthetic sequence
tccttgcgacttttgcaaataatattga

SEQ ID NO: 1036 - DNA, 32 bp, Artificial
  synthetic sequence
aaagatcttgattatgaaattcaagagcaatt

SEQ ID NO: 1037 - DNA, 30 bp, Artificial
  synthetic sequence
tttttcagcttgcaaacgctttattaaatt

SEQ ID NO: 1038 - DNA, 31 bp, Artificial
  synthetic sequence
tgaattgcctatttatacacgcaataaattt

SEQ ID NO: 1039 - DNA, 32 bp, Artificial
  synthetic sequence
tcggttaatttactgaatgcaaaaagtaaaaa

SEQ ID NO: 1040 - DNA, 30 bp, Artificial
  synthetic sequence
aatacaaataatctatcgctttttgggtgt

SEQ ID NO: 1041 - DNA, 31 bp, Artificial
  synthetic sequence
ttttacattctgtttaccaggatcaattaca

SEQ ID NO: 1042 - DNA, 30 bp, Artificial
  synthetic sequence
gccttcttcaaattctttatagctttttgc

SEQ ID NO: 1043 - DNA, 18 bp, Artificial
  synthetic sequence
tttcgcggtgtagagccg

SEQ ID NO: 1044 - DNA, 17 bp, Artificial
  synthetic sequence
ctgcagagccggccctc

SEQ ID NO: 1045 - DNA, 17 bp, Artificial
  synthetic sequence
gctgagccggtcaatgc

SEQ ID NO: 1046 - DNA, 19 bp, Artificial
  synthetic sequence
agtgtggcaccaatgaacc

SEQ ID NO: 1047 - DNA, 20 bp, Artificial
  synthetic sequence
gttccggtaaaagcaggtgt

SEQ ID NO: 1048 - DNA, 20 bp, Artificial
  synthetic sequence
acccgctggtcaatttctct

SEQ ID NO: 1049 - DNA, 30 bp, Artificial
  synthetic sequence
caccttacatgtaaaaattcttgcgatttc

SEQ ID NO: 1050 - DNA, 18 bp, Artificial
  synthetic sequence
ccggaaccccatccctgt

SEQ ID NO: 1051 - DNA, 20 bp, Artificial
  synthetic sequence
cttctgcatcccgaacctcc

SEQ ID NO: 1052 - DNA, 25 bp, Artificial
  synthetic sequence
tatttcgttggcaatagaagagcca

SEQ ID NO: 1053 - DNA, 26 bp, Artificial
  synthetic sequence
cacttttatactgtacctcgaccaca

SEQ ID NO: 1054 - DNA, 17 bp, Artificial
  synthetic sequence
gggcgtagtcggtgagt

SEQ ID NO: 1055 - DNA, 22 bp, Artificial
  synthetic sequence
cgaccctgacactttttgcatt

SEQ ID NO: 1056 - DNA, 28 bp, Artificial
  synthetic sequence
tcatgatgagaacttggagataaagcct

SEQ ID NO: 1057 - DNA, 22 bp, Artificial
  synthetic sequence
ctacgcccactttaaactgtgg

SEQ ID NO: 1058 - DNA, 27 bp, Artificial
  synthetic sequence
cagggtcgatatcgatatcgataatgt

SEQ ID NO: 1059 - DNA, 19 bp, Artificial
  synthetic sequence
tccttgcaggcattcaggt

SEQ ID NO: 1060 - DNA, 32 bp, Artificial
  synthetic sequence
actgactataaattgatattgtgtgatgacag

SEQ ID NO: 1061 - DNA, 22 bp, Artificial
  synthetic sequence
aagccgaaatctgaatgaccga

SEQ ID NO: 1062 - DNA, 23 bp, Artificial
  synthetic sequence
tcgaagaagcactgcatcatgtc

SEQ ID NO: 1063 - DNA, 22 bp, Artificial
  synthetic sequence
gtgcaggcgatctacaacattc

SEQ ID NO: 1064 - DNA, 25 bp, Artificial
  synthetic sequence
aataattatcagttgctcgcagcct

SEQ ID NO: 1065 - DNA, 29 bp, Artificial
  synthetic sequence
ctaaagctttgtctatcttatcaacagct

SEQ ID NO: 1066 - DNA, 23 bp, Artificial
  synthetic sequence
ggtaactcagacgagttctcgtg

SEQ ID NO: 1067 - DNA, 28 bp, Artificial
  synthetic sequence
agatggattgtttatccagttttctgtg

SEQ ID NO: 1068 - DNA, 33 bp, Artificial
  synthetic sequence
ggaactacactttcttttaatgcttttaaagat

SEQ ID NO: 1069 - DNA, 28 bp, Artificial
  synthetic sequence
gcgaataaatattctactgacgcttcat

SEQ ID NO: 1070 - DNA, 23 bp, Artificial
  synthetic sequence
tcttgttgccttcagttccaact

SEQ ID NO: 1071 - DNA, 28 bp, Artificial
  synthetic sequence
ccattgttgagtcgtcagcttcatttat

SEQ ID NO: 1072 - DNA, 27 bp, Artificial
  synthetic sequence
agctttagcaagagctataaaccaagt

SEQ ID NO: 1073 - DNA, 26 bp, Artificial
  synthetic sequence
gctgagacaattctttttcgaactca

SEQ ID NO: 1074 - DNA, 21 bp, Artificial
  synthetic sequence
gccagaagcgacagtagctta

SEQ ID NO: 1075 - DNA, 32 bp, Artificial
  synthetic sequence
tgatatcatcaacattaaacatctcatagtcc

SEQ ID NO: 1076 - DNA, 27 bp, Artificial
  synthetic sequence
accaagcttttataagagagttgctct

SEQ ID NO: 1077 - DNA, 28 bp, Artificial
  synthetic sequence
agcttggtaattcagacaaatcaattcg

SEQ ID NO: 1078 - DNA, 27 bp, Artificial
  synthetic sequence
gtctcagcatgattatttccattcacg

SEQ ID NO: 1079 - DNA, 17 bp, Artificial
  synthetic sequence
cgtcgccaagccttcga

SEQ ID NO: 1080 - DNA, 18 bp, Artificial
  synthetic sequence
tggttctggtcgacctgt

SEQ ID NO: 1081 - DNA, 18 bp, Artificial
  synthetic sequence
gacctcgcttacccggaa

SEQ ID NO: 1082 - DNA, 22 bp, Artificial
  synthetic sequence
acctcctgaatcttatccgcga

SEQ ID NO: 1083 - DNA, 19 bp, Artificial
  synthetic sequence
cacggtggccgctttaatg

SEQ ID NO: 1084 - DNA, 17 bp, Artificial
  synthetic sequence
tggcgacggtacttggc

SEQ ID NO: 1085 - DNA, 24 bp, Artificial
  synthetic sequence
catcagcgtcaaatcagtcaaccg

SEQ ID NO: 1086 - DNA, 17 bp, Artificial
  synthetic sequence
ggtacgctgttcgccgt

SEQ ID NO: 1087 - DNA, 23 bp, Artificial
  synthetic sequence
aggagtagacatccatgaatccg

SEQ ID NO: 1088 - DNA, 20 bp, Artificial
  synthetic sequence
ttcgcgtcatggcatatgct

SEQ ID NO: 1089 - DNA, 22 bp, Artificial
  synthetic sequence
ggaactggatgtatcgcgatga

SEQ ID NO: 1090 - DNA, 17 bp, Artificial
  synthetic sequence
gtcgccaaatgggcgat

SEQ ID NO: 1091 - DNA, 19 bp, Artificial
  synthetic sequence
tgtaaaaccggcgaggtgg

SEQ ID NO: 1092 - DNA, 18 bp, Artificial
  synthetic sequence
cgctcaaatgtcctcgct

SEQ ID NO: 1093 - DNA, 20 bp, Artificial
  synthetic sequence
tttgagcgcacaagtagggt

SEQ ID NO: 1094 - DNA, 19 bp, Artificial
  synthetic sequence
ccagttcccagtccatgca

SEQ ID NO: 1095 - DNA, 17 bp, Artificial
  synthetic sequence
ccggtttccctggttcg

SEQ ID NO: 1096 - DNA, 21 bp, Artificial
  synthetic sequence
ctgaatttacgcgtgaggtga

SEQ ID NO: 1097 - DNA, 24 bp, Artificial
  synthetic sequence
cgatcactccaaatccggagcata

SEQ ID NO: 1098 - DNA, 18 bp, Artificial
  synthetic sequence
aaccgggtggcagccgta

SEQ ID NO: 1099 - DNA, 17 bp, Artificial
  synthetic sequence
cggcacctttctggcac

SEQ ID NO: 1100 - DNA, 17 bp, Artificial
  synthetic sequence
gactgtggcttgctgca

SEQ ID NO: 1101 - DNA, 19 bp, Artificial
  synthetic sequence
ctgcccggtatttcgcatt

SEQ ID NO: 1102 - DNA, 20 bp, Artificial
  synthetic sequence
acgggcacagattatcgtgt

SEQ ID NO: 1103 - DNA, 28 bp, Artificial
  synthetic sequence
tttggagcaatgattatcggtccattaa

SEQ ID NO: 1104 - DNA, 28 bp, Artificial
  synthetic sequence
ctccaattaagcctgcagaaaaattacg

SEQ ID NO: 1105 - DNA, 25 bp, Artificial
  synthetic sequence
attacggtacctggaaatgaaggct

SEQ ID NO: 1106 - DNA, 32 bp, Artificial
  synthetic sequence
gatagcacgaccgatcaaataaaaatactatt

SEQ ID NO: 1107 - DNA, 24 bp, Artificial
  synthetic sequence
atggttggtatggcagttattggc

SEQ ID NO: 1108 - DNA, 25 bp, Artificial
  synthetic sequence
ttgataatgccttgtaagaatgccc

SEQ ID NO: 1109 - DNA, 23 bp, Artificial
  synthetic sequence
ccacaccatttttgccctttcac

SEQ ID NO: 1110 - DNA, 17 bp, Artificial
  synthetic sequence
cggcttcacccagttcg

SEQ ID NO: 1111 - DNA, 18 bp, Artificial
  synthetic sequence
tgaagccggatggcttga

SEQ ID NO: 1112 - DNA, 33 bp, Artificial
  synthetic sequence
tcttcaaattttaattcttagatgttgatccac

SEQ ID NO: 1113 - DNA, 17 bp, Artificial
  synthetic sequence
cgtcccagctgacgcaa

SEQ ID NO: 1114 - DNA, 22 bp, Artificial
  synthetic sequence
tcggtatgggattatccgtcct

SEQ ID NO: 1115 - DNA, 32 bp, Artificial
  synthetic sequence
ctttaaaatcagatccagattttcatgttcca

SEQ ID NO: 1116 - DNA, 21 bp, Artificial
  synthetic sequence
tgaagaaaattccgccgctga

SEQ ID NO: 1117 - DNA, 22 bp, Artificial
  synthetic sequence
gccatagaccgctctgacttcc

SEQ ID NO: 1118 - DNA, 22 bp, Artificial
  synthetic sequence
cgcagctcagaccattcattgg

SEQ ID NO: 1119 - DNA, 28 bp, Artificial
  synthetic sequence
ttggaagacgtcatcctcgatataatga

SEQ ID NO: 1120 - DNA, 20 bp, Artificial
  synthetic sequence
tcaatgcaaccctttcccag

SEQ ID NO: 1121 - DNA, 25 bp, Artificial
  synthetic sequence
agagtgagacaattacgctaccttg

SEQ ID NO: 1122 - DNA, 33 bp, Artificial
  synthetic sequence
ttgatatttcattttcaaggtgtttaaagtgag

SEQ ID NO: 1123 - DNA, 31 bp, Artificial
  synthetic sequence
agattctaaagaagtgctagatttaagtgcg

SEQ ID NO: 1124 - DNA, 31 bp, Artificial
  synthetic sequence
ttgatgacattttgagagaatgtcttgcata

SEQ ID NO: 1125 - DNA, 18 bp, Artificial
  synthetic sequence
ggaatgtgcgtcgaacgg

SEQ ID NO: 1126 - DNA, 18 bp, Artificial
  synthetic sequence
ccagctgcggttgcgatt

SEQ ID NO: 1127 - DNA, 21 bp, Artificial
  synthetic sequence
ccgtaccggattccagcgtat

SEQ ID NO: 1128 - DNA, 31 bp, Artificial
  synthetic sequence
gtctggaatgtagaactatgcgatgatatat

SEQ ID NO: 1129 - DNA, 18 bp, Artificial
  synthetic sequence
ctcttggcgcgaatggac

SEQ ID NO: 1130 - DNA, 18 bp, Artificial
  synthetic sequence
tgggcggctatctggatg

SEQ ID NO: 1131 - DNA, 28 bp, Artificial
  synthetic sequence
aaggacttatgcctcaattaattcaacc

SEQ ID NO: 1132 - DNA, 25 bp, Artificial
  synthetic sequence
tctaccgcagataaaactcccacta

SEQ ID NO: 1133 - DNA, 28 bp, Artificial
  synthetic sequence
acctatagtcatatcaactggaattgcg

SEQ ID NO: 1134 - DNA, 21 bp, Artificial
  synthetic sequence
aagtccttgcatccactttgg

SEQ ID NO: 1135 - DNA, 28 bp, Artificial
  synthetic sequence
tactggagatgtattagtgggagaagtt

SEQ ID NO: 1136 - DNA, 32 bp, Artificial
  synthetic sequence
ttgcataataatttgtaaggtttttcatcctc

SEQ ID NO: 1137 - DNA, 17 bp, Artificial
  synthetic sequence
cgttccatcccacccct

SEQ ID NO: 1138 - DNA, 24 bp, Artificial
  synthetic sequence
gcatccagaatgcttttcttaccg

SEQ ID NO: 1139 - DNA, 21 bp, Artificial
  synthetic sequence
tccccaatcttccgtatagcg

SEQ ID NO: 1140 - DNA, 21 bp, Artificial
  synthetic sequence
atcagcgaaatgccgttcaaa

SEQ ID NO: 1141 - DNA, 22 bp, Artificial
  synthetic sequence
aaagaccgccgttgcggtttta

SEQ ID NO: 1142 - DNA, 17 bp, Artificial
  synthetic sequence
atggaacggcccatgca

SEQ ID NO: 1143 - DNA, 21 bp, Artificial
  synthetic sequence
atgcatctgtttcctggccat

SEQ ID NO: 1144 - DNA, 25 bp, Artificial
  synthetic sequence
ttttgcaatctgaatgtgatctggg

SEQ ID NO: 1145 - DNA, 24 bp, Artificial
  synthetic sequence
aaacagatcacgtccaaggtcatc

SEQ ID NO: 1146 - DNA, 17 bp, Artificial
  synthetic sequence
gggccgatgcatggaga

SEQ ID NO: 1147 - DNA, 18 bp, Artificial
  synthetic sequence
atcggcccagtatccgat

SEQ ID NO: 1148 - DNA, 23 bp, Artificial
  synthetic sequence
atccgggttgattaggaggaaga

SEQ ID NO: 1149 - DNA, 31 bp, Artificial
  synthetic sequence
ttgcaaaataacatttgtaatcccaatttcc

SEQ ID NO: 1150 - DNA, 19 bp, Artificial
  synthetic sequence
aagagggcagagtatgccg

SEQ ID NO: 1151 - DNA, 23 bp, Artificial
  synthetic sequence
atgccctggattatcccaatgaa

SEQ ID NO: 1152 - DNA, 26 bp, Artificial
  synthetic sequence
ttcaatgcctcataatgcatctgatc

SEQ ID NO: 1153 - DNA, 23 bp, Artificial
  synthetic sequence
tcaacagcttgagtagtctcgtc

SEQ ID NO: 1154 - DNA, 22 bp, Artificial
  synthetic sequence
ttctgcagtaactgcagggtac

SEQ ID NO: 1155 - DNA, 23 bp, Artificial
  synthetic sequence
acggaatgttttccgcaatcgtt

SEQ ID NO: 1156 - DNA, 21 bp, Artificial
  synthetic sequence
cagggcataagaggcataagc

SEQ ID NO: 1157 - DNA, 18 bp, Artificial
  synthetic sequence
tgcagcatcacctgctga

SEQ ID NO: 1158 - DNA, 17 bp, Artificial
  synthetic sequence
gctgttgaagggctcgg

SEQ ID NO: 1159 - DNA, 30 bp, Artificial
  synthetic sequence
gcttattacgcacaatagcgaattaaaaca

SEQ ID NO: 1160 - DNA, 30 bp, Artificial
  synthetic sequence
aatagttttgtaataacaagatgcaaccag

SEQ ID NO: 1161 - DNA, 26 bp, Artificial
  synthetic sequence
aaccgaagaaggagagttaaagactt

SEQ ID NO: 1162 - DNA, 26 bp, Artificial
  synthetic sequence
cggtagtggtggtgttatcgttaaat

SEQ ID NO: 1163 - DNA, 27 bp, Artificial
  synthetic sequence
caggttgagggccatctaaataattca

SEQ ID NO: 1164 - DNA, 33 bp, Artificial
  synthetic sequence
attgacaaaatcatagttaaaaactcctttgaa

SEQ ID NO: 1165 - DNA, 24 bp, Artificial
  synthetic sequence
tttactaccatcgcgccgatattt

SEQ ID NO: 1166 - DNA, 17 bp, Artificial
  synthetic sequence
atcgccgcgttttgcgt

SEQ ID NO: 1167 - DNA, 19 bp, Artificial
  synthetic sequence
aaacggctcatctgcgtca

SEQ ID NO: 1168 - DNA, 23 bp, Artificial
  synthetic sequence
gttgcaccgtaaaagagaggact

SEQ ID NO: 1169 - DNA, 27 bp, Artificial
  synthetic sequence
aacctagccatactagtatagtccctt

SEQ ID NO: 1170 - DNA, 26 bp, Artificial
  synthetic sequence
gagttggtatcaggagatgaagaagc

SEQ ID NO: 1171 - DNA, 27 bp, Artificial
  synthetic sequence
ctgcaaacacatcaaaataaaaggcag

SEQ ID NO: 1172 - DNA, 31 bp, Artificial
  synthetic sequence
tgccaaaaataagatacaccttcctataaga

SEQ ID NO: 1173 - DNA, 26 bp, Artificial
  synthetic sequence
accaactctatatcggcaaaatttgt

SEQ ID NO: 1174 - DNA, 19 bp, Artificial
  synthetic sequence
acctgagggtgacgacttg

SEQ ID NO: 1175 - DNA, 25 bp, Artificial
  synthetic sequence
tgtccctcaacctaatttttggctt

SEQ ID NO: 1176 - DNA, 23 bp, Artificial
  synthetic sequence
gtttgcagataggtgttcaagca

SEQ ID NO: 1177 - DNA, 23 bp, Artificial
  synthetic sequence
gtttggctcaggaagagaaacct

SEQ ID NO: 1178 - DNA, 27 bp, Artificial
  synthetic sequence
gatactaccatcgctagaaacacagaa

SEQ ID NO: 1179 - DNA, 23 bp, Artificial
  synthetic sequence
gcaaaggcagaggtggacattac

SEQ ID NO: 1180 - DNA, 20 bp, Artificial
  synthetic sequence
tcaaacgaacagcctgttcc

SEQ ID NO: 1181 - DNA, 22 bp, Artificial
  synthetic sequence
tcgtttgacgaataacatgccg

SEQ ID NO: 1182 - DNA, 28 bp, Artificial
  synthetic sequence
agagcctatcatagaagacatcaatagc

SEQ ID NO: 1183 - DNA, 22 bp, Artificial
  synthetic sequence
agcacctaccttctggatgatc

SEQ ID NO: 1184 - DNA, 18 bp, Artificial
  synthetic sequence
agcagcacaggtcctgtt

SEQ ID NO: 1185 - DNA, 27 bp, Artificial
  synthetic sequence
ggatagcatggtgcatgttacagatat

SEQ ID NO: 1186 - DNA, 21 bp, Artificial
  synthetic sequence
gttccacaagagagatgggca

SEQ ID NO: 1187 - DNA, 21 bp, Artificial
  synthetic sequence
tttgggcagtaacctctaggg

SEQ ID NO: 1188 - DNA, 25 bp, Artificial
  synthetic sequence
tgccctagaagccatttatgacaaa

SEQ ID NO: 1189 - DNA, 24 bp, Artificial
  synthetic sequence
actgatatgcacgccatagatcac

SEQ ID NO: 1190 - DNA, 25 bp, Artificial
  synthetic sequence
ccaaagcattttaaccgaaaatggt

SEQ ID NO: 1191 - DNA, 17 bp, Artificial
  synthetic sequence
ggcgttgataccccagc

SEQ ID NO: 1192 - DNA, 32 bp, Artificial
  synthetic sequence
ttgtcagtctatattgtgagatgtttctcaaa

SEQ ID NO: 1193 - DNA, 23 bp, Artificial
  synthetic sequence
tggtccaacagctgtttctactt

SEQ ID NO: 1194 - DNA, 32 bp, Artificial
  synthetic sequence
atgaagcaaaagaaaaattattagcacaacaa

SEQ ID NO: 1195 - DNA, 26 bp, Artificial
  synthetic sequence
tttttgaggctaactttgccatttct

SEQ ID NO: 1196 - DNA, 21 bp, Artificial
  synthetic sequence
tcaacgccttctggtattccc

SEQ ID NO: 1197 - DNA, 27 bp, Artificial
  synthetic sequence
agattcggaccaagtttaactcttcaa

SEQ ID NO: 1198 - DNA, 25 bp, Artificial
  synthetic sequence
acctttagggaagtacggtattgaa

SEQ ID NO: 1199 - DNA, 23 bp, Artificial
  synthetic sequence
accaagactgctgacagcatatg

SEQ ID NO: 1200 - DNA, 19 bp, Artificial
  synthetic sequence
tgcaggcacgtatattggc

SEQ ID NO: 1201 - DNA, 19 bp, Artificial
  synthetic sequence
tgcctgcattgtgatggag

SEQ ID NO: 1202 - DNA, 22 bp, Artificial
  synthetic sequence
agacgacgtgtccaactatcag

SEQ ID NO: 1203 - DNA, 28 bp, Artificial
  synthetic sequence
cgaagcaattcaataaaacacgaaagtg

SEQ ID NO: 1204 - DNA, 23 bp, Artificial
  synthetic sequence
agttgcgtattatccagttgcga

SEQ ID NO: 1205 - DNA, 28 bp, Artificial
  synthetic sequence
cgatgaatactaagctcatactcttcgg

SEQ ID NO: 1206 - DNA, 30 bp, Artificial
  synthetic sequence
ttgcttcgaagtaagcgatatattgttttt

SEQ ID NO: 1207 - DNA, 23 bp, Artificial
  synthetic sequence
aaaattgcgacctcccgaaaaat

SEQ ID NO: 1208 - DNA, 32 bp, Artificial
  synthetic sequence
aattttctcacggatactcacattaatttcgt

SEQ ID NO: 1209 - DNA, 26 bp, Artificial
  synthetic sequence
accgataattacaccaaacaacatgg

SEQ ID NO: 1210 - DNA, 19 bp, Artificial
  synthetic sequence
cgtcgatcaacagtgcgtt

SEQ ID NO: 1211 - DNA, 24 bp, Artificial
  synthetic sequence
ccgatcacataagccacacctaac

SEQ ID NO: 1212 - DNA, 28 bp, Artificial
  synthetic sequence
gtgagtcaaatatcattgatgtgatcgt

SEQ ID NO: 1213 - DNA, 18 bp, Artificial
  synthetic sequence
tcatctggagcgacgtga

SEQ ID NO: 1214 - DNA, 25 bp, Artificial
  synthetic sequence
gaactgaccaacaaagatcaatgga

SEQ ID NO: 1215 - DNA, 23 bp, Artificial
  synthetic sequence
atccgtgccttaagtagtttgct

SEQ ID NO: 1216 - DNA, 32 bp, Artificial
  synthetic sequence
caaggaaggtataaatgatacacattatccca

SEQ ID NO: 1217 - DNA, 22 bp, Artificial
  synthetic sequence
ccttgatgcttggcttgatgtt

SEQ ID NO: 1218 - DNA, 25 bp, Artificial
  synthetic sequence
ggcaaaataagctcctaaaacatcg

SEQ ID NO: 1219 - DNA, 24 bp, Artificial
  synthetic sequence
tcctaccgtaaagctctgtgttac

SEQ ID NO: 1220 - DNA, 30 bp, Artificial
  synthetic sequence
tttattaggtttgatttttcagacctgcct

SEQ ID NO: 1221 - DNA, 33 bp, Artificial
  synthetic sequence
aggtattttctctatcctcttccctttaaaacc

SEQ ID NO: 1222 - DNA, 28 bp, Artificial
  synthetic sequence
gcaggcacttttaatattcaatgttccg

SEQ ID NO: 1223 - DNA, 20 bp, Artificial
  synthetic sequence
gaaagggtcaacattgccgt

SEQ ID NO: 1224 - DNA, 17 bp, Artificial
  synthetic sequence
gcgatcgccgtcgtgac

SEQ ID NO: 1225 - DNA, 21 bp, Artificial
  synthetic sequence
gaaggtgccgatcgagaagtg

SEQ ID NO: 1226 - DNA, 20 bp, Artificial
  synthetic sequence
accctttcaggattggcaca

SEQ ID NO: 1227 - DNA, 17 bp, Artificial
  synthetic sequence
ataaccggcgcggtctt

SEQ ID NO: 1228 - DNA, 18 bp, Artificial
  synthetic sequence
acctccgtgacagaggga

SEQ ID NO: 1229 - DNA, 23 bp, Artificial
  synthetic sequence
cgatcatcacgtttgaggctttg

SEQ ID NO: 1230 - DNA, 23 bp, Artificial
  synthetic sequence
tatgaatcttagcgcacgcaatc

SEQ ID NO: 1231 - DNA, 25 bp, Artificial
  synthetic sequence
gactcagattttcaacccctgtctg

SEQ ID NO: 1232 - DNA, 32 bp, Artificial
  synthetic sequence
tgctttatacgcataaaaataagcttaattca

SEQ ID NO: 1233 - DNA, 20 bp, Artificial
  synthetic sequence
atactccagggcacttgccg

SEQ ID NO: 1234 - DNA, 29 bp, Artificial
  synthetic sequence
tttacccttgggcattaccgtatatacta

SEQ ID NO: 1235 - DNA, 28 bp, Artificial
  synthetic sequence
attaaggttgttgaagaaagcagaagaa

SEQ ID NO: 1236 - DNA, 24 bp, Artificial
  synthetic sequence
aataccgcctcacttactatagcc

SEQ ID NO: 1237 - DNA, 24 bp, Artificial
  synthetic sequence
ttgtcgggacttcttgattatgca

SEQ ID NO: 1238 - DNA, 25 bp, Artificial
  synthetic sequence
tcggtatcgcagctgaatttatagt

SEQ ID NO: 1239 - DNA, 22 bp, Artificial
  synthetic sequence
ctgacagggacagaaagtaacg

SEQ ID NO: 1240 - DNA, 21 bp, Artificial
  synthetic sequence
tgcaacggctttgtactcact

SEQ ID NO: 1241 - DNA, 18 bp, Artificial
  synthetic sequence
ccgatcgttccgctttca

SEQ ID NO: 1242 - DNA, 21 bp, Artificial
  synthetic sequence
gtaactatcagcggcggtact

SEQ ID NO: 1243 - DNA, 31 bp, Artificial
  synthetic sequence
acatcgatgtttttgatggctttaatattgc

SEQ ID NO: 1244 - DNA, 17 bp, Artificial
  synthetic sequence
acgatcggcggcgatat

SEQ ID NO: 1245 - DNA, 32 bp, Artificial
  synthetic sequence
gaaaagccattttatattctcctgttcttttt

SEQ ID NO: 1246 - DNA, 29 bp, Artificial
  synthetic sequence
ctgaaaaagattggtgacatcacagatat

SEQ ID NO: 1247 - DNA, 19 bp, Artificial
  synthetic sequence
gcactgcgccagataggta

SEQ ID NO: 1248 - DNA, 17 bp, Artificial
  synthetic sequence
ggctcggtttccgcgat

SEQ ID NO: 1249 - DNA, 20 bp, Artificial
  synthetic sequence
tgtaagacctgcgcgttgtg

SEQ ID NO: 1250 - DNA, 19 bp, Artificial
  synthetic sequence
gcgatagcctgacccagtt

SEQ ID NO: 1251 - DNA, 21 bp, Artificial
  synthetic sequence
gcaaaaccctctcttgcttgt

SEQ ID NO: 1252 - DNA, 23 bp, Artificial
  synthetic sequence
tggtggccttgataagagtttga

SEQ ID NO: 1253 - DNA, 26 bp, Artificial
  synthetic sequence
gctgctcttcctgtcaggtattttag

SEQ ID NO: 1254 - DNA, 20 bp, Artificial
  synthetic sequence
ggttttgcaacaagggcttc

SEQ ID NO: 1255 - DNA, 17 bp, Artificial
  synthetic sequence
gcagggctggcgatcaa

SEQ ID NO: 1256 - DNA, 26 bp, Artificial
  synthetic sequence
atgggttttaaacgcttgaaaaatgc

SEQ ID NO: 1257 - DNA, 19 bp, Artificial
  synthetic sequence
gccaaggcctctcttctca

SEQ ID NO: 1258 - DNA, 18 bp, Artificial
  synthetic sequence
agccctgcccctaattgg

SEQ ID NO: 1259 - DNA, 19 bp, Artificial
  synthetic sequence
agcaggccttttctcagga

SEQ ID NO: 1260 - DNA, 22 bp, Artificial
  synthetic sequence
ggagcaacttgttagcagatgg

SEQ ID NO: 1261 - DNA, 19 bp, Artificial
  synthetic sequence
agttgcaggttttgcgagt

SEQ ID NO: 1262 - DNA, 26 bp, Artificial
  synthetic sequence
tgccaaaaagccttgagaatattctg

SEQ ID NO: 1263 - DNA, 27 bp, Artificial
  synthetic sequence
ttgacgaatctatttaaaccttaccgc

SEQ ID NO: 1264 - DNA, 25 bp, Artificial
  synthetic sequence
ggcctgctactaattcacttattgc

SEQ ID NO: 1265 - DNA, 18 bp, Artificial
  synthetic sequence
acggtggtcgctgtactg

SEQ ID NO: 1266 - DNA, 17 bp, Artificial
  synthetic sequence
gcagggtgctgaccgag

SEQ ID NO: 1267 - DNA, 20 bp, Artificial
  synthetic sequence
tcagcgcgcagagaatactg

SEQ ID NO: 1268 - DNA, 17 bp, Artificial
  synthetic sequence
accaccgtaaccggctc

SEQ ID NO: 1269 - DNA, 17 bp, Artificial
  synthetic sequence
caccctgcgggctgtct

SEQ ID NO: 1270 - DNA, 20 bp, Artificial
  synthetic sequence
ggattacgcatcggatcggg

SEQ ID NO: 1271 - DNA, 21 bp, Artificial
  synthetic sequence
tgcaatcttgtgagtggcaga

SEQ ID NO: 1272 - DNA, 19 bp, Artificial
  synthetic sequence
ctcgaccaccacgaatcgc

SEQ ID NO: 1273 - DNA, 23 bp, Artificial
  synthetic sequence
caatcttcggcgttttgctgtat

SEQ ID NO: 1274 - DNA, 24 bp, Artificial
  synthetic sequence
gttgaagatgacatgagcgttgac

SEQ ID NO: 1275 - DNA, 18 bp, Artificial
  synthetic sequence
cgccagcgaaggctattt

SEQ ID NO: 1276 - DNA, 21 bp, Artificial
  synthetic sequence
gtggtggatgttcctctggtg

SEQ ID NO: 1277 - DNA, 24 bp, Artificial
  synthetic sequence
cgtagccaaaactaatccggattg

SEQ ID NO: 1278 - DNA, 28 bp, Artificial
  synthetic sequence
catttggacttaagaggtattgcgattt

SEQ ID NO: 1279 - DNA, 26 bp, Artificial
  synthetic sequence
gcattaagagcaaatcactgggaatt

SEQ ID NO: 1280 - DNA, 30 bp, Artificial
  synthetic sequence
acgattattttaaaagcgttagaagaagcc

SEQ ID NO: 1281 - DNA, 24 bp, Artificial
  synthetic sequence
gttgttgtaaatgccatgggttcc

SEQ ID NO: 1282 - DNA, 28 bp, Artificial
  synthetic sequence
tctgaagtactagttgcagtgattcaac

SEQ ID NO: 1283 - DNA, 30 bp, Artificial
  synthetic sequence
cttaaagaaagtcataatcctcaccttccc

SEQ ID NO: 1284 - DNA, 24 bp, Artificial
  synthetic sequence
gcgtttgggtttatgagcttgaaa

SEQ ID NO: 1285 - DNA, 33 bp, Artificial
  synthetic sequence
ataaagaagcatatggtgaaaaataaaactctg

SEQ ID NO: 1286 - DNA, 19 bp, Artificial
  synthetic sequence
ggcatttgcgcccatactg

SEQ ID NO: 1287 - DNA, 21 bp, Artificial
  synthetic sequence
gtcgagtacgacttgcgagaa

SEQ ID NO: 1288 - DNA, 32 bp, Artificial
  synthetic sequence
gagtcacctatataagcatcactctataagat

SEQ ID NO: 1289 - DNA, 19 bp, Artificial
  synthetic sequence
tcgtcggttctggcctact

SEQ ID NO: 1290 - DNA, 25 bp, Artificial
  synthetic sequence
gagaagcgacgacatgattaactct

SEQ ID NO: 1291 - DNA, 18 bp, Artificial
  synthetic sequence
cgccacggcaatggtttc

SEQ ID NO: 1292 - DNA, 21 bp, Artificial
  synthetic sequence
gcgcaaacgtggttaatggta

SEQ ID NO: 1293 - DNA, 19 bp, Artificial
  synthetic sequence
cgttatgtcgggcgaacca

SEQ ID NO: 1294 - DNA, 26 bp, Artificial
  synthetic sequence
gcaatcatggaaaacatcaacgtcat

SEQ ID NO: 1295 - DNA, 21 bp, Artificial
  synthetic sequence
cttcaccgccatttccgtaac

SEQ ID NO: 1296 - DNA, 21 bp, Artificial
  synthetic sequence
ccacaccgttagcagcaatca

SEQ ID NO: 1297 - DNA, 19 bp, Artificial
  synthetic sequence
gacccatccggctgatacc

SEQ ID NO: 1298 - DNA, 21 bp, Artificial
  synthetic sequence
ccgtgctcggcaattttacat

SEQ ID NO: 1299 - DNA, 17 bp, Artificial
  synthetic sequence
cgcattggtgagctggc

SEQ ID NO: 1300 - DNA, 18 bp, Artificial
  synthetic sequence
gacagcaactcgcggatc

SEQ ID NO: 1301 - DNA, 22 bp, Artificial
  synthetic sequence
tccgtatcgatcctgaacacca

SEQ ID NO: 1302 - DNA, 17 bp, Artificial
  synthetic sequence
gccactcgccccttgtt

SEQ ID NO: 1303 - DNA, 18 bp, Artificial
  synthetic sequence
gtacccaacgggccgttt

SEQ ID NO: 1304 - DNA, 17 bp, Artificial
  synthetic sequence
cagatggtgcccagacg

SEQ ID NO: 1305 - DNA, 17 bp, Artificial
  synthetic sequence
gcctcgcgcgagggatt

SEQ ID NO: 1306 - DNA, 18 bp, Artificial
  synthetic sequence
accttggtcgaggccgct

SEQ ID NO: 1307 - DNA, 26 bp, Artificial
  synthetic sequence
acaagaaaggagcgataactttggtt

SEQ ID NO: 1308 - DNA, 31 bp, Artificial
  synthetic sequence
ctcatcaatatttaaagctctttgttcagct

SEQ ID NO: 1309 - DNA, 31 bp, Artificial
  synthetic sequence
tggatattaaaagtaaaactagctgatgtgg

SEQ ID NO: 1310 - DNA, 27 bp, Artificial
  synthetic sequence
atcatgttatccctcccaatttgttct

SEQ ID NO: 1311 - DNA, 32 bp, Artificial
  synthetic sequence
ttgatgagatatcaacggaaataactagtatg

SEQ ID NO: 1312 - DNA, 30 bp, Artificial
  synthetic sequence
aatttctcaccctagtaaatactgtttctc

SEQ ID NO: 1313 - DNA, 24 bp, Artificial
  synthetic sequence
gctccttgagtataaccattggtc

SEQ ID NO: 1314 - DNA, 24 bp, Artificial
  synthetic sequence
tcagatgaaacaaaagcggctttc

SEQ ID NO: 1315 - DNA, 33 bp, Artificial
  synthetic sequence
gaaattcacttcatcaattataccataaaccat

SEQ ID NO: 1316 - DNA, 21 bp, Artificial
  synthetic sequence
gctgttgcaactgctttgtca

SEQ ID NO: 1317 - DNA, 27 bp, Artificial
  synthetic sequence
tctaaggcaattgcttttatcattggg

SEQ ID NO: 1318 - DNA, 33 bp, Artificial
  synthetic sequence
tttctgaaattctcttttatgtcattttaggac

SEQ ID NO: 1319 - DNA, 28 bp, Artificial
  synthetic sequence
gaattctacaaccatcttcaccacttca

SEQ ID NO: 1320 - DNA, 26 bp, Artificial
  synthetic sequence
attcgctgatttttcaggtatttgct

SEQ ID NO: 1321 - DNA, 18 bp, Artificial
  synthetic sequence
cgcctatgttcaggcagc

SEQ ID NO: 1322 - DNA, 18 bp, Artificial
  synthetic sequence
cgtcactcgattccccgt

SEQ ID NO: 1323 - DNA, 22 bp, Artificial
  synthetic sequence
gagtgacggaatcttttacccc

SEQ ID NO: 1324 - DNA, 19 bp, Artificial
  synthetic sequence
gagcctctgggttctgctg

SEQ ID NO: 1325 - DNA, 32 bp, Artificial
  synthetic sequence
caaaaccaattaaagagttagagcaacatatg

SEQ ID NO: 1326 - DNA, 31 bp, Artificial
  synthetic sequence
aaatgtggattaatttgactgtaaagtgcat

SEQ ID NO: 1327 - DNA, 31 bp, Artificial
  synthetic sequence
tcctatcaagaatactcattggacattgatt

SEQ ID NO: 1328 - DNA, 30 bp, Artificial
  synthetic sequence
tggttttgtaattcttctcaatacactgat

SEQ ID NO: 1329 - DNA, 23 bp, Artificial
  synthetic sequence
caacctttagcctcgccatagaa

SEQ ID NO: 1330 - DNA, 29 bp, Artificial
  synthetic sequence
acctttgaaaatacaacagaggtgataaa

SEQ ID NO: 1331 - DNA, 18 bp, Artificial
  synthetic sequence
gagtcgacaaccgtctgc

SEQ ID NO: 1332 - DNA, 29 bp, Artificial
  synthetic sequence
cgagtatctgctgaaatgagtgatataac

SEQ ID NO: 1333 - DNA, 18 bp, Artificial
  synthetic sequence
agctaaggcgccttgcaa

SEQ ID NO: 1334 - DNA, 25 bp, Artificial
  synthetic sequence
gtcttcacctttagaatccatcgct

SEQ ID NO: 1335 - DNA, 31 bp, Artificial
  synthetic sequence
tgcaaagctaagcaatttagtcaagctttta

SEQ ID NO: 1336 - DNA, 26 bp, Artificial
  synthetic sequence
gcaatgttgatactttgtcttcacct

SEQ ID NO: 1337 - DNA, 31 bp, Artificial
  synthetic sequence
ttcaaaaacatatcttctagatcttcttggt

SEQ ID NO: 1338 - DNA, 28 bp, Artificial
  synthetic sequence
atggccaccataattttgcttttaaagg

SEQ ID NO: 1339 - DNA, 17 bp, Artificial
  synthetic sequence
gccctccgcatcgctgt

SEQ ID NO: 1340 - DNA, 21 bp, Artificial
  synthetic sequence
acgtataccaggctcaaggct

SEQ ID NO: 1341 - DNA, 17 bp, Artificial
  synthetic sequence
tcgcccaggtgctctcc

SEQ ID NO: 1342 - DNA, 17 bp, Artificial
  synthetic sequence
gggttggtggaacgcga

SEQ ID NO: 1343 - DNA, 18 bp, Artificial
  synthetic sequence
gccgcagccgaactggtt

SEQ ID NO: 1344 - DNA, 17 bp, Artificial
  synthetic sequence
accgcgaactcgggtgg

SEQ ID NO: 1345 - DNA, 17 bp, Artificial
  synthetic sequence
ttcgcggtcgacaccaa

SEQ ID NO: 1346 - DNA, 21 bp, Artificial
  synthetic sequence
gagttgaggtgctgatcaacg

SEQ ID NO: 1347 - DNA, 23 bp, Artificial
  synthetic sequence
gtgagcgaatcaagaaagttcgt

SEQ ID NO: 1348 - DNA, 26 bp, Artificial
  synthetic sequence
agaagctagtgtatacactgcttgtc

SEQ ID NO: 1349 - DNA, 26 bp, Artificial
  synthetic sequence
tatagttggcgtggagcaaaaattga

SEQ ID NO: 1350 - DNA, 32 bp, Artificial
  synthetic sequence
attttaatattttccccagtatctttagtgca

SEQ ID NO: 1351 - DNA, 28 bp, Artificial
  synthetic sequence
aaggtctaaattttgtccatctagcatg

SEQ ID NO: 1352 - DNA, 26 bp, Artificial
  synthetic sequence
tgctttctcaaaaaggatctcaaggt

SEQ ID NO: 1353 - DNA, 28 bp, Artificial
  synthetic sequence
aaaacgaaaacgaaaaagatgaaggttt

SEQ ID NO: 1354 - DNA, 28 bp, Artificial
  synthetic sequence
tctctcataaaaacgcataccactaagt

SEQ ID NO: 1355 - DNA, 29 bp, Artificial
  synthetic sequence
agaaagcatcaaaaccaataaaggatcag

SEQ ID NO: 1356 - DNA, 28 bp, Artificial
  synthetic sequence
tgctataaaagatggagaacgctatagt

SEQ ID NO: 1357 - DNA, 32 bp, Artificial
  synthetic sequence
aataaggttttgattgcaaaattctttaggaa

SEQ ID NO: 1358 - DNA, 23 bp, Artificial
  synthetic sequence
ccactttagacataggtggtggt

SEQ ID NO: 1359 - DNA, 19 bp, Artificial
  synthetic sequence
agccgcaaatgaatacggc

SEQ ID NO: 1360 - DNA, 19 bp, Artificial
  synthetic sequence
ccatggagctggttggttg

SEQ ID NO: 1361 - DNA, 25 bp, Artificial
  synthetic sequence
ggtataaatggatcgtacgtttcga

SEQ ID NO: 1362 - DNA, 22 bp, Artificial
  synthetic sequence
tccgccaacaaaacctatgtct

SEQ ID NO: 1363 - DNA, 20 bp, Artificial
  synthetic sequence
ggcaaccacttccggaattt

SEQ ID NO: 1364 - DNA, 17 bp, Artificial
  synthetic sequence
ttgcggctggatgaggt

SEQ ID NO: 1365 - DNA, 29 bp, Artificial
  synthetic sequence
gggatggacaattattttatggattctga

SEQ ID NO: 1366 - DNA, 17 bp, Artificial
  synthetic sequence
ctggccagtaacggcga

SEQ ID NO: 1367 - DNA, 24 bp, Artificial
  synthetic sequence
agtattttggctcaccaagcatca

SEQ ID NO: 1368 - DNA, 21 bp, Artificial
  synthetic sequence
tgccattgatccacctcactt

SEQ ID NO: 1369 - DNA, 32 bp, Artificial
  synthetic sequence
attatgattattggtggaggatggtatactgt

SEQ ID NO: 1370 - DNA, 21 bp, Artificial
  synthetic sequence
aattacgccaacgtacccacc

SEQ ID NO: 1371 - DNA, 20 bp, Artificial
  synthetic sequence
ctggccagtattttggcggt

SEQ ID NO: 1372 - DNA, 26 bp, Artificial
  synthetic sequence
acagttgaggctgagagaaaactttg

SEQ ID NO: 1373 - DNA, 18 bp, Artificial
  synthetic sequence
gccaatccccgtcatagc

SEQ ID NO: 1374 - DNA, 19 bp, Artificial
  synthetic sequence
gatccggcggctgatattc

SEQ ID NO: 1375 - DNA, 18 bp, Artificial
  synthetic sequence
ccggtttttgcgcgcttc

SEQ ID NO: 1376 - DNA, 17 bp, Artificial
  synthetic sequence
gcgatggcagaagcgtt

SEQ ID NO: 1377 - DNA, 25 bp, Artificial
  synthetic sequence
aaaccttgatgattgcttttggcaa

SEQ ID NO: 1378 - DNA, 18 bp, Artificial
  synthetic sequence
agacccgtaatgccgcct

SEQ ID NO: 1379 - DNA, 17 bp, Artificial
  synthetic sequence
gccatcgctcttggcgt

SEQ ID NO: 1380 - DNA, 28 bp, Artificial
  synthetic sequence
actttggtttgaatcaagacttgatcac

SEQ ID NO: 1381 - DNA, 20 bp, Artificial
  synthetic sequence
gtgatcgtcatgtgcgatcc

SEQ ID NO: 1382 - DNA, 30 bp, Artificial
  synthetic sequence
aaggatggatcaaccgttatccttaataaa

SEQ ID NO: 1383 - DNA, 23 bp, Artificial
  synthetic sequence
gctggttcaggtattacaactgc

SEQ ID NO: 1384 - DNA, 29 bp, Artificial
  synthetic sequence
gcgattacgatttgaaaagttctcacttt

SEQ ID NO: 1385 - DNA, 23 bp, Artificial
  synthetic sequence
ttattgcagggtatggtagccag

SEQ ID NO: 1386 - DNA, 20 bp, Artificial
  synthetic sequence
ctccacctagtccctgtccg

SEQ ID NO: 1387 - DNA, 20 bp, Artificial
  synthetic sequence
aaatcaccctggtggagcga

SEQ ID NO: 1388 - DNA, 23 bp, Artificial
  synthetic sequence
ctactgccttcttccgggaaaat

SEQ ID NO: 1389 - DNA, 24 bp, Artificial
  synthetic sequence
taatgacgagatgcgtttggacag

SEQ ID NO: 1390 - DNA, 33 bp, Artificial
  synthetic sequence
ctgaattaaatttagtgcattttctagcaaagc

SEQ ID NO: 1391 - DNA, 24 bp, Artificial
  synthetic sequence
cggtttaaacgatgctactctcga

SEQ ID NO: 1392 - DNA, 29 bp, Artificial
  synthetic sequence
tttcagcataccaaagtggatatttccat

SEQ ID NO: 1393 - DNA, 17 bp, Artificial
  synthetic sequence
gcagcgaaagtccgtcg

SEQ ID NO: 1394 - DNA, 17 bp, Artificial
  synthetic sequence
atatccgcgctgcgctg

SEQ ID NO: 1395 - DNA, 17 bp, Artificial
  synthetic sequence
ctgatgcgtgccgtgcc

SEQ ID NO: 1396 - DNA, 18 bp, Artificial
  synthetic sequence
agaacagcgcatgcgctc

SEQ ID NO: 1397 - DNA, 24 bp, Artificial
  synthetic sequence
caaaccacttgttcaacttccctg

SEQ ID NO: 1398 - DNA, 21 bp, Artificial
  synthetic sequence
gtcagcaatgtaaccgtcagg

SEQ ID NO: 1399 - DNA, 19 bp, Artificial
  synthetic sequence
aggcatgagcatgaaacgc

SEQ ID NO: 1400 - DNA, 19 bp, Artificial
  synthetic sequence
ggtggaactgaccgtaggc

SEQ ID NO: 1401 - DNA, 18 bp, Artificial
  synthetic sequence
tttggccacagcatggga

SEQ ID NO: 1402 - DNA, 26 bp, Artificial
  synthetic sequence
aaaatgcttcttgttccagttcatcc

SEQ ID NO: 1403 - DNA, 18 bp, Artificial
  synthetic sequence
cccggtcgtgtttatggg

SEQ ID NO: 1404 - DNA, 18 bp, Artificial
  synthetic sequence
tctgcgcattcatgtccg

SEQ ID NO: 1405 - DNA, 17 bp, Artificial
  synthetic sequence
ccggagggagtggagtt

SEQ ID NO: 1406 - DNA, 22 bp, Artificial
  synthetic sequence
cccttacccgtatctttcacgg

SEQ ID NO: 1407 - DNA, 27 bp, Artificial
  synthetic sequence
gaggaaaaggcggagtttatagatctg

SEQ ID NO: 1408 - DNA, 20 bp, Artificial
  synthetic sequence
ccctccggcatcatcaattg

SEQ ID NO: 1409 - DNA, 24 bp, Artificial
  synthetic sequence
tgcgcagattcaggatatttgtgc

SEQ ID NO: 1410 - DNA, 31 bp, Artificial
  synthetic sequence
ccagatacgctttattataataattctcgcc

SEQ ID NO: 1411 - DNA, 21 bp, Artificial
  synthetic sequence
ccgcaacctggtcttaaagag

SEQ ID NO: 1412 - DNA, 19 bp, Artificial
  synthetic sequence
ttggcgcttcagccagtat

SEQ ID NO: 1413 - DNA, 17 bp, Artificial
  synthetic sequence
gtgcccgctgaaacgga

SEQ ID NO: 1414 - DNA, 18 bp, Artificial
  synthetic sequence
ccggtcaagttccgggca

SEQ ID NO: 1415 - DNA, 21 bp, Artificial
  synthetic sequence
cctttaagagcagccgggatt

SEQ ID NO: 1416 - DNA, 19 bp, Artificial
  synthetic sequence
gcctgagtcaatcccgacc

SEQ ID NO: 1417 - DNA, 17 bp, Artificial
  synthetic sequence
gcgacggatgacgtcct

SEQ ID NO: 1418 - DNA, 19 bp, Artificial
  synthetic sequence
ggatgttgctagctagcgg

SEQ ID NO: 1419 - DNA, 17 bp, Artificial
  synthetic sequence
cgcgcgaaatgctgaga

SEQ ID NO: 1420 - DNA, 17 bp, Artificial
  synthetic sequence
ggtgaagcgatggcgaa

SEQ ID NO: 1421 - DNA, 18 bp, Artificial
  synthetic sequence
gcttcaccgaatccgtcg

SEQ ID NO: 1422 - DNA, 33 bp, Artificial
  synthetic sequence
tttagcatctattgaaaatagtaggatttcacc

SEQ ID NO: 1423 - DNA, 26 bp, Artificial
  synthetic sequence
ggtttgatggcaaaaatttgtgtggt

SEQ ID NO: 1424 - DNA, 30 bp, Artificial
  synthetic sequence
agttaattgtggctttagctaggataaatt

SEQ ID NO: 1425 - DNA, 23 bp, Artificial
  synthetic sequence
tgtaagcggcgttgtatttgtcc

SEQ ID NO: 1426 - DNA, 21 bp, Artificial
  synthetic sequence
ccaataccagtccagtgcagc

SEQ ID NO: 1427 - DNA, 26 bp, Artificial
  synthetic sequence
cattatcaacggttttcagcgtgtag

SEQ ID NO: 1428 - DNA, 26 bp, Artificial
  synthetic sequence
aagaaagtaaaccttactatcacggc

SEQ ID NO: 1429 - DNA, 26 bp, Artificial
  synthetic sequence
taggtcctatattccccagactcaaa

SEQ ID NO: 1430 - DNA, 28 bp, Artificial
  synthetic sequence
agtagttttgtctactcttggagtagtg

SEQ ID NO: 1431 - DNA, 32 bp, Artificial
  synthetic sequence
tattgattcaagttttgtgaagagagaaaaac

SEQ ID NO: 1432 - DNA, 27 bp, Artificial
  synthetic sequence
aggacctatacttgcaatttaaacgac

SEQ ID NO: 1433 - DNA, 23 bp, Artificial
  synthetic sequence
ggaactcacgaactgaccaaaga

SEQ ID NO: 1434 - DNA, 32 bp, Artificial
  synthetic sequence
cagatttaataaaagcatccccatttttagcc

SEQ ID NO: 1435 - DNA, 29 bp, Artificial
  synthetic sequence
gcgcccattccaactaatacattatcttc

SEQ ID NO: 1436 - DNA, 30 bp, Artificial
  synthetic sequence
ccaatgtacaggataactctgtattacacg

SEQ ID NO: 1437 - DNA, 29 bp, Artificial
  synthetic sequence
aaaagaagcggatagttgagttaatcagc

SEQ ID NO: 1438 - DNA, 25 bp, Artificial
  synthetic sequence
cacttgtggactgtagaatatggca

SEQ ID NO: 1439 - DNA, 19 bp, Artificial
  synthetic sequence
gctggatggcggtatcact

SEQ ID NO: 1440 - DNA, 21 bp, Artificial
  synthetic sequence
gagcatcaatccatgtcggat

SEQ ID NO: 1441 - DNA, 17 bp, Artificial
  synthetic sequence
tgatgctccgccaccca

SEQ ID NO: 1442 - DNA, 19 bp, Artificial
  synthetic sequence
aggtgtctacggcactcac

SEQ ID NO: 1443 - DNA, 33 bp, Artificial
  synthetic sequence
aacttgaaaaagcaaaagatacaagagttaatg

SEQ ID NO: 1444 - DNA, 33 bp, Artificial
  synthetic sequence
agcttatactaacgataataaaaattaacccga

SEQ ID NO: 1445 - DNA, 28 bp, Artificial
  synthetic sequence
agaaagcccaacggtataaacattacaa

SEQ ID NO: 1446 - DNA, 33 bp, Artificial
  synthetic sequence
caatcgctgtctcttacttcatttattttatga

SEQ ID NO: 1447 - DNA, 17 bp, Artificial
  synthetic sequence
cggcgtgatcagcgcca

SEQ ID NO: 1448 - DNA, 22 bp, Artificial
  synthetic sequence
ggttgctgtgcctcttatgtgg

SEQ ID NO: 1449 - DNA, 29 bp, Artificial
  synthetic sequence
agctttatacaaaagcatatctgctcctt

SEQ ID NO: 1450 - DNA, 25 bp, Artificial
  synthetic sequence
ctttaacgaacgtgttcgctaaaaa

SEQ ID NO: 1451 - DNA, 21 bp, Artificial
  synthetic sequence
agctcgttctcattcagcaga

SEQ ID NO: 1452 - DNA, 20 bp, Artificial
  synthetic sequence
actcaggaagctttggcaga

SEQ ID NO: 1453 - DNA, 32 bp, Artificial
  synthetic sequence
cctccatataccaacttaaatactaaacatgt

SEQ ID NO: 1454 - DNA, 24 bp, Artificial
  synthetic sequence
cccaagaatattttgccaaggtca

SEQ ID NO: 1455 - DNA, 23 bp, Artificial
  synthetic sequence
tcttgggctatacccatagacct

SEQ ID NO: 1456 - DNA, 30 bp, Artificial
  synthetic sequence
gagtcgataataaagaggcttttaagtgat

SEQ ID NO: 1457 - DNA, 26 bp, Artificial
  synthetic sequence
agccactttttgttcgtcttagtact

SEQ ID NO: 1458 - DNA, 28 bp, Artificial
  synthetic sequence
attcagcatatttaccacttgcaatgtt

SEQ ID NO: 1459 - DNA, 28 bp, Artificial
  synthetic sequence
tggatggattttatgatgcttatccaca

SEQ ID NO: 1460 - DNA, 24 bp, Artificial
  synthetic sequence
aagtggctttttagttccttctgc

SEQ ID NO: 1461 - DNA, 18 bp, Artificial
  synthetic sequence
cacaagggtcgccgcgtc

SEQ ID NO: 1462 - DNA, 20 bp, Artificial
  synthetic sequence
ccgcgaaatacggcgaactg

SEQ ID NO: 1463 - DNA, 33 bp, Artificial
  synthetic sequence
aaacataaacgatggaaaacagattatggaaaa

SEQ ID NO: 1464 - DNA, 29 bp, Artificial
  synthetic sequence
taagaaattaacggaaggagatgaaacac

SEQ ID NO: 1465 - DNA, 19 bp, Artificial
  synthetic sequence
tcaatgtaccggtgggcaa

SEQ ID NO: 1466 - DNA, 25 bp, Artificial
  synthetic sequence
acagacagcctaattaacgtagtcc

SEQ ID NO: 1467 - DNA, 17 bp, Artificial
  synthetic sequence
ttcggaaccatccggca

SEQ ID NO: 1468 - DNA, 22 bp, Artificial
  synthetic sequence
ccatgcagaaaaaccgattccg

SEQ ID NO: 1469 - DNA, 23 bp, Artificial
  synthetic sequence
gccattgcgcatcgtcaaaaata

SEQ ID NO: 1470 - DNA, 23 bp, Artificial
  synthetic sequence
cattgcaggcaaggaatgaagag

SEQ ID NO: 1471 - DNA, 23 bp, Artificial
  synthetic sequence
taagccgaaatctgaatgaccga

SEQ ID NO: 1472 - DNA, 24 bp, Artificial
  synthetic sequence
cagctgatggatgagatgatcgaa

SEQ ID NO: 1473 - DNA, 20 bp, Artificial
  synthetic sequence
ccttaacggcaaccacgatg

SEQ ID NO: 1474 - DNA, 17 bp, Artificial
  synthetic sequence
gcgcttccagcatgcca

SEQ ID NO: 1475 - DNA, 23 bp, Artificial
  synthetic sequence
ccggtatgggaataggaaaaagc

SEQ ID NO: 1476 - DNA, 18 bp, Artificial
  synthetic sequence
atgcccccgcgcaaaatc

SEQ ID NO: 1477 - DNA, 25 bp, Artificial
  synthetic sequence
ccagcactccgactatagatttagt

SEQ ID NO: 1478 - DNA, 28 bp, Artificial
  synthetic sequence
aatacaaaagtattctgatgacggagag

SEQ ID NO: 1479 - DNA, 28 bp, Artificial
  synthetic sequence
agctactgatccccaaagtaaaattctc

SEQ ID NO: 1480 - DNA, 22 bp, Artificial
  synthetic sequence
cggacaacgaagtccgttgttt

SEQ ID NO: 1481 - DNA, 17 bp, Artificial
  synthetic sequence
agcgtaccggaagctcg

SEQ ID NO: 1482 - DNA, 17 bp, Artificial
  synthetic sequence
gtcggcaatgccggcac

SEQ ID NO: 1483 - DNA, 22 bp, Artificial
  synthetic sequence
ggccgaatatgtttcgcggata

SEQ ID NO: 1484 - DNA, 20 bp, Artificial
  synthetic sequence
gcgaggtcaagatatacggc

SEQ ID NO: 1485 - DNA, 18 bp, Artificial
  synthetic sequence
cgccaccccacctcaatt

SEQ ID NO: 1486 - DNA, 18 bp, Artificial
  synthetic sequence
acccccgttgcgcacatt

SEQ ID NO: 1487 - DNA, 26 bp, Artificial
  synthetic sequence
gtcagattctctgcataatttttccg

SEQ ID NO: 1488 - DNA, 20 bp, Artificial
  synthetic sequence
agcgtcaatcaggatgaggt

SEQ ID NO: 1489 - DNA, 19 bp, Artificial
  synthetic sequence
ttgacgctgtcatcctgct

SEQ ID NO: 1490 - DNA, 21 bp, Artificial
  synthetic sequence
aaaaatcgaggatctgctgcg

SEQ ID NO: 1491 - DNA, 33 bp, Artificial
  synthetic sequence
gagaagataagtacctaaatctgaaagaaacgc

SEQ ID NO: 1492 - DNA, 27 bp, Artificial
  synthetic sequence
caatgaaaactggatcacccttctgat

SEQ ID NO: 1493 - DNA, 26 bp, Artificial
  synthetic sequence
aaggatgtgtccaacatgaatcagga

SEQ ID NO: 1494 - DNA, 28 bp, Artificial
  synthetic sequence
tcaagaaatactgtctttcttctgaccg

SEQ ID NO: 1495 - DNA, 24 bp, Artificial
  synthetic sequence
gaagccaatcctggtcctggttta

SEQ ID NO: 1496 - DNA, 33 bp, Artificial
  synthetic sequence
aaatgggaaataaacttcatgaatacctcctat

SEQ ID NO: 1497 - DNA, 28 bp, Artificial
  synthetic sequence
agtcattatgaaggagaccaatttcgac

SEQ ID NO: 1498 - DNA, 20 bp, Artificial
  synthetic sequence
gggcggatagatttccggca

SEQ ID NO: 1499 - DNA, 17 bp, Artificial
  synthetic sequence
atccgcccagcttagcc

SEQ ID NO: 1500 - DNA, 27 bp, Artificial
  synthetic sequence
ctgattttgtagagaatccctcgttga

SEQ ID NO: 1501 - DNA, 20 bp, Artificial
  synthetic sequence
aaccttgcacatcgaagagg

SEQ ID NO: 1502 - DNA, 33 bp, Artificial
  synthetic sequence
attgctttatcgttactgaaattcataatcttc

SEQ ID NO: 1503 - DNA, 26 bp, Artificial
  synthetic sequence
agacaattcttggcaaacaattctgg

SEQ ID NO: 1504 - DNA, 23 bp, Artificial
  synthetic sequence
gcaaggttcctacgaaatcaagc

SEQ ID NO: 1505 - DNA, 18 bp, Artificial
  synthetic sequence
accctccttaccccacca

SEQ ID NO: 1506 - DNA, 26 bp, Artificial
  synthetic sequence
aacaggcgaaggaaaaatgtacttac

SEQ ID NO: 1507 - DNA, 19 bp, Artificial
  synthetic sequence
agcgtcgacgctctatcca

SEQ ID NO: 1508 - DNA, 20 bp, Artificial
  synthetic sequence
aggagggtgaacgttttggt

SEQ ID NO: 1509 - DNA, 31 bp, Artificial
  synthetic sequence
aaacagaagaacaaattcaaatgcgtaacaa

SEQ ID NO: 1510 - DNA, 23 bp, Artificial
  synthetic sequence
tttgcatggtattctagctcagc

SEQ ID NO: 1511 - DNA, 33 bp, Artificial
  synthetic sequence
ggatatgtataatctcaatccacaagatatcac

SEQ ID NO: 1512 - DNA, 24 bp, Artificial
  synthetic sequence
cgacatgatatgcactcccagaga

SEQ ID NO: 1513 - DNA, 31 bp, Artificial
  synthetic sequence
ttatgcaacgaatatcctaaatacaatggat

SEQ ID NO: 1514 - DNA, 30 bp, Artificial
  synthetic sequence
aaactccattaagcataggtaatgatgaga

SEQ ID NO: 1515 - DNA, 28 bp, Artificial
  synthetic sequence
agtctaaattctaaatctagggcaacgg

SEQ ID NO: 1516 - DNA, 24 bp, Artificial
  synthetic sequence
attgccgattttcaggataagcca

SEQ ID NO: 1517 - DNA, 27 bp, Artificial
  synthetic sequence
tcggcaatatcattttgatttccttca

SEQ ID NO: 1518 - DNA, 32 bp, Artificial
  synthetic sequence
aatagttgcggattatataatcaacaatccaa

SEQ ID NO: 1519 - DNA, 18 bp, Artificial
  synthetic sequence
gagcagtcgggtgtctcc

SEQ ID NO: 1520 - DNA, 21 bp, Artificial
  synthetic sequence
gggaaatcagcccttgagatc

SEQ ID NO: 1521 - DNA, 24 bp, Artificial
  synthetic sequence
aaccgggaatgactaatcaagtgt

SEQ ID NO: 1522 - DNA, 22 bp, Artificial
  synthetic sequence
ccgattcatcaaagcatacccc

SEQ ID NO: 1523 - DNA, 28 bp, Artificial
  synthetic sequence
acaaaagaaattattggaaccattggca

SEQ ID NO: 1524 - DNA, 19 bp, Artificial
  synthetic sequence
tcccggttctaccgaaacc

SEQ ID NO: 1525 - DNA, 23 bp, Artificial
  synthetic sequence
ccggagtttgataccatgggaca

SEQ ID NO: 1526 - DNA, 19 bp, Artificial
  synthetic sequence
atacctgctgcccggttga

SEQ ID NO: 1527 - DNA, 20 bp, Artificial
  synthetic sequence
gccgcttttactggcattgt

SEQ ID NO: 1528 - DNA, 20 bp, Artificial
  synthetic sequence
tctctttttcctgtcccgca

SEQ ID NO: 1529 - DNA, 25 bp, Artificial
  synthetic sequence
ttgtttgcgtcttatactcgtgtct

SEQ ID NO: 1530 - DNA, 33 bp, Artificial
  synthetic sequence
cgataatttcttaaaatttagatgtctgacaca

SEQ ID NO: 1531 - DNA, 28 bp, Artificial
  synthetic sequence
agtcattttgcttgactgtatttttggt

SEQ ID NO: 1532 - DNA, 25 bp, Artificial
  synthetic sequence
gcaaacaaacggatttacgaagcta

SEQ ID NO: 1533 - DNA, 30 bp, Artificial
  synthetic sequence
aaaaacaaacaaatttgagagcatagagga

SEQ ID NO: 1534 - DNA, 31 bp, Artificial
  synthetic sequence
ttttgttttactttatcgtccatatcgactt

SEQ ID NO: 1535 - DNA, 17 bp, Artificial
  synthetic sequence
gtacaggctcccggcgt

SEQ ID NO: 1536 - DNA, 17 bp, Artificial
  synthetic sequence
gcttgctgcagccctcg

SEQ ID NO: 1537 - DNA, 17 bp, Artificial
  synthetic sequence
ctccaccgtcgggttgt

SEQ ID NO: 1538 - DNA, 19 bp, Artificial
  synthetic sequence
ttccaacatgttggctcgc

SEQ ID NO: 1539 - DNA, 21 bp, Artificial
  synthetic sequence
tgttggaatgcccgcttatca

SEQ ID NO: 1540 - DNA, 17 bp, Artificial
  synthetic sequence
cttacgccgtggccggt

SEQ ID NO: 1541 - DNA, 17 bp, Artificial
  synthetic sequence
cgcgcctcgtcgatctt

SEQ ID NO: 1542 - DNA, 18 bp, Artificial
  synthetic sequence
cgccgtgctttttgacga

SEQ ID NO: 1543 - DNA, 17 bp, Artificial
  synthetic sequence
gcacggcgtcaatgctt

SEQ ID NO: 1544 - DNA, 28 bp, Artificial
  synthetic sequence
tgccaacggctttatatatttctacatc

SEQ ID NO: 1545 - DNA, 24 bp, Artificial
  synthetic sequence
tcctagatttgcgatcagcgtaag

SEQ ID NO: 1546 - DNA, 17 bp, Artificial
  synthetic sequence
agccgttttacgcgctg

SEQ ID NO: 1547 - DNA, 19 bp, Artificial
  synthetic sequence
gcggcgattgagcgaaatt

SEQ ID NO: 1548 - DNA, 20 bp, Artificial
  synthetic sequence
tgggcgagagtttatcgtgc

SEQ ID NO: 1549 - DNA, 25 bp, Artificial
  synthetic sequence
ccataacggtcttactgctcttgaa

SEQ ID NO: 1550 - DNA, 28 bp, Artificial
  synthetic sequence
agttacaggtagtcccatctctatacag

SEQ ID NO: 1551 - DNA, 23 bp, Artificial
  synthetic sequence
agacttgcatgttctcctgatga

SEQ ID NO: 1552 - DNA, 24 bp, Artificial
  synthetic sequence
gatcgtaaacgtaaccacatggtc

SEQ ID NO: 1553 - DNA, 28 bp, Artificial
  synthetic sequence
ttgataatgtgtttaccaacatcaccac

SEQ ID NO: 1554 - DNA, 25 bp, Artificial
  synthetic sequence
cagacggtctcagtattgttctgat

SEQ ID NO: 1555 - DNA, 19 bp, Artificial
  synthetic sequence
accgcaacccttgtgaggt

SEQ ID NO: 1556 - DNA, 17 bp, Artificial
  synthetic sequence
aggtgctaacggcgaga

SEQ ID NO: 1557 - DNA, 25 bp, Artificial
  synthetic sequence
gatccaaagtgatgggtccatagag

SEQ ID NO: 1558 - DNA, 24 bp, Artificial
  synthetic sequence
tgcccaaaatctccaaaagattgt

SEQ ID NO: 1559 - DNA, 19 bp, Artificial
  synthetic sequence
tgctttggcttctcccact

SEQ ID NO: 1560 - DNA, 32 bp, Artificial
  synthetic sequence
cgattttatggattgcttaaaaagggttaaga

SEQ ID NO: 1561 - DNA, 27 bp, Artificial
  synthetic sequence
tgtggaacaaatgagtattctagccaa

SEQ ID NO: 1562 - DNA, 24 bp, Artificial
  synthetic sequence
ataaacatcggtcgcacgattagt

SEQ ID NO: 1563 - DNA, 28 bp, Artificial
  synthetic sequence
aaaacttatgattgacaatcgaggcatt

SEQ ID NO: 1564 - DNA, 22 bp, Artificial
  synthetic sequence
tggctgatgtttggtctgtaca

SEQ ID NO: 1565 - DNA, 25 bp, Artificial
  synthetic sequence
aaacggaagaaggagtctatcatga

SEQ ID NO: 1566 - DNA, 30 bp, Artificial
  synthetic sequence
atcctacacgactaatcattagagaaagtt

SEQ ID NO: 1567 - DNA, 17 bp, Artificial
  synthetic sequence
cgtagagccttcccggt

SEQ ID NO: 1568 - DNA, 20 bp, Artificial
  synthetic sequence
gggcaccgatgagaaaagtt

SEQ ID NO: 1569 - DNA, 22 bp, Artificial
  synthetic sequence
tgatcactccggctacaaaggt

SEQ ID NO: 1570 - DNA, 25 bp, Artificial
  synthetic sequence
tccggatatagatactattgcaccg

SEQ ID NO: 1571 - DNA, 25 bp, Artificial
  synthetic sequence
aaacgccttaaattgattcaagcga

SEQ ID NO: 1572 - DNA, 21 bp, Artificial
  synthetic sequence
gtggtgaaagtttctgtgccc

SEQ ID NO: 1573 - DNA, 27 bp, Artificial
  synthetic sequence
tcaagtttccttctaaaagtagctcgt

SEQ ID NO: 1574 - DNA, 24 bp, Artificial
  synthetic sequence
ggcgttttctggtgtttatgttct

SEQ ID NO: 1575 - DNA, 33 bp, Artificial
  synthetic sequence
aatctttgattggaaggttagaagtataaaagg

SEQ ID NO: 1576 - DNA, 29 bp, Artificial
  synthetic sequence
acgcaagattttcattcttgaaagaggag

SEQ ID NO: 1577 - DNA, 21 bp, Artificial
  synthetic sequence
ctttgcgaccacacttagctc

SEQ ID NO: 1578 - DNA, 28 bp, Artificial
  synthetic sequence
attcataagcggtcgtgacttttaactt

SEQ ID NO: 1579 - DNA, 24 bp, Artificial
  synthetic sequence
tgactcaccttcatattcaaagcc

SEQ ID NO: 1580 - DNA, 21 bp, Artificial
  synthetic sequence
acgttttgagcgatacggtcc

SEQ ID NO: 1581 - DNA, 33 bp, Artificial
  synthetic sequence
aattactcctctcttcttttaacctttgatctg

SEQ ID NO: 1582 - DNA, 31 bp, Artificial
  synthetic sequence
taccttattatgatatcgtcatcaaatcgcc

SEQ ID NO: 1583 - DNA, 28 bp, Artificial
  synthetic sequence
tctcttgatgtacttgttaataatgccg

SEQ ID NO: 1584 - DNA, 21 bp, Artificial
  synthetic sequence
agagcactattcgacgctacc

SEQ ID NO: 1585 - DNA, 18 bp, Artificial
  synthetic sequence
agtgctcttagcggacgc

SEQ ID NO: 1586 - DNA, 28 bp, Artificial
  synthetic sequence
ttctaatagacgttcacgtgatattggt

SEQ ID NO: 1587 - DNA, 24 bp, Artificial
  synthetic sequence
cttccatcctcaggtatactccag

SEQ ID NO: 1588 - DNA, 31 bp, Artificial
  synthetic sequence
tgctctgtaaatggaaaatagtccatcaaat

SEQ ID NO: 1589 - DNA, 23 bp, Artificial
  synthetic sequence
gcggtatttatgaagaacagcgt

SEQ ID NO: 1590 - DNA, 27 bp, Artificial
  synthetic sequence
cccgacaaaatttcttcaagagtatcc

SEQ ID NO: 1591 - DNA, 20 bp, Artificial
  synthetic sequence
ccgttgcaaaggctttacac

SEQ ID NO: 1592 - DNA, 20 bp, Artificial
  synthetic sequence
cggcccagtaaccagaagta

SEQ ID NO: 1593 - DNA, 23 bp, Artificial
  synthetic sequence
ggttctggtttttcgaaagcgag

SEQ ID NO: 1594 - DNA, 23 bp, Artificial
  synthetic sequence
cctgtcagcaatagttcagcact

SEQ ID NO: 1595 - DNA, 20 bp, Artificial
  synthetic sequence
cctccacaaatttgagggct

SEQ ID NO: 1596 - DNA, 29 bp, Artificial
  synthetic sequence
acaaggactatatgaagtatatgcaagcg

SEQ ID NO: 1597 - DNA, 28 bp, Artificial
  synthetic sequence
tcactaatcttttacttgccatctctcc

SEQ ID NO: 1598 - DNA, 17 bp, Artificial
  synthetic sequence
tgtggaggcgttggcat

SEQ ID NO: 1599 - DNA, 21 bp, Artificial
  synthetic sequence
ttgccgctataggagcagtaa

SEQ ID NO: 1600 - DNA, 25 bp, Artificial
  synthetic sequence
attctgctttaattgaacgcaatcg

SEQ ID NO: 1601 - DNA, 18 bp, Artificial
  synthetic sequence
agcagcagtcgtgtttgg

SEQ ID NO: 1602 - DNA, 20 bp, Artificial
  synthetic sequence
agcggcaacaactgagatga

SEQ ID NO: 1603 - DNA, 20 bp, Artificial
  synthetic sequence
ttttggcaacttgggctagg

SEQ ID NO: 1604 - DNA, 19 bp, Artificial
  synthetic sequence
acccaagtgacattgcgct

SEQ ID NO: 1605 - DNA, 163 bp, Artificial
  synthetic sequence
gatatcagggataggccggaggcctcgtaatgtgtcttcggattgttcatatcgggcatatagacatgtcgtaagcgctgatggcattgacgagatccatgatcggaagtcacgatggttatgcagtcatcatgcaaatgccattgatgttcgaatccatagg

SEQ ID NO: 1606 - DNA, 158 bp, Artificial
  synthetic sequence
gtatgcatagtgatggggctggtggtcatcattctcggattcagaggacggcgtaccggtggtctgattcctctcggactggttgccggtggatgcgcgctctgcatgaccatcgtttcaggcacgtatggcgtgtactaccgtgatcttggtgccag

SEQ ID NO: 1607 - DNA, 140 bp, Artificial
  synthetic sequence
tcaactgtatttgtagattttatagttgctgttaacttgttatcagaatcttctgctaaagttgcattgtaagcattaactgcatctactatttcttgagcagttttgtagttttcaattttatagtcaactacttttcc

SEQ ID NO: 1608 - DNA, 143 bp, Artificial
  synthetic sequence
aagaaagttatgtgggagatgaaattatgagtttagattttagttttttaagtagatttgggacttcttttttggaaggaacaggtgtgacagtatcaatttctcttgtggcattatgctttggatttataataggtataatt

SEQ ID NO: 1609 - DNA, 134 bp, Artificial
  synthetic sequence
tctgttaaagagtttattttattttgtaattgagttgcattagttaagtttacattgtctacttttatatcgtaaactctatcatttacatttgctcctgcttttgtatcttcaaacttaacttctaatgcttt

SEQ ID NO: 1610 - DNA, 150 bp, Artificial
  synthetic sequence
ctttttctatttcttcttcttgttcaacaaatagtcccaccaacttctcacttaaaataagtgagttaatactttctagctccaaaagttctttaagaaatttatcatagattagctcaaaatactctaatacgacttcttccttatttt

SEQ ID NO: 1611 - DNA, 154 bp, Artificial
  synthetic sequence
gctgaactcgttatcgctaacgtcattgaccttcgtgccttccaatctatctcagcctatgattcagttgttgctgatgatacacacaaaggtgctgaaaacctcattaatgactttgctgacgaagcaaaaaaagctggcgttaaaaaagtca

SEQ ID NO: 1612 - DNA, 155 bp, Artificial
  synthetic sequence
gggaatttcaatacccacagcagctttccccggaatcggagcaataatccgtatgctcgaagcttggagttttaaagctatatcattttctaaagatttgattttctgaaccttaactccagaatgaggtaacacttcaaaagctgctaatgtcg

SEQ ID NO: 1613 - DNA, 129 bp, Artificial
  synthetic sequence
ctcaacttgtaggcgaagaagacgcccagtcccaaaaggaaatcgactttctctcgcagtgtgacaagctctcttggcgtgcgttcctcaaaaatagctacgagatcatcccaacatttaaagagatgg

SEQ ID NO: 1614 - DNA, 139 bp, Artificial
  synthetic sequence
atcttaagttgcgacagcgagcccctttgagacttgcctcaaagttgttccgctttttagatgttccctcgattcgatttagtagctaagctatcgggaagattctcctgcaacactcctaggagatggtgtataagaa

SEQ ID NO: 1615 - DNA, 136 bp, Artificial
  synthetic sequence
gaagtttaggttgaaggttttagagtcagatttagaagggattctagctcagactgagagtgctgagagtctgttaactcaagaagaacttccgattcttgcaactcggggagccttagagaaagctgttttcaaa

SEQ ID NO: 1616 - DNA, 142 bp, Artificial
  synthetic sequence
ttcaagcatttcattaataagttgttctatgttttcagctggaaaatcatcacctaattcttcattaatttcttcataagttataatcccttcttctactgctttttttattaaagctctagctttttcattttttattagc

SEQ ID NO: 1617 - DNA, 79 bp, Artificial
  synthetic sequence
gagcgctaatgctcagacaatggctccaaattacttccatgccgatccgcagcaattcaaacacaggattgtaaaagaa

SEQ ID NO: 1618 - DNA, 159 bp, Artificial
  synthetic sequence
caggtggcacgcatcgcgtgggaactatgttgccaagtggcatagtaaggccccattacatggcaattgatacaaactcgtggatcgtcacttaagtagctataagctttggacatatatacaaggtatgcgcctaatccaacgaatacaccaactagt

SEQ ID NO: 1619 - DNA, 157 bp, Artificial
  synthetic sequence
cacaagactcaatagctctgcaaaggtatcttgtgggataaagagcatacttgctccactaaaaatcgcttttttaagctcatctttattttgcaccccaataaatggctcaaagctaaggcgccttgcaaagctaagcaatttagtcaagctttta

SEQ ID NO: 1620 - DNA, 136 bp, Artificial
  synthetic sequence
tctgacaaatcaagcatataggcttcaaaatgtccaagcgtttccatttgctcctcaagtgcataggctctatgaatataagagagagaatctgcacaaaaagtagcagattctataaataatctttgggcaattt

SEQ ID NO: 1621 - DNA, 151 bp, Artificial
  synthetic sequence
aattttcttcattgtgataatcaactctattattggtattatccaagaaaagaaagcccaagcttctcttgccgctctaaaaacaatgagtgctccaactgcaacagtaattagaaatggatctgaaaaaattgtttcagctagtgaatta

SEQ ID NO: 1622 - DNA, 150 bp, Artificial
  synthetic sequence
ttctaaaatataatctatactatctctaaaaaatatagaaatcaagagaggataaagatctatgtatttagatgatttcttaattttaatttctgatctccatcctaattttcaatttttttatcaaaataagaaaaatggcgtaattga

SEQ ID NO: 1623 - DNA, 150 bp, Artificial
  synthetic sequence
gattagtttagtgatttgactatctgtaagattgcgcagcagttgaccagcgattgcaattgtttgatcttcgatttcaaaattatcttgaataggcaaaatagttgttgcaaagctaaaactggctaaaagactagcccagtttttttc

SEQ ID NO: 1624 - DNA, 141 bp, Artificial
  synthetic sequence
tttacgctactagcatcttttaaaaagtaacctgctctaattctagttattccacttaaaacttcaactaaaggaaaacggggaaaagccggaaaatgatataagtcttctgcttcgtgttctatctcatccttaacatta

SEQ ID NO: 1625 - DNA, 163 bp, Artificial
  synthetic sequence
gaacggacaagctcgaagtatcaaagcggttggattcgtcggatggggctcggcggagaaaccgaaagccgtgaggaacacgcggattttcgtcatatgatcggccaggctgaatttgtcactgggggagtgctccgtgtgatccgggacgttggccatcgct

SEQ ID NO: 1626 - DNA, 163 bp, Artificial
  synthetic sequence
cgtcaccgacctggcagcgatgtcgtcagcaaccttgcggccagatcgtacctcacgatcggccgccgcgaggtcaaccggcctgcccgtaatgcagcgacgccgcttccaagagaggatgcgcagcaccgattcgtcgagacgccgctcgctaacccgaccg

SEQ ID NO: 1627 - DNA, 149 bp, Artificial
  synthetic sequence
gattaaaataagcgggagtctaaagaccttaaattgctcatagatttcagaatttaaattgacttctggctgaatttcatcgtcttttttgattttaaaaaatttcaacttttcaaacaaaaccaattcctagatcaaaataaattctt

SEQ ID NO: 1628 - DNA, 136 bp, Artificial
  synthetic sequence
aagttcctaaaattgatttttgtttcaatttattctcattcaatcgctatatttaatcaaaaagaaagcaattttatagtagaatgtagcatttagaactcaagtagagaaaatgtagaaggaaggaatacatgaa

SEQ ID NO: 1629 - DNA, 147 bp, Artificial
  synthetic sequence
cagttgtagttctaagtgatagaaatctaaattcaaatccaaatcttaagtcttatttataaagaaataaaagctaagacaggagctgccttaagtaaggctagatcatgtattggtaaatactgttcttttaaatagtttagaaag

SEQ ID NO: 1630 - DNA, 135 bp, Artificial
  synthetic sequence
tgatcatatcggaaaaactttctctctagtataaataagtcagtagtttttagattaaaaataagattttcagcaatgcataaataattagaatattttttcttataagctttgatgaagatattgtattaaatt

SEQ ID NO: 1631 - DNA, 124 bp, Artificial
  synthetic sequence
cattaatggttattttccataaggaatataaaagtattattttgtgagacagggcataagctcatcatttgtgtctatggttagtaactagtactcgggggggggggataattaactaaatata

SEQ ID NO: 1632 - DNA, 151 bp, Artificial
  synthetic sequence
gtcatttttcaccttccactggaagcctctactctattgtctataatagtatcgggtattgcttttattattttatctataggacgcctatagtctaacctttgggagaagtatttgcttcgttatctaatttcttgtcgtgatctcgttg

SEQ ID NO: 1633 - DNA, 155 bp, Artificial
  synthetic sequence
aaaagcggtttctatagtttcatcaaaaggtgttttcgtaagctggatttttttagttaacaaagaaggttttgcttgtgtcaatacagcaaatttaaatcttttagaaaaccctgaagggagaatctcgctttgaataaagttcacgagacctt

SEQ ID NO: 1634 - DNA, 145 bp, Artificial
  synthetic sequence
tgaagaagaggcttattgagttgacacgttaaacaccactttgcagtgaaatttacaaaaactggaatccctttttcgcgtaaatcagctagcttttcgggagaaaaagattgccaatcagagctatgtgcaggagggacgttct

SEQ ID NO: 1635 - DNA, 76 bp, Artificial
  synthetic sequence
caaagaagtcttagaactttctataagtgaattttgagtatgctctctaataggtaaaataccttcaaaaccagca

SEQ ID NO: 1636 - DNA, 117 bp, Artificial
  synthetic sequence
atatcaagagatatgcaagaaataattctattattttttattaaacacaattcactagaaccaccacctatgtctaaagtggttccatccttaaaaggacttaataaatttagagct

SEQ ID NO: 1637 - DNA, 93 bp, Artificial
  synthetic sequence
aaatacgcaaaatcaaagtgtattgccaagtgaacctatagcaactcaagacaataacaatgatacttcttttgaaagtatgccaattacaga

SEQ ID NO: 1638 - DNA, 160 bp, Artificial
  synthetic sequence
tggttttcttccctgccttttcttaatatcaatagtatgctaaattttaaaaatctgtttctggtaagtgttgctctgtggtcggcagtaggaatggttcgtgcccaggagttcgatccgaagcaaagctacgagatccatacccagaacggacttgtcc

SEQ ID NO: 1639 - DNA, 137 bp, Artificial
  synthetic sequence
gcatccccttccacaaagccctcctgcaacagatactcaattccgacacctactccgcacaaaccgtcaccataagtcaccggaagttccaaagaacaattctccatcacctcatccagcaacacttctgctttctc

SEQ ID NO: 1640 - DNA, 164 bp, Artificial
  synthetic sequence
ctatccagtcaatcaggtaaattaaatgctctttcattcgtagcaccttgatgtcttcctcacctttcctccgggacaaccggtaatacagataataagcgagaccacaaatacctttcccgatgcctaaagttccgatcgccctactattaatcgtgttaaat

SEQ ID NO: 1641 - DNA, 75 bp, Artificial
  synthetic sequence
agagcaagaaaaaagacattgttatttctaacagcgccgatttcgatcaacaagaatatgacaccgcagttggta

SEQ ID NO: 1642 - DNA, 106 bp, Artificial
  synthetic sequence
atgttctcccattaaaatgattttcgcatggctagtaccaatcccttgttgtttcaccatcgtaacctactttctacataaaaattcaaacttaatcatagcataa

SEQ ID NO: 1643 - DNA, 151 bp, Artificial
  synthetic sequence
aaaaacgatggaaagcggtgagacaaccagaagcatttgtctcaccgctttttctatcggattttaggtatgcgctacttgacttcgactaaccgtaaagggtatgcgagaatgctgtttcatcgtttttcagaaaaagaatggaactttc

SEQ ID NO: 1644 - DNA, 108 bp, Artificial
  synthetic sequence
cgtgttccgggctgattcggaacgatgagcattccgcagagtgctgtgatttgacttcaagcggcttcaaggttgtatggtgctttctgaaccgatgttcagaatgat

SEQ ID NO: 1645 - DNA, 115 bp, Artificial
  synthetic sequence
gggggccggtgacatccgagtgatgccatcggcccccaccatatccggaagaatcccggaagaatcccggaagaatcataggcccgcatccgccagcgaaatgtagccgggttca

SEQ ID NO: 1646 - DNA, 117 bp, Artificial
  synthetic sequence
attgatgatgccttttgtcggtgttgatcgccaaggaatggagaatctttacaccatgttaccggtccgccgtactaccattgtcgccggccattatctgttcggtttgatgacagt

SEQ ID NO: 1647 - DNA, 157 bp, Artificial
  synthetic sequence
catcctgtgcaaaactcagttgaccgtcatttgctacattaattgcattgacactctttgtccctgtacccgttacattaagatccaaagtgctgccacttgcaacgaagaagcctccggtacctttaatattgataaagccatagccaagtttagg

SEQ ID NO: 1648 - DNA, 83 bp, Artificial
  synthetic sequence
ccgatagtagccgctggtttgtatctgatataaagtcggaagtacggccgacatacgcattggcaagcctcgttcaattagct

SEQ ID NO: 1649 - DNA, 63 bp, Artificial
  synthetic sequence
gccggacagggactaggtggaggtaatgctggttcaggtattacaactgcacaatcgttggga

SEQ ID NO: 1650 - DNA, 68 bp, Artificial
  synthetic sequence
tcgccatgattttcgcgttgatttccgtttggagtggagacctgacacattgactacgattattttcc

SEQ ID NO: 1651 - DNA, 134 bp, Artificial
  synthetic sequence
tacagaactgaataataattattattcacaaaataaagacttactatagcagttaccggaatcaagaataagaatgaaataacaaatcaaaacacataggatttttttaactgttggaaatatagctttgttac

SEQ ID NO: 1652 - DNA, 142 bp, Artificial
  synthetic sequence
acataaagttcattgtaatcttttggggtatttgttgaatacattaatttagaaggattttgaacatatgcatcaaacttagtttgatcaaatacattgttagcaattaatttatttaataatccaattgctaataaaccat

SEQ ID NO: 1653 - DNA, 145 bp, Artificial
  synthetic sequence
attacttccattattagttgttaaactaacacccatcgctcttaatgtgtcactagagaatgccttttgaattcttgtgtcattttctaaagaagatccatttgatgttgatgaattaggtaaagtttttacttcatatttattc

SEQ ID NO: 1654 - DNA, 142 bp, Artificial
  synthetic sequence
aactaatgtattaaatagaatagttacaaattgaataaaggatattacttgtacttttgatcagaaaattttatttctagatactgattgagtaattaaatcaaaatcaattgaatttctaatattgtttgtggatattata

SEQ ID NO: 1655 - DNA, 142 bp, Artificial
  synthetic sequence
gaatgtaaccactcaaagccctgtagataatagtactaataatgatgttaatgtaaataattctaatttagctgatacacaagcagaattaattgattcaaatacacagttttatgaaagttcgcctttaattgatcaaatt

SEQ ID NO: 1656 - DNA, 107 bp, Artificial
  synthetic sequence
gcgagtccaaatgcagataattacactactgttaataactataatgatcttcaaagagctgttagcaattatagtgtaagcggagtaaatatcgatggtgatattta

SEQ ID NO: 1657 - DNA, 146 bp, Artificial
  synthetic sequence
attgttgaacaaaatcaatcatcaagtgaaggtgctcaacaagatattaatgcagcaaatgatgtatctgcacaaaatgatcaaaaaagtgttaataaaataaatgatgaaattataaaaaatgaaaatgtagacgctgatattaa

SEQ ID NO: 1658 - DNA, 145 bp, Artificial
  synthetic sequence
taaaggatataacattcaatcaagtactgttaatgtcgatgataatgcttcactaacaattaatcgctcatctgttggcgatggtatccatttgttaagtaatggtattgttaatgttggtaattatagccaattaactattaat

SEQ ID NO: 1659 - DNA, 152 bp, Artificial
  synthetic sequence
ccgagcgctgcatgtactcagacgcggcatgatgcagggcaccggtcagcgttgctgcgtgatgcggcaggctgcggcgcggtgctttccacagcgccgaaaccggcggatgcgggttgcgggcggagcgggttgtcatgggctgttctccg

SEQ ID NO: 1660 - DNA, 166 bp, Artificial
  synthetic sequence
ccgcacggcttaactgtttccagcgtatcatggtcagcctgtcatggtcgtagttgcgcgcgggcatgtgccagcggcctgaggtgtctatgaacatgacgcggcagtcgcctatctgcgcccattgtgcgctgttttctgtcagacgcagagctgccgcactggc

SEQ ID NO: 1661 - DNA, 164 bp, Artificial
  synthetic sequence
ggtcagcgccacggcggccacgtcgtcatggcatttgaagcgcggaaacatgcggcagtcggggtcctgactctgcagcgcgtgtatatgccggtgcagtccctcaaggcctctggtcaggtaggcgcgggccagatcgccgaacgatgttccgtactccggtg

SEQ ID NO: 1662 - DNA, 161 bp, Artificial
  synthetic sequence
gtgtaaaaaattgtaagcatgagagtgtccggttgatgaatggcagccggacggcatgaccgcccggcaaagaaggacgatcagcataccccctcttggcagggctttcaatacgccggagtatgtaaaatggaactgtcaggaatcgttgtgttttgcat

SEQ ID NO: 1663 - DNA, 160 bp, Artificial
  synthetic sequence
cagcaacgaaggcaattcatggagaagtgtccttacctctattctcggacgcgtattctattcctaccaaaataaatacttattcaccgccactatccgccgggacggttcctccaaattcggtaagaacaatcgatatggttacttcccctctttttca

SEQ ID NO: 1664 - DNA, 97 bp, Artificial
  synthetic sequence
aaccatcttgccgccaaaaccaacaacagcgactggtggtattattatgaaattccaatgataaggaagacaagaacatggatgaactctcagaccg

SEQ ID NO: 1665 - DNA, 154 bp, Artificial
  synthetic sequence
tgccaatgaccctatacgcaatgcgggcaagatacgtaacaatggctttgaattcaatttaggatggatggaccaacccaatccggatatttcgtatggcatcaacttaattgggtctttcaataaaaacaaagtaatagccatgggaagtgaa

SEQ ID NO: 1666 - DNA, 125 bp, Artificial
  synthetic sequence
ctgccggagcagttttaatacgtttttcatttgagattccgtagcgcctttgtcccaagcgaatttcgcttctatatgggcttttgtcaattcttcctctacacgcatgcgtatggcgtagactt

SEQ ID NO: 1667 - DNA, 145 bp, Artificial
  synthetic sequence
ctctgaatgcgatcgtaggcttctcccaattgctcaattcggatatgcctttggaaccggaggaaaaggcggagtttatagatctgattaccaaaaacagtgacctgttgcttaagctgatcaacgatatcttggatctatcacg

SEQ ID NO: 1668 - DNA, 125 bp, Artificial
  synthetic sequence
cctggcctttgccagaagccttttgctggatcccctggctaactacgccttgcgcctggcggtgtgcgaggacctggtcaagctgggggttaaagaagagatgcaggttatgatcctgggggact

SEQ ID NO: 1669 - DNA, 163 bp, Artificial
  synthetic sequence
attaagccgcttttgaccatgaacaatgaccaaattcaagtcctgcgggcagaagctggcaagatagcggacaaattgcagctggtcggctttttaagcgtccacttcgccatcagccaccggggtacggaaatggtctacaagctcttggccgttaagccac

SEQ ID NO: 1670 - DNA, 164 bp, Artificial
  synthetic sequence
gccgtcttgctcttgaagatcatcgacaagctggcttctttgccccaggcaactttgaatgttctgggctctttggccagtggccttatccgggacacgggggacgtgatcaaggtgattgctgaccagtcccggcaaagcaggcgcaaactgcccaaagacaa

SEQ ID NO: 1671 - DNA, 161 bp, Artificial
  synthetic sequence
aaataggggatgtagtcccgaaaatacggggcgaaacgcctcaaaatatctcttagtttcagctcttttttactcattcgtatcccaaattttaaattttctcccacatcgtgccttgggcggtatccattatggcgatatccatcgcattgagttttttc

SEQ ID NO: 1672 - DNA, 154 bp, Artificial
  synthetic sequence
taagctcatagtcactgatgtgaggaagaagaaattttaaggattgctccttactcaaatgctgatcgcatcctccatattctcgcaagcaaattgcaggaaaaatgcgaacagcgtttgagtagtgtaacgaagcaaaattcccttaaaattt

SEQ ID NO: 1673 - DNA, 78 bp, Artificial
  synthetic sequence
tttaacttctaaaatatatgatctttcactcataaaatttagccaagttatatatatcaattgataaaatcaacttta

SEQ ID NO: 1674 - DNA, 160 bp, Artificial
  synthetic sequence
aaagagtaatatttcattataatttttaaataaattaaagattactttaatattatcgagttacaataacgcccaaataatacgtaaatttatagtaaaggagcttttatgagatccataaccaacaaaatagcactcatgctattgattgcgttgttta

SEQ ID NO: 1675 - DNA, 138 bp, Artificial
  synthetic sequence
tagacaacatatgatcaaaagtttcttcttcaagtctatttccgattaattcactaaatttatcgtgtatatacttgagattgtatcttatttgtcttgattgtaaatattcaccattttgataaacaaccaaaaatg

SEQ ID NO: 1676 - DNA, 145 bp, Artificial
  synthetic sequence
gttttttagcaatttttccatcgtctgtttcatccgttttagttaaaattagaatatgtggcggtctttttgcgatttttaaaaattcttcataatctcttgtatcatcatgaatgcttgctaaaaacaacaccaaatcagcatc

SEQ ID NO: 1677 - DNA, 144 bp, Artificial
  synthetic sequence
ttctaaaataaaatctctgtatatatcgcgtaaatttgtgttactgatgatttgcggatcaaagaaatactcatgctccggcaataatttagcaatctctcttaaaatttcagcacgataaactttttttttaatatttacagg

SEQ ID NO: 1678 - DNA, 124 bp, Artificial
  synthetic sequence
ccaggaatttcgccaacatcagttccaaaatatatattttgaatcttgatgttataaattttattcaaagatgtaattatgtcattaaaataataaaatatctcatcaaaaatttggattatat

SEQ ID NO: 1679 - DNA, 87 bp, Artificial
  synthetic sequence
cttttataagtccttttaagagcgaattttcagctccgccagagcttcgcctaaagtggataagagaaatttggggcggcctagaga

SEQ ID NO: 1680 - DNA, 138 bp, Artificial
  synthetic sequence
atacgcccaaagccgtttattgctactttaactgacatcttagctccttttgatataattacgcctaattctacaaaaaagaattttaaaacaaatataaacaaggcactttaatagatgaagttagcactttttggc

SEQ ID NO: 1681 - DNA, 76 bp, Artificial
  synthetic sequence
agtgacgcaaagatcgtcagtatcaatggtgatgaggttttaatcgacgttggcaagaagtcagaaggcattttaa

SEQ ID NO: 1682 - DNA, 122 bp, Artificial
  synthetic sequence
tcctaacgaaccccaagtcaaaccggacccccgcggcggtttttcaggaagccgccgctgagagaccgcacaattccgggtgaagccgctttacacacttgccaatagtgggaagcgtgcta

SEQ ID NO: 1683 - DNA, 82 bp, Artificial
  synthetic sequence
tggggagagtaaaactagattgccaactggatgagatagttgaccacgctgtgaagaaagatgtcgaacgatgcaacaaacg

SEQ ID NO: 1684 - DNA, 109 bp, Artificial
  synthetic sequence
tctcttctttcgtgggaaatgagggggcctgcggggaggccccctcattaaacctgatgtagattcctctacaagttcctgaggaacttagtcaaggatttcgctgata

SEQ ID NO: 1685 - DNA, 115 bp, Artificial
  synthetic sequence
ctgtgcgaagtcgcgccgggcggcaacggcgaaccggtcgtcggcgatgacgaaagcatgcgcgtcgggtggttcgcgctcgacgatctgcccgaaccgctcagcgacagcacac

SEQ ID NO: 1686 - DNA, 113 bp, Artificial
  synthetic sequence
atctcaggcaccgtgcggaaggaagcgcacgggcacagttcgcgttcgacggggtcatcgagcatctgtaggccgcatacagcggcatatgaatcaatggatgctgccgaact

SEQ ID NO: 1687 - DNA, 161 bp, Artificial
  synthetic sequence
ggactgggagccgctgttgctgtctccattgccggagttgccgttgctcccgctgctgccgttgctattgctcggtgaggggctggggcttgggctttccttgggctcagtggtgagtgtcacctcggtacctggattgacctgagaccctgcgctcggat

SEQ ID NO: 1688 - DNA, 162 bp, Artificial
  synthetic sequence
ttgctattggctgccaccttccacttgaggttgagagccgaatcggtgagtgcggccttggcttccccgagtgtacggcctacaacgttcggcactgctaccttgccgttcgacacccagatggtcacggaggcgcctcgctccaccgatgtgccctcgttc

SEQ ID NO: 1689 - DNA, 161 bp, Artificial
  synthetic sequence
gtaggcctatatgaagccttaatctcagaatctgctgcatcaacgcattctagtaactcatcttgtacacaggcatcaaacacttcttgtaaagttaatgcaccaaatacctgctcagactcatccaaaagcgcaggcgcaattagctctgtgaggcgtgc

SEQ ID NO: 1690 - DNA, 146 bp, Artificial
  synthetic sequence
aggaattcataatgaatcactagcttaaagacagcttgtgttcagatgcttcttgtttgcccacaagttgtgtaactgtttctttaatttctaatgcaagatcaataaaatcttgagcagtaacacatctcactgacttgccacgc

SEQ ID NO: 1691 - DNA, 149 bp, Artificial
  synthetic sequence
agatgtaatatcatcaaagctaggtcttttttctgccattcttcaatcctttctttattattcattttattttgtaacatcaattaaatactaactgcatcaaataaatttttctaacattatcttaactcccaaaaacggccataaag

SEQ ID NO: 1692 - DNA, 81 bp, Artificial
  synthetic sequence
aatagatattggtccacatcgcgtaaaagcagggctagatatcattttgtcaggtgctattggagatcactccattgccgt

SEQ ID NO: 1693 - DNA, 74 bp, Artificial
  synthetic sequence
cgtctcagtgagaatatgtggggaactcacgaactgaccaaagaagctatggaacgctctttgcgtgctctaaa

SEQ ID NO: 1694 - DNA, 66 bp, Artificial
  synthetic sequence
gtacagtcagtatgtaatatattagggtatgaccctttatatttagcgaatgaagggaaagtggtt

SEQ ID NO: 1695 - DNA, 129 bp, Artificial
  synthetic sequence
tttcatcatttgtcatacttaagcatattttttatcaatcattataacaaaaattgtacagagcagagatgaaatatatcttgtatctctatgattttaatgtatttataacgcgtatgaattatttta

SEQ ID NO: 1696 - DNA, 165 bp, Artificial
  synthetic sequence
aattgattgcacaagcggaagccgaaaaacaacggttgattgatgagaccaacgtctggataaacgggcagcaatggccgtctaaattagcgctgggccgcctctctgaggatgaaaaagcgcagtttaacgaatggctggactatctggacgcggtgagtgccg

SEQ ID NO: 1697 - DNA, 143 bp, Artificial
  synthetic sequence
gtgggtttttatatcgaaggtgtgtctgcggttccctccaatgctattgaagttagcgcggatatttataatgagtttgccggagtggcgtggcctgatgggaaagtactaggtgctgatgattcaggatatccgacatggat

SEQ ID NO: 1698 - DNA, 85 bp, Artificial
  synthetic sequence
caaccccatccgcaaaaaacagcgcgcccgagggaagtaaatgcgtcagtgactttagctaattgtgctgaaatttacccgtaat

SEQ ID NO: 1699 - DNA, 78 bp, Artificial
  synthetic sequence
ccaaaagtgtgttattggaagaaagcgttgaaaactttgatgctgttgctaccttgacaggagttgacgaagaaaata

SEQ ID NO: 1700 - DNA, 146 bp, Artificial
  synthetic sequence
aatcgtgtggaaatgattctcttccacaactttgtcaaaaccaaaatcattaaaaatctgatgattatcggcgcaggacgaatcgcatactatctcctcaacatcttaaaacatacaagaatcaatcttaaagtgattgaaaacaa

SEQ ID NO: 1701 - DNA, 76 bp, Artificial
  synthetic sequence
ctttcaatatcttttaattgatgataaatgtgatattcctcatcagcggttacgaccttgaccatatgaatttttt

SEQ ID NO: 1702 - DNA, 146 bp, Artificial
  synthetic sequence
ctttctggtttctttaataagcggacctttcgtactccagaaattttttctagctgttgtttcacttgattgagctgttcaaaatcagtactgtctatgtcaatcaatatgtagacatgctcattcttatggttacgcgatatatc

SEQ ID NO: 1703 - DNA, 163 bp, Artificial
  synthetic sequence
cacggccagccactttctttactgtcagttgaaggatctgctcctcctcagattgtgtgagcgtagaagattctcctgttgtacctaaaactaataatccgtctgtttgttcatctaaatggaattggatcaatttttccaaaccagcataatctactgatcc

SEQ ID NO: 1704 - DNA, 148 bp, Artificial
  synthetic sequence
atgtattcactcggctgtcatattcgtgattgttatcagcaatattgaaccagaatttatacatgtcgtttttgtattcccaataagtagttttcgtcactttttcagcatcgccgtctgtcttttctactttatttgtttcgttatc

SEQ ID NO: 1705 - DNA, 153 bp, Artificial
  synthetic sequence
attagtataccaaatagctcaactatagctgatataaatataagtctgcccatatttataggtacacttcccatagtctccttggttctggcatttactgcaacatagtggaggatattttcactaccctttttctccatataggagtatagc

SEQ ID NO: 1706 - DNA, 140 bp, Artificial
  synthetic sequence
ttggtatccctcttctcagatgtgtagcctcttaggtagtttgaattatacttgaccacattatctgtatcaaaaggcattatggaatttataatgttgttggtcttgcgcctgttagattggtctagcttgtctgagct

SEQ ID NO: 1707 - DNA, 143 bp, Artificial
  synthetic sequence
tagtcctaaccttctggtcgctcgtctccatattttttatattgtattgggtttctcgctcataggtatgtcttgcatttgaatttctatacctcaaatacttgattataaagaatataaatcctaataggtagaatacccaa

SEQ ID NO: 1708 - DNA, 142 bp, Artificial
  synthetic sequence
ttatatacatctacatcatatactaccttcttgttgtcgtcagacccaattgtatattcacatatagtctcttcaccaacgccccttaggtccacatgggccttcatgtcaactatcatataaggtaagtatacaccactta

SEQ ID NO: 1709 - DNA, 123 bp, Artificial
  synthetic sequence
ctgtttaaaataaaaataggattatttgtattatctgcaattacataattaacaagatttttaatcttgcctgaagttaaattgattttatcttcgcaatgagcaaaaataaattttctaatt

SEQ ID NO: 1710 - DNA, 94 bp, Artificial
  synthetic sequence
ctttttctaatcattctaattctttgtttttttcattaacttcatcaataattttttgtttttcttcgttagttaatttctttagttttaatct

SEQ ID NO: 1711 - DNA, 138 bp, Artificial
  synthetic sequence
aagagatgaaaaaatatttggttttttaaatgaaaatgaaactaaaaaactagtcaataaattgcacaaatataacaaaaaatatttactaaaatcaattaaatactttagaattggtaaaattgtagaaagaaaaaa

SEQ ID NO: 1712 - DNA, 87 bp, Artificial
  synthetic sequence
gctaatggattagaaattttagatggtaaaattatgaatgtagaaagtgatggaatgctttgctcagcagaatctttaggtttagaa

SEQ ID NO: 1713 - DNA, 163 bp, Artificial
  synthetic sequence
tttcagcacagtggtcagcagcatgtaggccgccacgacagccagcagaaagccaaagtagcgcggcgggaggatggtcagccccagcacgctgaacagcggggtaaaggaaagcccggtgaacagcaggataccggcaacggtgatgagcatgaccggggca

SEQ ID NO: 1714 - DNA, 120 bp, Artificial
  synthetic sequence
gtattttgcttttttcacgttcggacattctctgccagacgttgagccagccaggggtcagcccggcgaaaaaggcggctccggccgccagaaagatcagcccgaaaataatgcagtata

SEQ ID NO: 1715 - DNA, 160 bp, Artificial
  synthetic sequence
attctgcgatgatctcgatgcggccgccgggcaggtcgttgctgtccaggcttaccaggtacattttccggttccgcaccgcgttgatgaggtagctgcgcaggcggccctcataccgctcgtcgcacacaacggatacggtgtagcggttgtccgtctc

SEQ ID NO: 1716 - DNA, 104 bp, Artificial
  synthetic sequence
ttgcgattaaaaaagccggacataagcccggctactgaacctgctcccacttggcggaaaccttgtcctcatttttcaggcagctcgtggtgatctgctcaatg

SEQ ID NO: 1717 - DNA, 131 bp, Artificial
  synthetic sequence
ttaataaatacatcttttgtcataactttgtcttctccttttgtccagccggattactactcatgtttacttttacacttattagatgcatcggaaaggaaatcggttctcataaaagtatttttttccgt

SEQ ID NO: 1718 - DNA, 157 bp, Artificial
  synthetic sequence
tcatccaaacggcgttccgtctgcaactccgtcggtatatctaaaatataagacaaccaataattcacctgagcagataaagtataagaggaatcatctttaatcaattccggcattaaaggattagatttttctttttcaaatgaacctactatat

SEQ ID NO: 1719 - DNA, 150 bp, Artificial
  synthetic sequence
ataatacttatttctaatcgtatcgaatgtcagattcacaatagtatccagtaaaatttgtccattttttcctatcctgcgaacaggaagtaataccgactgtatcaaacttgacttacctgccgagttaacacccgttacaattgtaaa

SEQ ID NO: 1720 - DNA, 145 bp, Artificial
  synthetic sequence
cgaaattttggaatgcaactccgccccgattctattggcagacaaatagtataaattttgctctatgtcgatcggcatgctggcatcctcttccgaaggaagaaaaaccaaagagagttcatttgttccgtgataggaaatatgc

SEQ ID NO: 1721 - DNA, 149 bp, Artificial
  synthetic sequence
attgatcgtacaggcatatttttttcgcatcctggcatagtgctcttatgtgcctgatcgccttgtctctatgggcatttctataaaaacaaccggtgatatggctactgatctgatcggacatgatattgacatacggataatccgtt

SEQ ID NO: 1722 - DNA, 135 bp, Artificial
  synthetic sequence
gcccacgggggtgtatttgatggcgttatccaccagattgacaacgacctgcatgatcagccgtgcatccacattgaccaggaggatctcgtccccatactgtgttgtgatggtgtgttcgcagcttttccggtt

SEQ ID NO: 1723 - DNA, 147 bp, Artificial
  synthetic sequence
ccgccgcgccacgccgatcgtcaggctagcgctttggtagcttcatgagttcctgccggtccgcaaagcttaggtccgttcaggtgctgtgtctaaaggacgccccgaccccacacgacacaagagtgggcggaacgcgcagcactc

SEQ ID NO: 1724 - DNA, 148 bp, Artificial
  synthetic sequence
gatttcttttcttcagttgtaagagtgttgtctgaattaactttatccttaatactatttgcataagcagttaattctttttttgcagcttcttttgcttttaaagctttttgatcatcattatctgatgcttttaatacatttgttg

SEQ ID NO: 1725 - DNA, 139 bp, Artificial
  synthetic sequence
cgatttgtattggtatatttttgttttttaaaaatactatgaatttaaatttcctaccttggagaaatgcatatttgattgttacattctatgtttcagctgtttgtacattaatggcatttatagctattcctaaaac

SEQ ID NO: 1726 - DNA, 149 bp, Artificial
  synthetic sequence
ataagtttataaatggaattttgggaactatcgttagagcaaaaaaataaaatatatttttaggaggtagttataatgttacttaatactttattgttagttgtgttcgttggtattgttttttcaggcatagctgtgtcaactttttt

SEQ ID NO: 1727 - DNA, 145 bp, Artificial
  synthetic sequence
aattttaaattgcttctttaactcctcatcaataacttttttagatatatccttaattttatttttaacaactgaagcctcaccaatcttttgtttcatctctctttttattaaatcaacatacttatgagtatgtaagatatta

SEQ ID NO: 1728 - DNA, 153 bp, Artificial
  synthetic sequence
ttatggcgttctaacaatatacgaagtatctctttataattagcattaggatacttatcaagatatgccaactgagtttctaaaagtttatcaaaacgtttatcaagtgcttctttactcttagggcgagaatctgaaccttggttaacacga

SEQ ID NO: 1729 - DNA, 138 bp, Artificial
  synthetic sequence
aatgtaaatgattttgagcgtaatattgaaatatcatatactagttgaggatcgttatctttaaacattacgtaattaccaatgatgtcaccattagtataacttggtaaaatttcggtgttagattcattattaact

SEQ ID NO: 1730 - DNA, 133 bp, Artificial
  synthetic sequence
taaactagtagcttcttctggaacactaaaaaagacattgtctttgtattgtagttgaaattccagtgctttttcttgagaaaatccttcttctggtgttgcataataaattgttactttttgagaacttact

SEQ ID NO: 1731 - DNA, 165 bp, Artificial
  synthetic sequence
gtatttcctgctcgtcgttcttgctgaccagtccttgggcgccggcctgcgccacgtcgaatccgaacgtctccttggcgaacgaggtcatggccagaagcttcaccatgctgtcgcgtcggcggatacgacggcataccatgacgcccgacatggattccatcg

SEQ ID NO: 1732 - DNA, 160 bp, Artificial
  synthetic sequence
tacaagatctgcattgagttcgacggagggcatcacgccggtcaatggctggaagatgcacgccggcggcaggcaatcgaagacgagaagtggcggtatatccaagtcaccaagcttgacctcggtgatgaatggagtgaggaagctttggccagacgga

SEQ ID NO: 1733 - DNA, 164 bp, Artificial
  synthetic sequence
ccgagccgtttcgctatcgataagtcagtcagcccacgcgacataagatcgagcacctgcacttcgcggttggagaccaggtcagcccgtttcggcgtctcatgcgcgagctggtcgaatgaggcacgggcgtcaacgaacccgaaatcaccgtaaacgcctcc

SEQ ID NO: 1734 - DNA, 159 bp, Artificial
  synthetic sequence
cttcccctttcctgaatatggataaccgtagtacccatatggttagtggtcatattgtaggcgcataatgtggacagccgacgctaggctagagttagtggaatggcggtcgcgaggctgccgcggattgcgatttgtggagtgtgatgacgatgggcg

SEQ ID NO: 1735 - DNA, 103 bp, Artificial
  synthetic sequence
ccgaccaacgccaagatgatgccgagctcgatcgactcggaaacctgctttgcgcgttgcatgcaccctccctctcgaatatgccgtcagtgcaactccctac

SEQ ID NO: 1736 - DNA, 160 bp, Artificial
  synthetic sequence
catgcacaatcgagcgaggtgcgatcgatgccatctcggtgccgtagtcccgatgatgagccggaatttataatcaaggcgttgagatgggaggttgcttgtatgatttggttcacatccgacacgcacttcggccatgccaacgtgctgcatttcaccg

SEQ ID NO: 1737 - DNA, 163 bp, Artificial
  synthetic sequence
tcaaaataccctacttgtgcgccgagccacgtgagggagatcggcaaaaccgcaggatttgttggcgtggatgcgctcgggtgcaaggtcggtgggctccaggcatcatttgcaacggcaaaaccgcaggattgctgcgcacgaatgaatatacatgacggca

SEQ ID NO: 1738 - DNA, 151 bp, Artificial
  synthetic sequence
attttgaccactatcgcaaaaacgtatcaaccgtcgagggcgagggcctctgcgcccgctgagatgcgagtctgaaagtcgggttctgcgcgaagtgatcgtcaacttgacacatatgccgagcacgacggcgggtttatcatgggcgccc

SEQ ID NO: 1739 - DNA, 162 bp, Artificial
  synthetic sequence
aaacggcaaaaaaagtccccaccagtaatacgattggaaatatatatgaaataattccaaataaaccaaaaaagaagcggctgactgtaccgccgatcgtaccgccaaatccaaagttactgataaacagcaaaagtgaaacagcaaccacgatccataaaa

SEQ ID NO: 1740 - DNA, 157 bp, Artificial
  synthetic sequence
acatatgggaaagtccgcctccgatcagcccgcctccactttttgcatcaaaactgtaccgataagcatccattgcactttttgcatcagttccatcggaaatgagttcaaaaaacatacataaaaatgccacaaacaaaatgaccgccactaattt

SEQ ID NO: 1741 - DNA, 166 bp, Artificial
  synthetic sequence
cgttttttgtccatgacgctatggtaaacccaatactcacaaacgtcaacattcctattgtcttttaagaaacattttagattttggttatatttccacatatggatatcttcttatctattgatatctgatttaagcaggacgataagccgggttatgtctaaac

SEQ ID NO: 1742 - DNA, 152 bp, Artificial
  synthetic sequence
taaatatctctggttctcttcgtaacgctttgacacattccgtgagagtattctgaaataggaataaattaacaatgcgaggccaagccagtataaaatatttacccggaaaaatgcagataaaaatgtggatacaagtaacagaaccatcg

SEQ ID NO: 1743 - DNA, 71 bp, Artificial
  synthetic sequence
tgggtggcatgcttcaattttttgatcatatcttttctcgaaaagtaaagactggctatgagatgctcttt

SEQ ID NO: 1744 - DNA, 108 bp, Artificial
  synthetic sequence
gggtcgtcttgaaggtggctgaggtcccgattggcttcggcaaacaagtgcaaggtgtggtgaaaaacttcttcccgaaaggattgcggttcactctggaataaacga

SEQ ID NO: 1745 - DNA, 118 bp, Artificial
  synthetic sequence
ggtagtgcaggattcatcgcattggcgataacgattgctttttataattttggaaatccattagcaggggaagccatctataaagtttggactcaagaatcatttccaacagaatctc

SEQ ID NO: 1746 - DNA, 160 bp, Artificial
  synthetic sequence
caatagacaattcttggcaaacaattctggcagtctactccttcctgatatttgcccattccttcgcaaccctgggaggagccttctaccgtaagtttcctgtgcttctgacagcatgtacgggattggcactttgtctgattttgggttatattatcaa

SEQ ID NO: 1747 - DNA, 147 bp, Artificial
  synthetic sequence
tttcgtaggaaccttgcacatcgaagagggttcttctgctcaatattgtgctgtattcacctcgtctgcagtatttcttgctttggctgccttcaactattgggcatcctacaagctcttcacccgtatgcaggttatctgcaacaa

SEQ ID NO: 1748 - DNA, 88 bp, Artificial
  synthetic sequence
cagacgaccttgcggactctgtctggaaacacgctgtccgcgtgccatcagaagctttttcactcgataataatccagcgttaaacga

SEQ ID NO: 1749 - DNA, 75 bp, Artificial
  synthetic sequence
ataattccggtgccagaacaatcgcgggattaagaaatccgatcgccatcggcgtaggtgctgaccggctggcaa

SEQ ID NO: 1750 - DNA, 89 bp, Artificial
  synthetic sequence
ttcgactgcccttttaataatcgctgatcacaggccatctcgatatcattttccgcctgattgttcatcagccagacgaacggattaaa

SEQ ID NO: 1751 - DNA, 107 bp, Artificial
  synthetic sequence
tagagggtcttttcagtgagcttgatttcaggatggctttgtagaatggcatagaccgactggccctgcgctaacagaggcttgattagaagaccgagctgcttgat

SEQ ID NO: 1752 - DNA, 68 bp, Artificial
  synthetic sequence
ccttttagagcaagatgaagcagggctattatatgagtatctgggctttattaaaagccgtgatgaca

SEQ ID NO: 1753 - DNA, 71 bp, Artificial
  synthetic sequence
ttatggcaagaatactttgcaaaaacgcatacgcatgtatcacaagaagcaatcattagtagtggtaaaaa

SEQ ID NO: 1754 - DNA, 164 bp, Artificial
  synthetic sequence
ggatatgcatcggcggtgtagaaacggcgtgcatgcgacatcgcacttagacggggacatgcgaagcgcatcgcagcgtctgcgtctagacaacgggtgcgcggcgacgcagcgtccatgcctggatagtaggcgcgatgtaccgtacctcgaatgttgtctgc

SEQ ID NO: 1755 - DNA, 140 bp, Artificial
  synthetic sequence
cgagcgcgccgtcgcgatacatcagcagcgctgccgttttagagaggcgctcttcttcgtgggcaagcttcacgtcgtccattatgcccaatctgttttcgagggtcatccaaccacctgcctgccggtaccgaattcgg

SEQ ID NO: 1756 - DNA, 164 bp, Artificial
  synthetic sequence
gccgagcttctgatagatgtgcttgatatgggtcttgacagtgttgtaggaaagcacaagctcctgttcaatgaactttccgtcgcgcccgcgcgcaagctggcccagaatctcgagctcgcgcgtcgtgagcccatatgctcgagcaagcacttcgcacctct

SEQ ID NO: 1757 - DNA, 137 bp, Artificial
  synthetic sequence
tttaatagtaagtttgattatagctattttgatgcaatatataattggagttcctataatttggttgacagaaagtgtaaattcacttcttaaaagtttaagctctaagccagaatattctatgatttttggagttg

SEQ ID NO: 1758 - DNA, 147 bp, Artificial
  synthetic sequence
tattctatagcggacaaagctggaatagcaccaggaattattttgggtgttttatgtaagacaaatggttatggatttttaggtggtatagtagtaggatttttagctggatatttaacaaaaatagttttaagtaatttaaaactt

SEQ ID NO: 1759 - DNA, 69 bp, Artificial
  synthetic sequence
tctgaagttaatgatgatgataatgacaataggttttatgaacaagtaggaagatttcctgaaataata

SEQ ID NO: 1760 - DNA, 159 bp, Artificial
  synthetic sequence
gcagcaactgcctcacgggctcattgaaaaccgcatagcaccccaacgtcagcacatcacccacggcaagcacatcactcacgacaaccaacacatcaacaaacagcacgaacatcaaccgattggagaagctatgacaaaccaccgcgctgaagacgg

SEQ ID NO: 1761 - DNA, 158 bp, Artificial
  synthetic sequence
tggatgagatttacaagattaagacgagcggaaaataccattccttcgtccctgtttatcaagatcgcggaaatcatcgttatgctatttcccgatcggcgccaaaacaggacttttctatccttctatgcgaggacagtaagtctggtttccagttc

SEQ ID NO: 1762 - DNA, 157 bp, Artificial
  synthetic sequence
agtagatcgagcatatgaagtttgagttttagcgtgtaagagaaggaagatcggcaaagtacaaccccaaacgcaatgacaacttaatgaggtaactgccacatgtgaggcacccagggcattgctgtctcgattttgagcacgatgccttccgcct

SEQ ID NO: 1763 - DNA, 143 bp, Artificial
  synthetic sequence
tctcaatctttcttccttttacaattaatgaaaatgtccccgtcattacattaattcctgcaaatacaccatctacatcggttacaaggataccatgacacatttttttcttcaagtccaaaattgaggattctgttttctca

SEQ ID NO: 1764 - DNA, 159 bp, Artificial
  synthetic sequence
tgttccgaaccaatgtgctgcacttggtccctgattgattgcacccgaatcaattttctcatatccatacccactgatggccggtccgaatataatgaaaaatataagaacaagaaggataatacctgccagaagcgctactttattttctttaaatct

SEQ ID NO: 1765 - DNA, 108 bp, Artificial
  synthetic sequence
tctcggacgagcaggaacctcttcatctttctcaagtccgatgatttcaaacatttcatctgggatattttctgtcatatcaaatgtattctggttttccatcatgta

SEQ ID NO: 1766 - DNA, 150 bp, Artificial
  synthetic sequence
acatcagattttggcgattgtttaaaaccatttcctgtaggttcgatttttaattttttcgcaagttctttatttacaagttgtgttttaaatgttccttcttttatcaggtatttttctttcacaggtattccttcatcatcaattcta

SEQ ID NO: 1767 - DNA, 150 bp, Artificial
  synthetic sequence
ttgaaatttgtagcagtagcggaaccaagagcggatcgacgggaagagtttgcaaagcttcatgatattgcacctcaaaacgctgtggaatcggacatggagcttttgaaccgtccgaaaatggcggactgtgttctgatctgtacacag

SEQ ID NO: 1768 - DNA, 155 bp, Artificial
  synthetic sequence
ttaatcatatgtttctttccttcccattctctttttttcttttgcagaagtgatcacgtgccggattgccatgattggatgataaaataacattctcggtccggcaaaccgcatcacatttcgaatttcttctctcatctgcggcttgtaacaat

SEQ ID NO: 1769 - DNA, 153 bp, Artificial
  synthetic sequence
gtaattctgcttccgccggtgatcttgttctgctgtttcagcaagtactttattgaagcactgtctggtggggcagtaaaaggctaaaaggagagaaaaaacatgaaacaagtaacagccattcttttgggagccggacagagaggggcagag

SEQ ID NO: 1770 - DNA, 112 bp, Artificial
  synthetic sequence
tccaatgttttttcaaacagctgctggatcatatttcctgccgcaaacactgctgcgatctgaaacagcagtgcgatccactgccagaaaatattagctccgatatattttc

SEQ ID NO: 1771 - DNA, 139 bp, Artificial
  synthetic sequence
ttttatgctttttattccagcaaccttcattaagctctactaatcctattatgtttttaaaacttaaaatttgatagttctaaatttattaaagtgcttattaatcgtatcgcaattgatactcgaaggcttatttgtt

SEQ ID NO: 1772 - DNA, 94 bp, Artificial
  synthetic sequence
taaaagaacataacataaaatccatagatttacgttataaagaaacacagatagataacaacggcaatctaatcaaacaaacctctaccgttac

SEQ ID NO: 1773 - DNA, 98 bp, Artificial
  synthetic sequence
aatttatctttttgacaatcacaaaatttaaatttgacaattagcggccttgttgttagatttgaggataaattttggctcaagataagttaaaaact

SEQ ID NO: 1774 - DNA, 159 bp, Artificial
  synthetic sequence
cgccaaaatttagcgatgtcaagtccgattacacgagaatagtagatgttcatcacgcagatatttagcaaggtgatcgcaaaagccgtaccgcacgcagcgcccacgccaccgtaagccttagctagcgggatagaaatagcgatatttacgagcgtg

SEQ ID NO: 1775 - DNA, 146 bp, Artificial
  synthetic sequence
aattttatcacgcagacttcattctcgcggcagaaaaaatttgccagcacgcttagcacgcgctcggcaccgcccttgcctaaagcagaaattaccatagctattttcattttatgagcctaaacttatttttaaaaatttcatcg

SEQ ID NO: 1776 - DNA, 146 bp, Artificial
  synthetic sequence
aacagattattccaatatgttttagccttttcataatgtttgttatctggcaaaactacacctcctctacttagtttttgtttagatcaataaattctgctatcttgttgacagacctagcttgctgtttttcaggactaataata

SEQ ID NO: 1777 - DNA, 142 bp, Artificial
  synthetic sequence
tatttatcaatttatcatttaaactatttaggtggccttctgaagatatcatatagtagtagtattccatggaatcacttgtctgtctcataatatctcttgcaaggtctgtaaacctcatgtccctactagatggattgac

SEQ ID NO: 1778 - DNA, 132 bp, Artificial
  synthetic sequence
gctatttccaccctctatagcatagtatttagacttgctcggtaggtttttcttggcttccttaattctagtaaaatcaagaagtccgtcatttgtaccccatatagacaataccggcatatttactaggtt

SEQ ID NO: 1779 - DNA, 152 bp, Artificial
  synthetic sequence
ggctattatttgatttataatgtgcttaaataggtatattatactcctagcagtcaccttgtcataataagatggcttgtacataagctttatagacattccctttgtaagactgaccttcatatataaatcaaggtctttctcttttatcg

SEQ ID NO: 1780 - DNA, 150 bp, Artificial
  synthetic sequence
ataaaatatgaaacaaaaaacttttccttaccagacaagatgccattgtaccctggaggtgatggagcattaagagctttcttatctttgaacttacattatcctgaaaaggcacaagcttttggtgtagaaggtagaagtctcatgaag

SEQ ID NO: 1781 - DNA, 147 bp, Artificial
  synthetic sequence
ggttgtcttcaatgttgaaatggatggaacagtgacgggagctcgtgttgcagatgtgaagaatgcccgtggaaccagcaagcgttttatgaagatggaaccagcaaaacaacaacggattcttaaagaatgcgttgattactacaa

SEQ ID NO: 1782 - DNA, 138 bp, Artificial
  synthetic sequence
aaatggacaccagctcaggagaacggacgccccgttcagagcaggacttctctgacaattgcctttcgggcctgaccattaaagaaactaactcatgataatacgaagagagcatatcgataagaagacaagctatag

SEQ ID NO: 1783 - DNA, 155 bp, Artificial
  synthetic sequence
gttgtcacgtcaacagaaacaggatcagactctgctccgtcagcatatacggcagttacgctgtagttatgctttgttccgtcaacggtaacatcaccactctccagcttgatgctgttagatagatattcaccatcacgatagatgttgtatga

SEQ ID NO: 1784 - DNA, 152 bp, Artificial
  synthetic sequence
tgtcaaattcttgcaagaatcgatgaaagtcgtctatgatcaccacttggtcaaggatttcattgaaaaggtttggattctcaatacctaccaaatctcgcccaagatgttggaaattctccaagatgagctcatgctagacattgtgcaaa

SEQ ID NO: 1785 - DNA, 154 bp, Artificial
  synthetic sequence
tgctaatttctttggtgttgcccaacatcgatgccgccacctcgtgcgccatgcgggcgatctgattgaccttatcagcgatgttctcaatgctttggtgctgatctttggagtaagacacgacatttttggcatctcttaaggaatgggtggc

SEQ ID NO: 1786 - DNA, 151 bp, Artificial
  synthetic sequence
acctcgcacatctaactccataaaagtgggggcgagcaaggacaccctacctaccaaaccgacaatcatgctaaaacttgctgatgtgctggcggctactgacccttaccagctctccattctctttatctagggcaaaatccgtcatttc

SEQ ID NO: 1787 - DNA, 151 bp, Artificial
  synthetic sequence
gccagttaggaaagtgatttttgaactagtggctattgttgctaccgcttcttcaacggttacttttttcatttcctttcacctctctcttattatacatctatctttcgtttattgattgatcgtactttttattcaaacgatttcattt

SEQ ID NO: 1788 - DNA, 145 bp, Artificial
  synthetic sequence
tgacagagtataaactcaaatcttttgttgtctctttctttacgagaatcaaacgaaaggatgtatcaatctgacaagttactcgactgtcggcaaaaggaccatctccgtcttcaatatcaagtaataactgttcatcttcgtt

SEQ ID NO: 1789 - DNA, 149 bp, Artificial
  synthetic sequence
aagtgaataatatttggtcttgctgttggatgatagatttttttcacaaatgaataaaatttttgtggctcattgttcattgcttcatgacttagaaggtattcgggttgttccaatccatgatagattccttttaacgatcgatagtc

SEQ ID NO: 1790 - DNA, 148 bp, Artificial
  synthetic sequence
atcctaattttatcaatgcttgactcgcttctggaacaaatcctcttccccaatagttcttattcagtgcatatccgatctctgcgttatcttcattttcttgtactcttaaatcaattgtcccgatgaattgttgattttcttttaa

SEQ ID NO: 1791 - DNA, 155 bp, Artificial
  synthetic sequence
cacggatatagtatgtatttcccggcttcaagccaccgattgttccataaatcgttgtatcgggcactaatgaaatctctttcagattggcaatggtaggttcttgtacctccgaactataacagaatcctttctctgtcaccaaagtactattg

SEQ ID NO: 1792 - DNA, 158 bp, Artificial
  synthetic sequence
acattggtagagtcttgcggagcacaggaagaaacaacgggaagatcagtcgtctttgttgttacataagttgttgtaccatacccacgcccgttggaattgatagcatacgcacgcactgcgtagagccttcccggtttcaagtcattgatacgtac

SEQ ID NO: 1793 - DNA, 134 bp, Artificial
  synthetic sequence
ttacaatatgatatggaaggaacttatgtattaccacgtttttccctaaccttatttcaacataaccataacaacttgaagaattcctaaaactactgttccaagaacaaattttttctatccattctgtttta

SEQ ID NO: 1794 - DNA, 142 bp, Artificial
  synthetic sequence
ctttcccttcgacaattctccataaattcaatcgtgaagaattaggagaatcaatatgatctaatttttctccattccaataattcttaatacttatatcatttaaaataaattcttttaactctaaattttctataataag

SEQ ID NO: 1795 - DNA, 92 bp, Artificial
  synthetic sequence
cgacaccttgattcattccacgcgtgaggaacgagatgacaaatacagcaacgatagctaatatgcatatataacccgtcttgcgcaagccc

SEQ ID NO: 1796 - DNA, 104 bp, Artificial
  synthetic sequence
cgaatgcgaaactgcgaaccgattcagctcccaacaagagaatacacaacaacacgataatagtactttgccccgtgttgatcgtacgaggtaacgtactgttc

SEQ ID NO: 1797 - DNA, 148 bp, Artificial
  synthetic sequence
atcaaagcaaaaaatatcacgataaacacactgtaccaaagggtgactctataaacgatactccccttatgcttctttgataacataacctaaacctcgttttgtcttgatcaaagctggatcttttgtctttttacggatatttttg

SEQ ID NO: 1798 - DNA, 157 bp, Artificial
  synthetic sequence
tccaagccttcgttttgatcggtggggctttgctcatcatctttatcggggtcttctcgatcgatggtggctttgcgactgttgcccataccgccgctagcaaccacaagatcctctccagtgctgactttaagatcaatgatctagcagcttttgt

SEQ ID NO: 1799 - DNA, 105 bp, Artificial
  synthetic sequence
attcattatttatcatatcggacgggtcgcggtggtaacttacctacctgtattagcggtcgcttcagtgactgatatcgatcctttactcgttgcagcctgtgt

SEQ ID NO: 1800 - DNA, 153 bp, Artificial
  synthetic sequence
attgttctttgttcttgctcttagcttaggtaaatggttcgttcctaagtttttagctgtttttagtcggttaaatgcaagtgaaaatgaaacgaccgcagctttggtcctttgttttggttttgcttttttagcagtcagtctggggatgag

SEQ ID NO: 1801 - DNA, 78 bp, Artificial
  synthetic sequence
tgtacagtgaagcaggttcttgataaactctacaatcactcctgctaacggtccgtatgcaaatgctccgataagtgc

SEQ ID NO: 1802 - DNA, 65 bp, Artificial
  synthetic sequence
ggtgacagtctcttgtatataagcactgtgataagtgttgatataagtccctttacgatggtaaa

SEQ ID NO: 1803 - DNA, 163 bp, Artificial
  synthetic sequence
aagcggcggccgcgtggcggcgctgacggcggaggaaccttcggcggccagcgtcattgacgccgccggactctgcgtctctccgggttttatcgacacacatatgcacgatgaagaggccgaggacggtgacacggtcgaacaggcgcttttgcggcagggg

SEQ ID NO: 1804 - DNA, 150 bp, Artificial
  synthetic sequence
gtggaaatacttcgttccctttttcctcctcctcttcgccgtgcagatggccttcatatttgtcgcggtaatgatcaattatcattaaagattacagtaatggaaaaatttgaacttcttatccggggaggagaggtcatcctccccgga

SEQ ID NO: 1805 - DNA, 165 bp, Artificial
  synthetic sequence
cgcgtacggttacgccttcacaccgaccatgatatcggaggctttgattatcgcgcagacctctttaccctctttaagtccgaggcgtcctgtgctggccttggtgatgatggaggcgatcttctcgccgccggcgagggtcacgaggatctcgcagtttaccgc

SEQ ID NO: 1806 - DNA, 154 bp, Artificial
  synthetic sequence
atcaccgcataggcctcggcgccctctttgaggccaaggttttcgcagctggtctcggtgatgatggaggtgagcatcgtaccgtccgcgaggcgaagcgatacttcgtcgttgacggctccctttttaactgtggcaacagtagcttttagct

SEQ ID NO: 1807 - DNA, 68 bp, Artificial
  synthetic sequence
aaaactttttataaaagaacaagtccatgtaagcagggacttatactctcttacatggacttgtgaaa

SEQ ID NO: 1808 - DNA, 78 bp, Artificial
  synthetic sequence
cactacaggtgccatagcctgcactgtatatactgcaatcctttcctgttctggccgccggaggatttatgttggtta

SEQ ID NO: 1809 - DNA, 128 bp, Artificial
  synthetic sequence
gcggtgatcctgctgtattgattgcatcaagcgataaggcgaaaactgtacttggctggaaacctgagtatgatgatctgggaacaattattaaaacagcgtggaaatggcattcaacacatcccaac

SEQ ID NO: 1810 - DNA, 151 bp, Artificial
  synthetic sequence
tacgaaaaaggaatcattcccgaaaatacagtaacatatcgcgacttatttgatgtgaaacttatggcttcacttgttaagcgaccgtcagaagtaataagagaattttggcagaattatagctgttctcctaagcttgcaaccgatagct

SEQ ID NO: 1811 - DNA, 135 bp, Artificial
  synthetic sequence
acagggattaaaaataaatgtgcgattttcaacaaagcttttaacaaagccgctgtgtgttaaaacgcttgatacaggctgggaatggaatttgtcagggaaagtagtacatggtaatcaacaaaggttatacat

SEQ ID NO: 1812 - DNA, 161 bp, Artificial
  synthetic sequence
ataagtatgctgttactgttggcgttgcccataccagtatagccgccgtagatatcgctgctgacagtgctgccgttaatgatctttactgtgttgctgctggctgaacctgaaccaaaggttcctgttgaggaataccctcccatgacctgggatgctat

SEQ ID NO: 1813 - DNA, 152 bp, Artificial
  synthetic sequence
cgcccgtattttcaaaacgaagcgtattgcctgttttcgcattgccactgctggagtcgccgccatagatggttctgccagacagatctactgcgcctctgatcgtgatgctgttgttattggcggttccataaccagtatggccgccgtag

SEQ ID NO: 1814 - DNA, 72 bp, Artificial
  synthetic sequence
atttgttcctcggcaggaacctgtttgaacgttcattaagtaaagagaataggaaacactttttgtaagcca

SEQ ID NO: 1815 - DNA, 113 bp, Artificial
  synthetic sequence
cgaaagtttcgggcggtggtttcgagcgtggagacaatctcagcgtaggcgatgttccgctcattcgtaggggcttcgtactggaaaatcacgaagaagcgacggctaacagc

SEQ ID NO: 1816 - DNA, 148 bp, Artificial
  synthetic sequence
gggcagggtatccgggtcgtcatagtagacaacacggtaccgcttgctgatgaaccgcagatgccgatgtcggttggcttcgagattgccctgcggtgtaggcgtaacgatacggcggcgcttcataaagcggaaccagtgtgccaca

SEQ ID NO: 1817 - DNA, 156 bp, Artificial
  synthetic sequence
tttgattttcattattattgccatcattggtgtgcgtatgatgagcacagagggcgggtttggggatcgttttctctcaactagtactaaaaatgttagctatcacgagcttaaacagttgatcgaaaacaaagaagtggacaatgtaagcattgg

SEQ ID NO: 1818 - DNA, 153 bp, Artificial
  synthetic sequence
acacccaagagaatgaagtatatacaatttatgcaaaagattttactcttctgcgcagagaccaagaaaatgaatgggtgtgcttgactctgtgcaggcattttaactcttaaggatatctatggacaatcgatcgcaaaatcctaaccccaa

SEQ ID NO: 1819 - DNA, 157 bp, Artificial
  synthetic sequence
atccagcgaacaagcccaatgcacgcgcatgcaaaccaagtactttgctacacttgacaaccactacagcaccctacaacatgcctatacaatattgttgcaagacattgtcgctgcttgccacacccgcgctagcaaacaggccgtattgcagagc

SEQ ID NO: 1820 - DNA, 162 bp, Artificial
  synthetic sequence
agacatccagggcacacctttagctaatggtgtagaaatccagcgtagcgatctgctcgcagaaatgcaagactctcaagaaacccaagccccgctcccccctccaacccagcaatctttccatgccctcttgaataattgtgctaggaacgatctttttaa

SEQ ID NO: 1821 - DNA, 108 bp, Artificial
  synthetic sequence
gcactagctgagcatgtaggaattttcaggacaacagttgctgcatgcttagcaagaatgattgcgggattatgtattatcgcaattgtatcggtatccttctcaacc

SEQ ID NO: 1822 - DNA, 133 bp, Artificial
  synthetic sequence
agtaaatatttatacattccaattctatttacagaaactatcgcattagcaggaataataatttttatttattttatttacaagcatgcagttagaaccggaatttatacttcagacgtcgcagatgaaaatc

SEQ ID NO: 1823 - DNA, 147 bp, Artificial
  synthetic sequence
ggatatctgcgtttagcagctagtgattttctttctaactatgcaactacactagcctcaactactattcaattatggctattgaactcactttttatcggttttcagcagtcaagccattatttatcgctttacctcaccctcact

SEQ ID NO: 1824 - DNA, 120 bp, Artificial
  synthetic sequence
taccagaatattaataccattatgggccagggtgtctgcgatgtctcccagttccccaggacgttcctgaggtaactttcgtatcagaggacggcatacattgctgaccgtaaagccggc

SEQ ID NO: 1825 - DNA, 163 bp, Artificial
  synthetic sequence
acccttgacgagtcagagagggctgaggccaccatcgccatagcggtttccagcgcctcctctggctcactgtcttgctgcggtttcaggagattcattcagaaagtatggcccattttttggtcacttccgctgcccgggcgtcatcatcggtaaggagaat

SEQ ID NO: 1826 - DNA, 163 bp, Artificial
  synthetic sequence
caccgtcttccaccagaaaatgcgcatgtccggcatcaggcgtggtgaatacgccgccgccttcgagccccacgccgttgttacccagcgccatacccattgcgccaagcgagcccggcgagttgctgagaatcacgtgaatgtcatacatctgactgtgctc

SEQ ID NO: 1827 - DNA, 165 bp, Artificial
  synthetic sequence
aaaaatggcggaagtaacacccgacacgattcgttattacgaaaagcagcagatgatggagcatgaagtgcgtaccgaaggtgggtttcgcctgtataccgaaagcgatctccagcgattgaaatttatccgccatgccagacaactaggtttcagtctggagtc

SEQ ID NO: 1828 - DNA, 161 bp, Artificial
  synthetic sequence
tacctgtcaggagtcaaaaggcattgtgcaggaaagattgcaggaagtcgaagcacggatagccgagttgcagagtatgcagcgttccttgcaacgccttaacgatgcctgttgtgggaccgcccatagcagtgtttattgctcgattcttgaagctcttg

SEQ ID NO: 1829 - DNA, 165 bp, Artificial
  synthetic sequence
gcccccgaccgtatgaatgcgacggcctatgcccccaccgagtccaagcgccgcaagccggcgggcccaatcgtggtcttgagcatactgggccttaccttcctctcctttgccggtctgatgggactgatttgggtaaacgacatgggcattatcggcattatg

SEQ ID NO: 1830 - DNA, 163 bp, Artificial
  synthetic sequence
ctccaccattctcgctcctttcgtttgcatagcgcagcaggcggaatactcgggcataatcgattctccattgaacgcagtcggcggctatctcttccttggttattcccttggcaagggccgagtcaaagatcggtaacgcaaaccgaaaatcaaggtctat

SEQ ID NO: 1831 - DNA, 143 bp, Artificial
  synthetic sequence
gagaaggataatatttcttccatgaaatttttgaggaataataatgtaaacgatagattaatatatacgaatgacattgtagaagtagtgatagattctgcaaagcaagaagtgttaaataaaaaaatacttaatggtactaa

SEQ ID NO: 1832 - DNA, 142 bp, Artificial
  synthetic sequence
ctgaacttgatacgttattaagtgataaagaatacgaggctggattagaataattaaagattaagatattattataattggggaaagtatagtaaaatttgagtgcacgcaaatttagctatactttccttttatcatatat

SEQ ID NO: 1833 - DNA, 133 bp, Artificial
  synthetic sequence
ataataagtataatgaaagagaaacttttgaaagaatacattctaaaatgctatgggcgtacatatcctgaagataaaaataatatatacatatattcactgaacatatttgctaaaaaagagatttttatga

SEQ ID NO: 1834 - DNA, 152 bp, Artificial
  synthetic sequence
ccagctgataaaagttggagccattttaaatttttatattttgctaataaatcaggctttggcagaccaactaatacttctgtttccagaaaatctgattctgtcagctcttcttcttttttaaattgaaactggtaagctttatttttctt

SEQ ID NO: 1835 - DNA, 146 bp, Artificial
  synthetic sequence
tttttaacagttttctttttacaaattgacaaaataagagtaaaattaaaatatagataaaaacttatgaaggagtcgcctatgttagataactataagaaaatccttgttggtattgatggttcggtagaagctactaaagcttt

SEQ ID NO: 1836 - DNA, 140 bp, Artificial
  synthetic sequence
actcctttgtataaaatgaattttaaagactacttaaagagaataaagtcaagccttgttttctttatcttctttctttgattatagcactttgccttaattttataaaaaatagaagtttgacaattctgaaattatca

SEQ ID NO: 1837 - DNA, 146 bp, Artificial
  synthetic sequence
tcataagactcttgacagccatttttcacccaatttcctaaaacataaaataaaccagcagccataaaatcgttccaaaatttttgctttgtccctagataatcagcccaagtcgttgtttcattataaaaaatagtcatcttttg

SEQ ID NO: 1838 - DNA, 164 bp, Artificial
  synthetic sequence
cctcgattcatccatgcatactcaggatatctatgttctagggctctctccgactgtctatattagagggaactatcacgtacagcactaccgtgttcgaggattttggccctcttgcctggattctctagcggcctgtgcggaaaatacatcagtacttccct

SEQ ID NO: 1839 - DNA, 159 bp, Artificial
  synthetic sequence
tctctattcagccacacatttgataacgcgatacggtatggtgagagatgcctgttggtttgttctgagggcatgggaatgcttccagaaacgcaacaacaaacatctcctttaacttcactagaagggggacatgaggtagctctagttctcaatccc

SEQ ID NO: 1840 - DNA, 127 bp, Artificial
  synthetic sequence
aataattttaataatgatttatcaaaaataaatttaaaaggtgatgtaagtattgaaattttaagtttacaaaaccattttaatgaaatgatagataagattaaatatttaagagaatatgaaatta

SEQ ID NO: 1841 - DNA, 102 bp, Artificial
  synthetic sequence
gaaatttcatatatgcaagaaattgacagcttaaaaaatcatttttttgaaatgatagttataagttgtttggcttctcttttaattacagttttaataaat

SEQ ID NO: 1842 - DNA, 111 bp, Artificial
  synthetic sequence
ttaatcgataaaaatccacgcctttagcactgtcctgtaggtgcctttttccgtatcggtatctcaatggacatccctaatgcttttgggcgtttttttgtcttttaggct

SEQ ID NO: 1843 - DNA, 153 bp, Artificial
  synthetic sequence
aaaggatctattcggtggatgagtcttcgggagagatcgaacacgaaagacgattctttttcaatgaaggcggatatatgattcgtgaggaggaatacgatggaaccgttcagatacctgtcagaaaatgggaatttgtccgcgatgacaagg

SEQ ID NO: 1844 - DNA, 151 bp, Artificial
  synthetic sequence
agctaagcaatttagtcaagcttttaccagataggggttgagcagggataagaatcgtatctgcgccaaaaagagcagattctaaaatctgatattcttctaaaaaaatatcgctatggataatcggaagtgtgctatgacggcgcaaaag

SEQ ID NO: 1845 - DNA, 140 bp, Artificial
  synthetic sequence
ccagataggggttgagcagggataagaatcgtatctgcgccaaaaagagcagattctaaaatctgatattcttctaaaaaaatatcgctatggataatcggaagtgtgctatgacggcgcaaaagagcgatggattctaa

SEQ ID NO: 1846 - DNA, 141 bp, Artificial
  synthetic sequence
aatcttcaattactgtaggtatatcatttataaactcaatgacattatcaccaaattcatcaaaaagtttttcatttatgttatcaattataacggcagccattaaatgatgctctttaagatatttgtttaggtcttttc

SEQ ID NO: 1847 - DNA, 162 bp, Artificial
  synthetic sequence
gacgacggcatcagcgtcatgggggttcagcaaaatgtcggatccggcttcgaaagcctgcaccgcaacacgcccccggatcggtttcataaaggcgttgaactcggcactcgcatgcccctcatcggccgccgtggggtcattgccctcggcgtcggcagc

SEQ ID NO: 1848 - DNA, 163 bp, Artificial
  synthetic sequence
caggcttctcgcggcggcgacgggatcgtcgctggtgtcgcgaatccaccggattgtcgaccggctcaggtgccgtaacagatcggccggtgaatttggtccggacaaggtccggctcgtgtatccccagtatggacggccccggcctgctgctgggagtttc

SEQ ID NO: 1849 - DNA, 162 bp, Artificial
  synthetic sequence
gactgcgaggtctacttgctcgtggtgagctgccaggacagtggtggtggcgctggcgcagaacacgtcgggagtgccttctcccacgtccaagcggctcgacaaatcgagggtgacgaagtgatgatcgctggtgtgcatggggcggtgcgtgctcaggcc

SEQ ID NO: 1850 - DNA, 162 bp, Artificial
  synthetic sequence
ggacatcgctgagctggtagaccgctccgcgggcggggtgggcggtggggtcaccgacgccgaccagaccgcctccggctgcgacaaatctgcgcactgccgaggtgacacgctcgtcggcccattcggatccaccactgaacgcagtgccggcggcaccga

SEQ ID NO: 1851 - DNA, 151 bp, Artificial
  synthetic sequence
gaattattaaaaacctatcgagaaggagttttttcagcttggctcttactcacctatgggaatcggcagacaccttataattttcttgtttattacgagctattctcagctcttccagacactcttaaactcgagttagaaagactgcctc

SEQ ID NO: 1852 - DNA, 142 bp, Artificial
  synthetic sequence
aaatattttaaattttcaaaatgattttaaaaatgttaaacttgtaaaacttgaacaaaactatcgttcagtagggactattttacaagcagcaaataatctcatatctcacaatgagcaacgacttggaaaaactttaatc

SEQ ID NO: 1853 - DNA, 143 bp, Artificial
  synthetic sequence
cttagaaaatgtaagttttcacttgaacttaaagttaaattttcatcaatttttacaaaaggtgctttaacattatcattcataaaagcaaagttaaccccttctatattcttaacttcacctttttcaaatttaacatcaac

SEQ ID NO: 1854 - DNA, 135 bp, Artificial
  synthetic sequence
atatatcgctcaagaagtgaaaaaattgctaaattctggagtagaagctaaagagatcgccattttatttcgagttaatgcactatcaagagcaatagaagaagcatttatgaagaaacaaatttcttataaact

SEQ ID NO: 1855 - DNA, 142 bp, Artificial
  synthetic sequence
aattattattttctttataagtataatgagcatttaagattaaatctttatattttaatacagcttgatcatcacctaaattaagttttagtttaaaagaattagcaaaaggcaaatttcctatataacgatcattaaccgc

SEQ ID NO: 1856 - DNA, 145 bp, Artificial
  synthetic sequence
tttgttctaaaattggttttataaattcttctaaagaatccatttttccagtatcatagaacaattcttttagcctaacagtgccaatatcaagagatatgcaagaaataattctattattttttattaaacacaattcactaga

SEQ ID NO: 1857 - DNA, 162 bp, Artificial
  synthetic sequence
tctcactcaaattccgctcaaaactgttcgacaaagcattctcatacttaccatcccaatcataaatgaaaagatccaactgtaatccaccgaactgcatcggctcggccggagtctttttatccggaacataccggctgtgccgatctctcaaccgcgcct

SEQ ID NO: 1858 - DNA, 153 bp, Artificial
  synthetic sequence
accggtaaaagccaaacaggtacgtcttcgtatcctcgacggatttgcctgtcctgctatccatacattcggagtgtacaaacaatcggctttatttcagtaaaaacaataggtagttgggttgaatataggtttgggctgtatcacacaggc

SEQ ID NO: 1859 - DNA, 119 bp, Artificial
  synthetic sequence
gcctttcctcttccgggggaaacgttctataatctccataacaacgggtcagataagcatcgtatcctgacggaaccggaaactccactccttcaaatcgtgcagtatccagatattcc

SEQ ID NO: 1860 - DNA, 109 bp, Artificial
  synthetic sequence
taatctttaatattggattttattggccagcttatcctattgccttatggatgattctagctctgttattaattgctttacaaattattcacaatcatgaattcattta

SEQ ID NO: 1861 - DNA, 155 bp, Artificial
  synthetic sequence
ttaattggtaacttggataacttgattgtaaaataagacgttttaattgtattgctgctaacttgtggtattatagatactagttaaatgtaaaaataggtggaggtcgcattccgttaggttgcgacctttcatttcgttgctgttcgcttact

SEQ ID NO: 1862 - DNA, 130 bp, Artificial
  synthetic sequence
taaccactttacaaatttaactagtaatagttcaaaagttgttaaaccaaaatatgttgaaaagaaaaatgtaaagcttgttgcactaggtgattcccttactcacggtcaaggggatgaaactaataat

SEQ ID NO: 1863 - DNA, 102 bp, Artificial
  synthetic sequence
attcggcatattatgctttaactatatatattggtagcttaattatttcaccatggttaccgttgatataaaaatattaagtgaattgaggctgggagaaaa

SEQ ID NO: 1864 - DNA, 92 bp, Artificial
  synthetic sequence
atcaagcaccacatgcgcaccccgcgcacactcgaccgcagcctgcagccgctcaccagcctcacccgcggaaaaaccagacgtgcacccag

SEQ ID NO: 1865 - DNA, 165 bp, Artificial
  synthetic sequence
cactggggtcatcacctcaactattggtatttgcgtaaaaagattgtaacgacccaatcttttgcgcaagcgccatcatttttgtgatagtcttaaatcatcatgaaacctttctgaaaggaagtctcacaattgaaaatgatcaatctcgggcgctccggctta

SEQ ID NO: 1866 - DNA, 157 bp, Artificial
  synthetic sequence
ggggaggcgtgcacatgcgtgatttggtcaaacttgttggcttggacctggctgtatttcatactaatagtaagaagtatttttggtttggtactttgatcagtatcgttttgttgcttctccctttcttgaacggtgacttagcaaccccgcttgc

SEQ ID NO: 1867 - DNA, 155 bp, Artificial
  synthetic sequence
catgcgcctaccgaatcttgatcgtccgcgcgcaacggaattgctcgatgctgcttacgatgtcggaattaacttctttgataacgccgatatttacagtaatggtaaggccgaacagttattcagtgacgcactgaaaaaagcgagcttcaccc

SEQ ID NO: 1868 - DNA, 150 bp, Artificial
  synthetic sequence
ttcgttgaggttgacagttccggtaccgtcaattcttaccgggatgtttccagttgcaccggtaatggataccgttgcattcttatcaacggttagattaccaccgtcttcaatatagattggtgcaaagccatctttcacaagtgcatt

SEQ ID NO: 1869 - DNA, 140 bp, Artificial
  synthetic sequence
acaatcgttgggagtcaacttcgctaaggatactaaaaagttgcagatcggggggaatgtacaatatggacattctgataatgacgctcgtcgcaaaacctcttcagaaacatttttgggggaaacatcttcttttgctc

SEQ ID NO: 1870 - DNA, 113 bp, Artificial
  synthetic sequence
gatcggtatgaagggggagtaatgatcagccgctttaaagatgatgcgagtctttcaattataggttctgcaaataatactaataataagggattttctgaatttggtgatgc

SEQ ID NO: 1871 - DNA, 82 bp, Artificial
  synthetic sequence
agtatctgatgcggtaaaagcaattcccctatatcgcatggctgagaaaggattaagagaggatgggtatccgatgggaccg

SEQ ID NO: 1872 - DNA, 74 bp, Artificial
  synthetic sequence
gggttcaattcccctcatctccatagataaaaatagaaccgctctagtaagttgtctagagcggtttttttgat

SEQ ID NO: 1873 - DNA, 75 bp, Artificial
  synthetic sequence
tggtattacttttggaaatggtgaatctcctttaaaagaaacaaagaatataaatttaaaaaattcaattttcaa

SEQ ID NO: 1874 - DNA, 134 bp, Artificial
  synthetic sequence
gtgaacagcagaatatgggctatgccgtccagcgacatttctccgtactgcagaaacctgctcatttccggctcaccgttcagaacgccgaaggtgcggttcatgctgcggcgtaccgatacaatctggtcgtg

SEQ ID NO: 1875 - DNA, 162 bp, Artificial
  synthetic sequence
gctgattccagtatgcgcgccgatgtgcgggcgccgtccagattgatgccggttttttgcggacgccgcgccagcgcggcctgcatcagctctgccagcttgtgcggttccagatcgtcgggctgcaggatgcgcagggcgcccagacgttcgagccgcagg

SEQ ID NO: 1876 - DNA, 155 bp, Artificial
  synthetic sequence
tccgtctgattctagccttgcacaactatgatatcactatacatgaacaagacaaacagacagcattgcaacaaataaatgaagtgtgcaatgactttcagaccatgagaaaacaattggaagagacctattcacagacccgttttatggaacaa

SEQ ID NO: 1877 - DNA, 162 bp, Artificial
  synthetic sequence
ttccgcctccgcacgggtaaggggcagcgtattgtcgggtcgggtgaaagccaccaggattttcaccgaatgtccgctggcgcccataaaggcgcaccgcgtctgcggcaacttccatgcctcccgtttcacctgctccacttccgccctgcccgccaaggg

SEQ ID NO: 1878 - DNA, 156 bp, Artificial
  synthetic sequence
tgatggttccccacactctgaaacggtgtggcgtggatacatcgcacagggagaatatggctggaacccaacagcacggacagtcgaagccttcaaagccgcacatgcccaacgagaatttggctttcatccaaatgacaaccatatggcttttct

SEQ ID NO: 1879 - DNA, 164 bp, Artificial
  synthetic sequence
ggttagttatcccaatatcccgatcatccggaaatatccgaatatgacgggcttttatgataaaccggattataagaggaatatagaattgatacggcggcttgttggtaattgcattgtcataagagtctcggacgatacctttcaggataatatgatgctgg

SEQ ID NO: 1880 - DNA, 161 bp, Artificial
  synthetic sequence
aaagataagggttccccatgaacctcttatcatccgttcggatcatttccggttgacgcaggtttgtaccaatttcattaataatgcggtgaagtttaccgctaagggatatatcgagatcggatacgaacttagcgcagatggaaaatcgatccttattt

SEQ ID NO: 1881 - DNA, 138 bp, Artificial
  synthetic sequence
attaccaaaaacagtgacctgttgcttaagctgatcaacgatatcttggatctatcacgcatagaatccggtagcatgtctttctcttatgagaacctcgatctgagtaaactgatgggagatatcttccatacgcat

SEQ ID NO: 1882 - DNA, 145 bp, Artificial
  synthetic sequence
cgtgaacaatatatattccttggatcgggtacgtttatccggaaagaacgggatttcgatatcggatatacctaagataaagccggatacgatgtatataagcacactcagtacgaaatcggcgaatgccctgattaagggattt

SEQ ID NO: 1883 - DNA, 160 bp, Artificial
  synthetic sequence
gcaggagattccggcggttgaacatggggaaaatgggcattttccagttaaagacacggacaaacgcaagctttttaaaggcaagatcaattaccggcaagcccaagtggacttaatcgaccgcttgcacgactttgtcgaagatgccgggcaaagggtc

SEQ ID NO: 1884 - DNA, 162 bp, Artificial
  synthetic sequence
tttgctcaagcaggatccggtttaccgggaatttatcacttctctggccagccgctaccaaaaccgcccaagcgaactgcccttgatcttggctgaaggaaatttcgcttttggccagctttatccctgccagggagattacgtgactaatcccgatgcttt

SEQ ID NO: 1885 - DNA, 160 bp, Artificial
  synthetic sequence
tagcccagtacctgcgccaggagagccaggaccgggacttccgcccggccagctaccggatgacggaagacttgtctaattgtgaagaggtcatcttggacctgctccgtgatgaagacggcaacctctgttttgtcggagcgactgggtctttggaacc

SEQ ID NO: 1886 - DNA, 164 bp, Artificial
  synthetic sequence
gaccgatgtaggcggtatagtaggcttgtaaaaatgtgcctaaattcttagcgacatagactatcacgatgccaaggggcagcagataaagccatgttttttctttttcgatgaaaatttcatttagcacgggctttaccatatatgcagtcgccgccgtgcct

SEQ ID NO: 1887 - DNA, 132 bp, Artificial
  synthetic sequence
gttcctgtaattacaacagttttttttgtgaaaacattttgtgaaatttcagttttttgggcgcttaaatgcaaaaaagaaagtaaattttcaattttttcgcgatttatctcacaaaaaccgacaaaactt

SEQ ID NO: 1888 - DNA, 120 bp, Artificial
  synthetic sequence
atttttaaaatttcatcaaaacttgcattcagccaattttcgccaaaaatttcagcgatttttctggcggccacttcgcctatatgttcgattccaagtgctgtaataaacctataaagt

SEQ ID NO: 1889 - DNA, 69 bp, Artificial
  synthetic sequence
ataagtgcgggtgctagcacacctgactggatcatacaaaaagtcgttgacagaatcaaaaaagtataa

SEQ ID NO: 1890 - DNA, 102 bp, Artificial
  synthetic sequence
agggcttccttgtacttgccttcgcggtacaggttgcggccttccgcaaggagctgcatggcttcctgggtttgcgcttcgcggcgggccatggctgtgcgc

SEQ ID NO: 1891 - DNA, 75 bp, Artificial
  synthetic sequence
atttgtttggcgtctcccggaatccggaagtcggaaccttcctctacttcaaagctggtatcccgttcggggccg

SEQ ID NO: 1892 - DNA, 135 bp, Artificial
  synthetic sequence
cttttcatacgagaaaatattatcaactgattgctcccctatatattccgcagctttatgttttaaaaaatcaagatttcgctctttaaccgcttcgggtctaaaccaactgcatatgaatacagaggttataag

SEQ ID NO: 1893 - DNA, 132 bp, Artificial
  synthetic sequence
tgaatataaagcggcatcttgctcgattgttccaatgatttctccattaacacttacaacccacaaaataccaccgtctaataattcattgtttttctctacaattgataaaattggaccagatatatacac

SEQ ID NO: 1894 - DNA, 102 bp, Artificial
  synthetic sequence
agctatggaacgctctttgcgtgctctaaaaggttttgtacacatggctgatgcaatggaggcaaatacgattaaagctgttgctaccgcagcagtacgttt

SEQ ID NO: 1895 - DNA, 77 bp, Artificial
  synthetic sequence
aatggtactagcgtgtactattgcaccatggccaattgttacgtaatctccaagaatgcaagccctgtcgtcatcaa

SEQ ID NO: 1896 - DNA, 77 bp, Artificial
  synthetic sequence
tatccgcttttaatgtatatgtaattatacgattttggcgttcttatcgtattcctcgccacccgcatcaggaagca

SEQ ID NO: 1897 - DNA, 160 bp, Artificial
  synthetic sequence
atgaataaaatttatttctctcaagacccggtgggtttttatatcgaaggtgtgtctgcggttccctccaatgctattgaagttagcgcggatatttataatgagtttgccggagtggcgtggcctgatgggaaagtactaggtgctgatgattcaggat

SEQ ID NO: 1898 - DNA, 164 bp, Artificial
  synthetic sequence
gccatgatgaattgattgcacaagcggaagccgaaaaacaacggttgattgatgagaccaacgtctggataaacgggcagcaatggccgtctaaattagcgctgggccgcctctctgaggatgaaaaagcgcagtttaacgaatggctggactatctggacgcg

SEQ ID NO: 1899 - DNA, 63 bp, Artificial
  synthetic sequence
cgatattgatgatacttctttttaaagttgccattttgatttcctccttctagtgattaatag

SEQ ID NO: 1900 - DNA, 114 bp, Artificial
  synthetic sequence
ggttcataataggcacaaagcggctgccacttgtaaagtcagaaataaacgataatggattaaaagaatagccttggataccgatatttttcagcaaaatcacataaatcaaaa

SEQ ID NO: 1901 - DNA, 161 bp, Artificial
  synthetic sequence
cgatcgaaccttttatcatcttcattcctccaatattcttgtccattcatgaactgctgggccagccatttgtatcgcatcctcaccagagatcatcaagtctccttgttccaagtgaacaactacctgatctgctgaaattttcccagtttccttagcaa

SEQ ID NO: 1902 - DNA, 146 bp, Artificial
  synthetic sequence
gggaatcagcactggaaacaattttttctgtttttgtttccgttactttttccattccaaagtgattggacaaattagcgacgatcaaacttagtgaagcgacgaagattagtccgaaaatcaaagataaaaaggtttgccatgtt

SEQ ID NO: 1903 - DNA, 159 bp, Artificial
  synthetic sequence
gaaaatatctctgctaatatattggttttcttttgataaaatatagtgaatcgaaacggcgcttggaaaaacattcgtgcggatggataattgaccgcttctctaaccgtaccgaacaaaagataatcttttaaggcttcaactgccaaacgtccgctg

SEQ ID NO: 1904 - DNA, 144 bp, Artificial
  synthetic sequence
tttagtagttaacctaaacctggtcatctaccatctgtacgtactctaacacatcaaatcctagtcttttataaaggtctatagccctcttattagttccacaaacttctaacctataccttactgcttcaggaaagttttcct

SEQ ID NO: 1905 - DNA, 147 bp, Artificial
  synthetic sequence
gtattcttcacttatataaaggtcctctagctgtatggtgattcctgccacctctgaagcataatagctggttactataccaaacccaaccaaatttccatcataccttgcttcatatccccttatagaatgctctcttgataagat

SEQ ID NO: 1906 - DNA, 141 bp, Artificial
  synthetic sequence
tttgttgaaccttcaaaaagaaataacttcacaaaaaatgttttttcttacattacaagagatagatttgattttggtgaagcttttaataataactatgatttcttttcaactatttttgaatacctaatttcagattac

SEQ ID NO: 1907 - DNA, 139 bp, Artificial
  synthetic sequence
agatgttgcattcaaatatgaagatacaattgattatttagttggatacattaatgaagatgatttttatcaaaaatttgacgatacattaattagaatttcagattataaacaaaatgaagcttttaatgttgatact

SEQ ID NO: 1908 - DNA, 156 bp, Artificial
  synthetic sequence
accgtcgaggaggtcacgcaggccctggcgcagctcctcggcgtaggcagactggaccggcagggtctccagggcctggtacaaagactgggcaagggcggaatccatcatgataaagcttgcgttttttttcatctgggttcctcctttctagat

SEQ ID NO: 1909 - DNA, 124 bp, Artificial
  synthetic sequence
aaggcagaggtatcaacacccggagggcagtctgccgcctggggatacggcgggcacgccgcctgcccgcaggcctgcttttctgatcgttttgtcggttccgctgttactgcaactgtccaag

SEQ ID NO: 1910 - DNA, 156 bp, Artificial
  synthetic sequence
agatgcagaggggagaaaagaattggaagaataatgttttaaaggcattctcgtcgtcgtttacagcgatgttccaaaacaacttgtcgattgtatgtggcagtgtctccttcatgttttcgtttgatgacaacaaatatttactaagttctcata

SEQ ID NO: 1911 - DNA, 161 bp, Artificial
  synthetic sequence
gtgtaattttagaaacaaggccataagcgcttgacaattccacctgttcgatcggctgattttccaatctgtagatacgctggtaaaagtagatactgctaattaaggctggaatgagcaatatggctgccgtgtaacgaaaatagcgaccgatcttttgt

SEQ ID NO: 1912 - DNA, 134 bp, Artificial
  synthetic sequence
tcggtgcagatcttgttccgggtctctgtatccagcgtttctccgttggaaagcagattgctggcattgccggaaatggaggtcagcggggtgcgcaggtcatgggagatcgtgcgcagcaggtttgcccgcag

SEQ ID NO: 1913 - DNA, 153 bp, Artificial
  synthetic sequence
gcccacgggggtgtatttgatggcgttatccaccagattgacaacgacctgcatgatcagccgtgcatccacattgaccaggaggatctcgtccccatactgtgttgtgatggtgtgttcgcagcttttccggttgacatgatgcagtgcttc

SEQ ID NO: 1914 - DNA, 163 bp, Artificial
  synthetic sequence
gtcttatccatcttgtcggacacgacaacgccgacgcgggtctttctcagattacgttcttccatcgtttaacctccttactgcttctcagccagaacggtcatcacgcgggcgatgtccttcttgactgcttcgatgcggccggggttctccagctggttga

SEQ ID NO: 1915 - DNA, 159 bp, Artificial
  synthetic sequence
agaatcctctttttcaatgcccaaaagcgtggtagaatagggaaaagattcagtatctgaaaaacggagcgcgcaacaatgaagattctggtcagcgcctgcctgctgggcgaaaactgcaaatacagcggcggaaacaattacaatcaggcggtctgt

SEQ ID NO: 1916 - DNA, 129 bp, Artificial
  synthetic sequence
atatgccctaacaagtcctcccgctcctagtaagattccaccgaaatatctagtggaaatcaccaagcaattagttaagtccttttttcttaaaacttcaagcattggaattccggcagttcctgaagg

SEQ ID NO: 1917 - DNA, 150 bp, Artificial
  synthetic sequence
attaatttttctctatcatttataaaatttttcataaattcaatctttttattttccataattatccccaaaatattattataaaatcgcattgattatatcatatatattagttagaatcaatttttgaatcttttttaatttcataaa

SEQ ID NO: 1918 - DNA, 163 bp, Artificial
  synthetic sequence
attggccgcgtacttgcggttcaggcggtggcatacgtggtgctattcggcgtgacgggcgtgctggagttcacgttcgggaaccagggcggtgtggcgcaaggggttgcgatcgcgctcgccgtggtgctgctcgtgctattccaggttgggtggccgttcc

SEQ ID NO: 1919 - DNA, 142 bp, Artificial
  synthetic sequence
tgccaattgccggcgtgcgttgcgtgtgattcaggaggggacggattcgtcgatggaaacgcgcacccgactcgttcccctcaaatacgggatagacgcgccctgcgtcaattacaagattggagtgaagcgtctgaaccgg

SEQ ID NO: 1920 - DNA, 162 bp, Artificial
  synthetic sequence
tagggactgtccctaaattaaagttctaaattgaggttgacagccctaatcctcttcgatgcctaaaaacacctgtgtgcgagggtagtaaagcaccgtcgacccagcctcggcgctggtgagctcggaaaggactcgcggccaatcgccgcgcttgaccga

SEQ ID NO: 1921 - DNA, 154 bp, Artificial
  synthetic sequence
gatctccccctccacatcaagaagcacaccgcgggacgcattctgccttaactgtaccagataatccgcatactccatgacgaatctgcggaaatgtgaaaggcttcctcggatcatatgtacctgaaacgcattttcgcagatatactgtaac

SEQ ID NO: 1922 - DNA, 143 bp, Artificial
  synthetic sequence
ccatcgcaagggaaaccagacggtacaggagataattcatgttcatctgtaccaattccgggttcattcccgcctcattcatctcctcatagatcgctgcaacattatcctcgatccttttcttgtcattctcttccacactc

SEQ ID NO: 1923 - DNA, 78 bp, Artificial
  synthetic sequence
tgtatcaagagtggtcaggtcgacaggttcaaccttctttactgcatggtgacttttggcgcggcaatgtgctgtttg

SEQ ID NO: 1924 - DNA, 76 bp, Artificial
  synthetic sequence
attgcttgcccagtttgggttatccggaacattaacgccgatcagcgggggtgacgtgaatcagacgttccggttg

SEQ ID NO: 1925 - DNA, 78 bp, Artificial
  synthetic sequence
ggcgtcttgtttgcatgtatgaggtatggttctaaaaaagcaagaaatggggcgactgctgctgcatttgtgcaagca

SEQ ID NO: 1926 - DNA, 152 bp, Artificial
  synthetic sequence
tataatcatactataggcattagagcatcgacgactttcggtataggcaattggatgaacggaagtgtttcggcaacaggaatctacagacatgacaagagtaacgatttctttgacttacccttcaatcgcaaacatatctctgccattct

SEQ ID NO: 1927 - DNA, 156 bp, Artificial
  synthetic sequence
gaagccatcacatccatttcatacttaacccattctatcagtcgaaagccattcaaggactctatgacatcaaatcagtctttctcttgattgctatgttgagatgggcttccgataatgataaatggagcattgtggttaaaggcagcaacatct

SEQ ID NO: 1928 - DNA, 146 bp, Artificial
  synthetic sequence
gttcttctgctcaatattgtgctgtattcacctcgtctgcagtatttcttgctttggctgccttcaactattgggcatcctacaagctcttcacccgtatgcaggttatctgcaacaagtggatcaacatctaagaattaaaattt

SEQ ID NO: 1929 - DNA, 151 bp, Artificial
  synthetic sequence
cagtctactccttcctgatatttgcccattccttcgcaaccctgggaggagccttctaccgtaagtttcctgtgcttctgacagcatgtacgggattggcactttgtctgattttgggttatattatcaacgaactgggtgaagccggatg

SEQ ID NO: 1930 - DNA, 156 bp, Artificial
  synthetic sequence
cggcaacaggaaacatattgcatctcactcagcaaaaaaacacgcctgcatatcaacctcaaatccctgaatccttttgctttactgggattacctagacagcaggcaaaccgtttccacatggcacgaagcttcagatgaatgtcagcgcatctg

SEQ ID NO: 1931 - DNA, 161 bp, Artificial
  synthetic sequence
ttttttctttttccaaccctatacgattttatagctcattttctaaaaaccctacaagattttatattaccgaaaaactttaaattaataaggtgtctttcaatgcacttattgcttaagacctatccccattttcctgactaatgatatcctgacttttc

SEQ ID NO: 1932 - DNA, 73 bp, Artificial
  synthetic sequence
tttgattgacttcatctttggtgaaaatttgatttatgatttactaacagattctgctgaaaatcttattaac

SEQ ID NO: 1933 - DNA, 74 bp, Artificial
  synthetic sequence
acatgattttcaagcagtcccgcaggatactgacttttatgctgagattgatgaaaaatttatcgccccattac

SEQ ID NO: 1934 - DNA, 114 bp, Artificial
  synthetic sequence
aagagaataaatagaaaatggaattaataatataggagtttaaaatgttaattaatatgaaagaaatgttgaaagttgctaacgagaataattttgctgtaccagcatttaata

SEQ ID NO: 1935 - DNA, 139 bp, Artificial
  synthetic sequence
gcagagtatttcctgtggcggctattaaggttatgttgctgtctaataatttacttactaatttttttatattatttatattatcttctttgttaatagtgtttattaaacttttttttctatttaaaaaaaattctat

SEQ ID NO: 1936 - DNA, 136 bp, Artificial
  synthetic sequence
ccaatatctcttaaaagtaaaattttcatttggtaaaaaccgtcaaaaccagaatgttgacacattctaacaacagttgcatcgcttacttttgtttcgtttgctatttcttttacactcataagagttactttgt

SEQ ID NO: 1937 - DNA, 161 bp, Artificial
  synthetic sequence
ttgcaatgcgattgtccctgtgtcgccctgaccgattatgattggcgaaaccagctttcgtccgttcatgactcgattgtatttgtcgatgagggcttaaaagagatccattctgatgagtttgcccatcatgtgctgtattcctcgaattatttcgtgct

SEQ ID NO: 1938 - DNA, 154 bp, Artificial
  synthetic sequence
tggaaaatccgaaaagtaaaattaaaggtagtaatacggaaaatacggaaacaaaagaaggggctgttcgctttgatattattttttatgttcgaatgaaagatggaatttctcagattattgtgaatatagaagctcaaaagaatagttcgcc

SEQ ID NO: 1939 - DNA, 148 bp, Artificial
  synthetic sequence
tgaaagcgcagtatgacgagaatgccaaaaagcttttaagtaacaaaatttttctggcacatattttaaaaggaacagtaacggaatttaaagatgcgaatccaagagatatcatttctttgattgaaggagaaccatatgtatctac

SEQ ID NO: 1940 - DNA, 158 bp, Artificial
  synthetic sequence
gatactgtttcgggacagtaaccagcgtatgatcgaagggaagcaggtactgatcctgacagattctgtgacgaccggtgctttgcttgcaaaagccgtggaagcagtgctgtattacggtggacgtgtatgtggtatctgtgcagtattcagtgcgg

SEQ ID NO: 1941 - DNA, 160 bp, Artificial
  synthetic sequence
tatggaactcactggcatataatggtgccagatggattgcatccgggcgatatcattacaatattgagactgtgttggatgagaggatccctttcataccctggacattggtaatctattttggatgttatctgttttggggaatcaattacattttgat

SEQ ID NO: 1942 - DNA, 142 bp, Artificial
  synthetic sequence
atatgcggattttaaattttgtgtatttctcataatatatccttgagaaagaggttaaaatataaaaacataataataaattaatgtttaatgtaagcttaagggattagtaaaatttaatatgaaatataaattcttatat

SEQ ID NO: 1943 - DNA, 141 bp, Artificial
  synthetic sequence
caaatttatctttttttgagtgccggtaaaataataatatttttgagcggtggtgccgttttctatgtttgagtttatcgtagcgaaatcggccgcaaaatttgaaacggcgagtaaaatagccgttgccgcaaccgaact

SEQ ID NO: 1944 - DNA, 122 bp, Artificial
  synthetic sequence
tatcaaaaacgtaaacggtatcggagaaaagacatttgaaaatttaaaaggcgatatctcgataagcggcgaaaacgtgatgcctgcaagcagtaaagtgtctaaaaaagtaaaagaagcta

SEQ ID NO: 1945 - DNA, 166 bp, Artificial
  synthetic sequence
cacccccggcttcgacgacgcctaagtcttccgaggtgtacatccagtgctggacatcgaggtcaggaggaccgagaggagcgtcgacaccagctgctgtccacgccagagcgttcgccgaacggcggacgtcggccccgatccaggcaagctcgtcaagcgccgc

SEQ ID NO: 1946 - DNA, 164 bp, Artificial
  synthetic sequence
gtgttctaccgaacggccagaaccacatcactggaagggacaggatgagggcaagaaacaccgtcacattgagaataaaattcaaagaagaggtaaacgccttcagaacccgaacaatcgatctcaacacattcatctcttttcaagtggatgacgatgccacc

SEQ ID NO: 1947 - DNA, 162 bp, Artificial
  synthetic sequence
ttcagttccgcgttcacttctgaaatattcatcggttgtattcgtttctgggattcgtggggttggacttttgacatgcagtcgcaccgagtatcagactcccgggaaggtcccgtccccgaggaattctctgcgcctcggcgcatatggaccgatgcccgc

SEQ ID NO: 1948 - DNA, 120 bp, Artificial
  synthetic sequence
aagctcagtgctttcaaaaaaccttaaatttttgcgcggaatttcggctaaaattttatctttaaagccctcataatcgttagttaaaacgatctgatttatgattttcaaagcaccact

SEQ ID NO: 1949 - DNA, 155 bp, Artificial
  synthetic sequence
ttgtctaaaattttaaaaagctgaatcagtttgagatctaagctcggatcgctctcgctcatgtaaaagctattttgtagcctctcatcgatgagccacagatagctatcctcgtggcttttggcgattttggctaacggatggttgccgttgcc

SEQ ID NO: 1950 - DNA, 159 bp, Artificial
  synthetic sequence
gacattagtattatctaaaaacgagattacgatgtcaaatttacgactttttagaagcctgtgcaaggctaaaattttatcatagcgcttttttatatttccaaaaactcctaaatcgcctacgcccaaatccaagctaataagctcgatcttaggatc

SEQ ID NO: 1951 - DNA, 120 bp, Artificial
  synthetic sequence
tgactttgttttttgcctgaagcacagctaggcctaaattttgaatcaacggcacgcttactggaagcaccaaaataagcgcgattgcgtatgagatctcgtaattcgcgcccgcccata

SEQ ID NO: 1952 - DNA, 104 bp, Artificial
  synthetic sequence
gaggcccacaatatgtatcacggtgagaaggttgcctttggaacttgtgtacagcttatattagaagatgctcctttggaagaaatagaagaaatatataattt

SEQ ID NO: 1953 - DNA, 153 bp, Artificial
  synthetic sequence
cactatacacaatatgccattcgaagttaacgaaaagaaggtatacagtgcaattatcgctgctgataatatgggaaggaagtatttaggcaaataatcgagaattaggaggtaataaaatgtcaaatgtagagtcaacaaaatacaggtgta

SEQ ID NO: 1954 - DNA, 130 bp, Artificial
  synthetic sequence
ttgtgctggccatcatcactacgcgtgtcaggcattagcacaacatgtgttgattatcagctccaatccaactaaacatagtctgatttataataacttactacaataactataaaagatgaattattat

SEQ ID NO: 1955 - DNA, 164 bp, Artificial
  synthetic sequence
tccggctccgtttttatcaatcctgttgtatggatcgcgttctgttcattatcttatgatggtctttttgccgttgatgacatagacgcccttgcccaatgacttcagactcttcgcatctttgagaacctgtttgccgtcgagtgtgtagacatcatatagaa

SEQ ID NO: 1956 - DNA, 151 bp, Artificial
  synthetic sequence
tctggggtctctatgccccaacatgttgaggttaggtccttgaatcaccaaaattttcatgccattctccttaccaagtgaaagattaaagaggtcattatagcataaaactcccgtttaaagcccaaaggcttagagtgtgaaattatgg

SEQ ID NO: 1957 - DNA, 149 bp, Artificial
  synthetic sequence
gtaagttttgatacaaccaatggtgttaaaagccgtccaaggactatcaatatgcaacttagcctgtttcatacccgactcaatttgcaccaaattatctaaaaacttatggttgaagtcttggatttttaaaatataaaggtgcaaaa

SEQ ID NO: 1958 - DNA, 149 bp, Artificial
  synthetic sequence
aaaagaatattaccatgaagttcagttatagcaaacccacgcccaagcacatggtggatttactcaccaaagtttgggttttttacatgtgtttgtccttgtgtctgatttggggactagcctattttttacgccactacaccaaagcc

SEQ ID NO: 1959 - DNA, 141 bp, Artificial
  synthetic sequence
accaaagaaacaattccttttgcggcaatcgtcatagtggattccgacgacattttagattcgaaagcctatcttgaaaactatgccagcttcggtgggtattttgatttttcgctgagcgatgaaatgatttatggcttc

SEQ ID NO: 1960 - DNA, 142 bp, Artificial
  synthetic sequence
atattatttaggatggatcgaaagccaaaaagtagaagctgatttaacaaatgaggataagcaaaagtagacgaagaaggagcgggaaaggatagttatctcgctcttcttcgtctatttggttaggatttatcagggttaa

SEQ ID NO: 1961 - DNA, 163 bp, Artificial
  synthetic sequence
ttcaagtcattgatacgtacctgatagttggacacgtcgtctatattctttgtgttgtccttctccgtaggcacataattcgcatctgtcgtctctttccagcaaaagccggaaaggaacatttcacctcctccgtcatccagcacagaagtagatacaataa

SEQ ID NO: 1962 - DNA, 153 bp, Artificial
  synthetic sequence
ttttaagaaagcattcttgggccagatagaactacccaacacaaaacaggactggaaaaagaaatatcctccaataaccaacataaaatctttcaacgtacgggtcaatgtataatagggaacgtttcctccgacacaatgtgacaacggaac

SEQ ID NO: 1963 - DNA, 154 bp, Artificial
  synthetic sequence
taatttaatatcttgtgataccattatcaacaaaatgcagataaacacagattaatgcatattaaaaccattgattccttgtacttcccacactgggaagttctccaggcggtgtttacgttggttccccacagattggcaccgagtttcacag

SEQ ID NO: 1964 - DNA, 120 bp, Artificial
  synthetic sequence
ttagggaggatataataaatagttaatagcgtttcaatatagagttttatacaatattacttcttgattttcagaatttctgtgaattgttttcagtgttttctttatagtatcacaaat

SEQ ID NO: 1965 - DNA, 138 bp, Artificial
  synthetic sequence
acaattctcactgatttttactgtaccgaggtaattcccatcaaaaaaaaagacaccccatgacaaagataccacatatctaaacaaaaaaatgcgacagatttttctgtcgcattcgtagcccataggagaatcgaa

SEQ ID NO: 1966 - DNA, 121 bp, Artificial
  synthetic sequence
gatcactttcatgtcggtgcctgagcgggcctttctctcagactggtcatatgcgatcggatcattagttatcatcccgatcatcccgatcttaaatcattattatgtccctttctttcgc

SEQ ID NO: 1967 - DNA, 155 bp, Artificial
  synthetic sequence
ccacacatgctcgcggatctggtctcttgttaagacttgtcctcgattgcgacataaatattccaacacttcgtattctttagctgtcagctcgatcaaagtcgcttcctttttcacctgctttttagcaatatttatcgttatatcacctattt

SEQ ID NO: 1968 - DNA, 66 bp, Artificial
  synthetic sequence
tattttttctcaacctctgtgaggaacttgtcatcaagctccgcctttataagtacgttctcatca

SEQ ID NO: 1969 - DNA, 145 bp, Artificial
  synthetic sequence
gtgctatgttcagaggagatgttgtagatactcccgatgatgaatggcttaaactttttgatattaatgttcacgcggtcttttatctttctagggaggccatacggcttatgcgggaacataaaatagcggggaacattgtaca

SEQ ID NO: 1970 - DNA, 149 bp, Artificial
  synthetic sequence
aaggggcatatcgcctacgcaactacaaaaggagcagtagtgcaaatgacacgttgcatggctttagactgtgcctcagatggaatacgcataaacgctgtatgccctggtgcaactgatactgcgatgccaatgtcaaagcatagtgc

SEQ ID NO: 1971 - DNA, 133 bp, Artificial
  synthetic sequence
ggcacttgccgcactacaggtgccatagcctgcactgtatatactgcaatcctttcctgttctggccgccggaggatttatgttggttatagtatatacggtaatgcccaagggtaaaatgctgtattctgct

SEQ ID NO: 1972 - DNA, 150 bp, Artificial
  synthetic sequence
ttacggcttaatattaagacttgtttcatacggaatcgatacagggcttattgaaaaagaggatataatctacacgcaaaataggcttttatcgttgttccatatggatgaacccgatgacagttgtacttgccttacagcagataacga

SEQ ID NO: 1973 - DNA, 144 bp, Artificial
  synthetic sequence
ctaataagaaagataagaagtataaaaaggaaaagaaggttattaaaaacccatttttctaaatttataataaaggaagacatacgatgtatatcaaacgccatttggagacgacaattgaaaaactgagcggttgttgtaagg

SEQ ID NO: 1974 - DNA, 141 bp, Artificial
  synthetic sequence
aggaaatggtttatctgcgcaatattgccagggataagtttggcatgaaatttttgtagttttacatgaaaattttgaattttattttcactgttggtatgtagtacaacagattgcttttaagatagctgctagttgatt

SEQ ID NO: 1975 - DNA, 146 bp, Artificial
  synthetic sequence
tccaagtatttgccaaagaaccctttgtgggcatcaaaagcgcgcacaaactccagagttggatgaaaaattctctccaagtgtgcgatcatcactggaggcatgttgactagggcaagtttggcgagattttctgcactcaagag

SEQ ID NO: 1976 - DNA, 155 bp, Artificial
  synthetic sequence
ttgcatgtctttttgaatactggaaatggcgcgttgctggtcatttgtgagaacaaagggtagggcctgtagaaattctctaaggagctgggcattagcatgcccaccaaacttgctttgaaaattccactttttggcattcaaggagagcatat

SEQ ID NO: 1977 - DNA, 125 bp, Artificial
  synthetic sequence
gctatccgctatgggattacgcttattcccacatgaccattccatctctacatgcagagtcaggaataattgtcatagctgctcttatccactttatactggtgcttatctgcatattcgataag

SEQ ID NO: 1978 - DNA, 101 bp, Artificial
  synthetic sequence
tttcctttttgctttcttccaaggagtagtaaatccaccattccaaacagtatttattcatgcagtagatgataatctcgttggacaggtaatgtctgtat

SEQ ID NO: 1979 - DNA, 150 bp, Artificial
  synthetic sequence
ggaatggcaacatttgtaaaaaaccaaacgtacaggactttagctccatttgcaatactcgaagctatcgcatctactggcataagctttgctggagtcctcttattctcaatggttctacatagtgcagaaggatatggctggtattta